European Patent Application EP 4 636 082 A2, published October 22, 2025. Title: PBase protein, fusion protein, nucleic acid, gene integration system and use thereof. Applicant: 北京精缮生物科技有限责任公司. Application EP. The sequence listing filed with the application follows.

SEQUENCE LISTING (140 sequences)

SEQ ID NO: 1 - protein, 1379 aa, synthetic construct
MDKKYSIGLDIGTNSVGWAVITDEYKVPSKKFKVLGNTDRHSIKKNLIGALLFDSGETAEATRLKRTARRRYTRRKNRICYLQEIFSNEMAKVDDSFFHRLEESFLVEEDKKHERHPIFGNIVDEVAYHEKYPTIYHLRKKLVDSTDKADLRLIYLALAHMIKFRGHFLIEGDLNPDNSDVDKLFIQLVQTYNQLFEENPINASGVDAKAILSARLSKSRRLENLIAQLPGEKKNGLFGNLIALSLGLTPNFKSNFDLAEDAKLQLSKDTYDDDLDNLLAQIGDQYADLFLAAKNLSDAILLSDILRVNTEITKAPLSASMIKRYDEHHQDLTLLKALVRQQLPEKYKEIFFDQSKNGYAGYIDGGASQEEFYKFIKPILEKMDGTEELLVKLNREDLLRKQRTFDNGSIPHQIHLGELHAILRRQEDFYPFLKDNREKIEKILTFRIPYYVGPLARGNSRFAWMTRKSEETITPWNFEEVVDKGASAQSFIERMTNFDKNLPNEKVLPKHSLLYEYFTVYNELTKVKYVTEGMRKPAFLSGEQKKAIVDLLFKTNRKVTVKQLKEDYFKKIECFDSVEISGVEDRFNASLGTYHDLLKIIKDKDFLDNEENEDILEDIVLTLTLFEDREMIEERLKTYAHLFDDKVMKQLKRRRYTGWGRLSRKLINGIRDKQSGKTILDFLKSDGFANRNFMQLIHDDSLTFKEDIQKAQVSGQGDSLHEHIANLAGSPAIKKGILQTVKVVDELVKVMGRHKPENIVIEMARENQTTQKGQKNSRERMKRIEEGIKELGSQILKEHPVENTQLQNEKLYLYYLQNGRDMYVDQELDINRLSDYDVDHIVPQSFLKDDSIDNKVLTRSDKNRGKSDNVPSEEVVKKMKNYWRQLLNAKLITQRKFDNLTKAERGGLSELDKAGFIKRQLVETRQITKHVAQILDSRMNTKYDENDKLIREVKVITLKSKLVSDFRKDFQFYKVREINNYHHAHDAYLNAVVGTALIKKYPKLESEFVYGDYKVYDVRKMIAKSEQEIGKATAKYFFYSNIMNFFKTEITLANGEIRKRPLIETNGETGEIVWDKGRDFATVRKVLSMPQVNIVKKTEVQTGGFSKESILPKRNSDKLIARKKDWDPKKYGGFDSPTVAYSVLVVAKVEKGKSKKLKSVKELLGITIMERSSFEKNPIDFLEAKGYKEVKKDLIIKLPKYSLFELENGRKRMLASAGELQKGNELALPSKYVNFLYLASHYEKLKGSPEDNEQKQLFVEQHKHYLDEIIEQISEFSKRVILADANLDKVLSAYNKHRDKPIREQAENIIHLFTLTNLGAPAAFKYFDTTIDRKRYTSTKEVLDATLIHQSITGLYETRIDLSQLGGDSRADPKKKRKV

SEQ ID NO: 2 - protein, 15 aa, synthetic construct
GGGGSGGGGSGGGGS

SEQ ID NO: 3 - protein, 594 aa, synthetic construct
MGSSLDDEHILSALLQSDDELVGEDSDSEVSDHVSEDDVQSDTEEAFIDEVHEVQPTSSGSEILDEQNVIEQPGSSLASNRILTLPQRTIRGKNKHCWSTSKSTRRSRVSALNIVRSQRGPTRMCRNIYDPLLCFKLFFTDEIISEIVKWTNAEISLKRRESMTSATFRDTNEDEIYAFFGILVMTAVRKDNHMSTDDLFDRSLSMVYVSVMSRDRFDFLIRCLRMDDKSIRPTLRENDVFTPVRKIWDLFIHQCIQNYTPGAHLTIDEQLLGFRGRCPFRVYIPNKPSKYGIKILMMCDSGTKYMINGMPYLGRGTQTNGVPLGEYYVKELSKPVHGSCRNITCDNWFTSIPLAKNLLQEPYKLTIVGTVRSNKREIPEVLKNSRSRPVGTSMFCFDGPLTLVSYKPKPAKMVYLLSSCDEDASINESTGKPQMVMYYNQTKGGVDTLDQMCSVMTCSRKTNRWPMALLYGMINIACINSFIIYSHNVSSKGEKVQSRKKFMRNLYMSLTSSFMRKRLEAPTLKRYLRDNISNILPKEVPGTSDDSTEEPVMKKRTYCTYCPSKIRRKANASCKKCKKVICREHNIDMCQSCF

SEQ ID NO: 4 - protein, 1987 aa, synthetic construct
MDKKYSIGLDIGTNSVGWAVITDEYKVPSKKFKVLGNTDRHSIKKNLIGALLFDSGETAEATRLKRTARRRYTRRKNRICYLQEIFSNEMAKVDDSFFHRLEESFLVEEDKKHERHPIFGNIVDEVAYHEKYPTIYHLRKKLVDSTDKADLRLIYLALAHMIKFRGHFLIEGDLNPDNSDVDKLFIQLVQTYNQLFEENPINASGVDAKAILSARLSKSRRLENLIAQLPGEKKNGLFGNLIALSLGLTPNFKSNFDLAEDAKLQLSKDTYDDDLDNLLAQIGDQYADLFLAAKNLSDAILLSDILRVNTEITKAPLSASMIKRYDEHHQDLTLLKALVRQQLPEKYKEIFFDQSKNGYAGYIDGGASQEEFYKFIKPILEKMDGTEELLVKLNREDLLRKQRTFDNGSIPHQIHLGELHAILRRQEDFYPFLKDNREKIEKILTFRIPYYVGPLARGNSRFAWMTRKSEETITPWNFEEVVDKGASAQSFIERMTNFDKNLPNEKVLPKHSLLYEYFTVYNELTKVKYVTEGMRKPAFLSGEQKKAIVDLLFKTNRKVTVKQLKEDYFKKIECFDSVEISGVEDRFNASLGTYHDLLKIIKDKDFLDNEENEDILEDIVLTLTLFEDREMIEERLKTYAHLFDDKVMKQLKRRRYTGWGRLSRKLINGIRDKQSGKTILDFLKSDGFANRNFMQLIHDDSLTFKEDIQKAQVSGQGDSLHEHIANLAGSPAIKKGILQTVKVVDELVKVMGRHKPENIVIEMARENQTTQKGQKNSRERMKRIEEGIKELGSQILKEHPVENTQLQNEKLYLYYLQNGRDMYVDQELDINRLSDYDVDHIVPQSFLKDDSIDNKVLTRSDKNRGKSDNVPSEEVVKKMKNYWRQLLNAKLITQRKFDNLTKAERGGLSELDKAGFIKRQLVETRQITKHVAQILDSRMNTKYDENDKLIREVKVITLKSKLVSDFRKDFQFYKVREINNYHHAHDAYLNAVVGTALIKKYPKLESEFVYGDYKVYDVRKMIAKSEQEIGKATAKYFFYSNIMNFFKTEITLANGEIRKRPLIETNGETGEIVWDKGRDFATVRKVLSMPQVNIVKKTEVQTGGFSKESILPKRNSDKLIARKKDWDPKKYGGFDSPTVAYSVLVVAKVEKGKSKKLKSVKELLGITIMERSSFEKNPIDFLEAKGYKEVKKDLIIKLPKYSLFELENGRKRMLASAGELQKGNELALPSKYVNFLYLASHYEKLKGSPEDNEQKQLFVEQHKHYLDEIIEQISEFSKRVILADANLDKVLSAYNKHRDKPIREQAENIIHLFTLTNLGAPAAFKYFDTTIDRKRYTSTKEVLDATLIHQSITGLYETRIDLSQLGGDSRADPKKKRKVGGGGSGGGGSGGGGSGSSLDDEHILSALLQSDDELVGEDSDSEVSDHVSEDDVQSDTEEAFIDEVHEVQPTSSGSEILDEQNVIEQPGSSLASNRILTLPQRTIRGKNKHCWSTSKSTRRSRVSALNIVRSQRGPTRMCRNIYDPLLCFKLFFTDEIISEIVKWTNAEISLKRRESMTSATFRDTNEDEIYAFFGILVMTAVRKDNHMSTDDLFDRSLSMVYVSVMSRDRFDFLIRCLRMDDKSIRPTLRENDVFTPVRKIWDLFIHQCIQNYTPGAHLTIDEQLLGFRGRCPFRVYIPNKPSKYGIKILMMCDSGTKYMINGMPYLGRGTQTNGVPLGEYYVKELSKPVHGSCRNITCDNWFTSIPLAKNLLQEPYKLTIVGTVRSNKREIPEVLKNSRSRPVGTSMFCFDGPLTLVSYKPKPAKMVYLLSSCDEDASINESTGKPQMVMYYNQTKGGVDTLDQMCSVMTCSRKTNRWPMALLYGMINIACINSFIIYSHNVSSKGEKVQSRKKFMRNLYMSLTSSFMRKRLEAPTLKRYLRDNISNILPKEVPGTSDDSTEEPVMKKRTYCTYCPSKIRRKANASCKKCKKVICREHNIDMCQSCF

SEQ ID NO: 5 - protein, 594 aa, synthetic construct
MGSSLDDEHILSALLQSDDELVGEDSDSEVSDHVSEDDVQSDTEEAFIDEVHEVQPTSSGSEILDEQNVIEQPGSSLASNRILTLPQRTIRGKNKHCWSTSKSTRRSRVSALNIVRSQRGPTRMCRNIYDPLLCFKLFFTDEIISEIVKWTNAEISLKRRESMTSATFRDTNEDEIYAFFGILVMTAVRKDNHMSTDDLFDRSLSMVYVSVMSRDRFDFLIRCLRMDDKSIRPTLRENDVFTPVRKIWDLFIHQCIQNYTPGAHLTIDEQLLGFRGRCPFRVYIPNKPSKYGIKILMMCDSGTKYMINGMPYLGAGTQTNGVPLGEYYVKELSKPVHGSCRNITCDEWFTSIPLAKNLLQEPYKLTIVGTVRSNKREIPEVLKNSRSRPVGTSMFCFDGPLTLVSYKPKPAKMVYLLSSCDEDASINESTGKPQMVMYYNQTKGGVDTLNQMCSVMTCSRKTNRWPMALLYGMINIACINSFIIYSHNVSSKGEKVQSRKKFMRNLYMSLTSSFMRKRLEAPTLKRYLRDNISNILPKEVPGTSDDSTEEPVMKKRTYCTYCPSKIRRKANASCKKCKKVICREHNIDMCQSCF

SEQ ID NO: 6 - protein, 1987 aa, synthetic construct
MDKKYSIGLDIGTNSVGWAVITDEYKVPSKKFKVLGNTDRHSIKKNLIGALLFDSGETAEATRLKRTARRRYTRRKNRICYLQEIFSNEMAKVDDSFFHRLEESFLVEEDKKHERHPIFGNIVDEVAYHEKYPTIYHLRKKLVDSTDKADLRLIYLALAHMIKFRGHFLIEGDLNPDNSDVDKLFIQLVQTYNQLFEENPINASGVDAKAILSARLSKSRRLENLIAQLPGEKKNGLFGNLIALSLGLTPNFKSNFDLAEDAKLQLSKDTYDDDLDNLLAQIGDQYADLFLAAKNLSDAILLSDILRVNTEITKAPLSASMIKRYDEHHQDLTLLKALVRQQLPEKYKEIFFDQSKNGYAGYIDGGASQEEFYKFIKPILEKMDGTEELLVKLNREDLLRKQRTFDNGSIPHQIHLGELHAILRRQEDFYPFLKDNREKIEKILTFRIPYYVGPLARGNSRFAWMTRKSEETITPWNFEEVVDKGASAQSFIERMTNFDKNLPNEKVLPKHSLLYEYFTVYNELTKVKYVTEGMRKPAFLSGEQKKAIVDLLFKTNRKVTVKQLKEDYFKKIECFDSVEISGVEDRFNASLGTYHDLLKIIKDKDFLDNEENEDILEDIVLTLTLFEDREMIEERLKTYAHLFDDKVMKQLKRRRYTGWGRLSRKLINGIRDKQSGKTILDFLKSDGFANRNFMQLIHDDSLTFKEDIQKAQVSGQGDSLHEHIANLAGSPAIKKGILQTVKVVDELVKVMGRHKPENIVIEMARENQTTQKGQKNSRERMKRIEEGIKELGSQILKEHPVENTQLQNEKLYLYYLQNGRDMYVDQELDINRLSDYDVDHIVPQSFLKDDSIDNKVLTRSDKNRGKSDNVPSEEVVKKMKNYWRQLLNAKLITQRKFDNLTKAERGGLSELDKAGFIKRQLVETRQITKHVAQILDSRMNTKYDENDKLIREVKVITLKSKLVSDFRKDFQFYKVREINNYHHAHDAYLNAVVGTALIKKYPKLESEFVYGDYKVYDVRKMIAKSEQEIGKATAKYFFYSNIMNFFKTEITLANGEIRKRPLIETNGETGEIVWDKGRDFATVRKVLSMPQVNIVKKTEVQTGGFSKESILPKRNSDKLIARKKDWDPKKYGGFDSPTVAYSVLVVAKVEKGKSKKLKSVKELLGITIMERSSFEKNPIDFLEAKGYKEVKKDLIIKLPKYSLFELENGRKRMLASAGELQKGNELALPSKYVNFLYLASHYEKLKGSPEDNEQKQLFVEQHKHYLDEIIEQISEFSKRVILADANLDKVLSAYNKHRDKPIREQAENIIHLFTLTNLGAPAAFKYFDTTIDRKRYTSTKEVLDATLIHQSITGLYETRIDLSQLGGDSRADPKKKRKVGGGGSGGGGSGGGGSGSSLDDEHILSALLQSDDELVGEDSDSEVSDHVSEDDVQSDTEEAFIDEVHEVQPTSSGSEILDEQNVIEQPGSSLASNRILTLPQRTIRGKNKHCWSTSKSTRRSRVSALNIVRSQRGPTRMCRNIYDPLLCFKLFFTDEIISEIVKWTNAEISLKRRESMTSATFRDTNEDEIYAFFGILVMTAVRKDNHMSTDDLFDRSLSMVYVSVMSRDRFDFLIRCLRMDDKSIRPTLRENDVFTPVRKIWDLFIHQCIQNYTPGAHLTIDEQLLGFRGRCPFRVYIPNKPSKYGIKILMMCDSGTKYMINGMPYLGAGTQTNGVPLGEYYVKELSKPVHGSCRNITCDEWFTSIPLAKNLLQEPYKLTIVGTVRSNKREIPEVLKNSRSRPVGTSMFCFDGPLTLVSYKPKPAKMVYLLSSCDEDASINESTGKPQMVMYYNQTKGGVDTLNQMCSVMTCSRKTNRWPMALLYGMINIACINSFIIYSHNVSSKGEKVQSRKKFMRNLYMSLTSSFMRKRLEAPTLKRYLRDNISNILPKEVPGTSDDSTEEPVMKKRTYCTYCPSKIRRKANASCKKCKKVICREHNIDMCQSCF

SEQ ID NO: 7 - protein, 594 aa, synthetic construct
MGSSLDDEHILSALLQSDDELVGEDSDSEVSDHVSEDDVQSDTEEAFIDEVHEVQPTSSGSEILDEQNVIEQPGSSLASNRILTLPQRTIRGKNKHCWSTSKSTRRSRVSALNIVRSQRGPTRMCRNIYDPLLCFKLFFTDEIISEIVKWTNAEISLKRRESMTSATFRDTNEDEIYAFFGILVMTAVRKDNHMSTDDLFDRSLSMVYVSVMSRDRFDFLIRCLRMDDKSIRPTLRENDVFTPVRKIWDLFIHQCIQNYTPGAHLTIDEQLLGFRGRCPFRVYIPNKPSKYGIKILMMCDSGTKYMINGMPYLGRGTQTNGVPLGEYYVKELSKPVHGSCRNITCDEWFTSIPLAKNLLQEPYKLTIVGTVRSNKEEIPEVLKNSRSRPVGTSMFCFDGPLTLVSYKPKPAKMVYLLSSCDEDASINESTGKPQMVMYYNQTKGGVDTLNQMCSVMTCSRKTNRWPMALLYGMINIACINSFIIYSHNVSSKGEKVQSRKKFMRNLYMSLTSSFMRKRLEAPTLKRYLRDNISNILPKEVPGTSDDSTEEPVMKKRTYCTYCPSKIRRKANASCKKCKKVICREHNIDMCQSCF

SEQ ID NO: 8 - protein, 1987 aa, synthetic construct
MDKKYSIGLDIGTNSVGWAVITDEYKVPSKKFKVLGNTDRHSIKKNLIGALLFDSGETAEATRLKRTARRRYTRRKNRICYLQEIFSNEMAKVDDSFFHRLEESFLVEEDKKHERHPIFGNIVDEVAYHEKYPTIYHLRKKLVDSTDKADLRLIYLALAHMIKFRGHFLIEGDLNPDNSDVDKLFIQLVQTYNQLFEENPINASGVDAKAILSARLSKSRRLENLIAQLPGEKKNGLFGNLIALSLGLTPNFKSNFDLAEDAKLQLSKDTYDDDLDNLLAQIGDQYADLFLAAKNLSDAILLSDILRVNTEITKAPLSASMIKRYDEHHQDLTLLKALVRQQLPEKYKEIFFDQSKNGYAGYIDGGASQEEFYKFIKPILEKMDGTEELLVKLNREDLLRKQRTFDNGSIPHQIHLGELHAILRRQEDFYPFLKDNREKIEKILTFRIPYYVGPLARGNSRFAWMTRKSEETITPWNFEEVVDKGASAQSFIERMTNFDKNLPNEKVLPKHSLLYEYFTVYNELTKVKYVTEGMRKPAFLSGEQKKAIVDLLFKTNRKVTVKQLKEDYFKKIECFDSVEISGVEDRFNASLGTYHDLLKIIKDKDFLDNEENEDILEDIVLTLTLFEDREMIEERLKTYAHLFDDKVMKQLKRRRYTGWGRLSRKLINGIRDKQSGKTILDFLKSDGFANRNFMQLIHDDSLTFKEDIQKAQVSGQGDSLHEHIANLAGSPAIKKGILQTVKVVDELVKVMGRHKPENIVIEMARENQTTQKGQKNSRERMKRIEEGIKELGSQILKEHPVENTQLQNEKLYLYYLQNGRDMYVDQELDINRLSDYDVDHIVPQSFLKDDSIDNKVLTRSDKNRGKSDNVPSEEVVKKMKNYWRQLLNAKLITQRKFDNLTKAERGGLSELDKAGFIKRQLVETRQITKHVAQILDSRMNTKYDENDKLIREVKVITLKSKLVSDFRKDFQFYKVREINNYHHAHDAYLNAVVGTALIKKYPKLESEFVYGDYKVYDVRKMIAKSEQEIGKATAKYFFYSNIMNFFKTEITLANGEIRKRPLIETNGETGEIVWDKGRDFATVRKVLSMPQVNIVKKTEVQTGGFSKESILPKRNSDKLIARKKDWDPKKYGGFDSPTVAYSVLVVAKVEKGKSKKLKSVKELLGITIMERSSFEKNPIDFLEAKGYKEVKKDLIIKLPKYSLFELENGRKRMLASAGELQKGNELALPSKYVNFLYLASHYEKLKGSPEDNEQKQLFVEQHKHYLDEIIEQISEFSKRVILADANLDKVLSAYNKHRDKPIREQAENIIHLFTLTNLGAPAAFKYFDTTIDRKRYTSTKEVLDATLIHQSITGLYETRIDLSQLGGDSRADPKKKRKVGGGGSGGGGSGGGGSGSSLDDEHILSALLQSDDELVGEDSDSEVSDHVSEDDVQSDTEEAFIDEVHEVQPTSSGSEILDEQNVIEQPGSSLASNRILTLPQRTIRGKNKHCWSTSKSTRRSRVSALNIVRSQRGPTRMCRNIYDPLLCFKLFFTDEIISEIVKWTNAEISLKRRESMTSATFRDTNEDEIYAFFGILVMTAVRKDNHMSTDDLFDRSLSMVYVSVMSRDRFDFLIRCLRMDDKSIRPTLRENDVFTPVRKIWDLFIHQCIQNYTPGAHLTIDEQLLGFRGRCPFRVYIPNKPSKYGIKILMMCDSGTKYMINGMPYLGRGTQTNGVPLGEYYVKELSKPVHGSCRNITCDEWFTSIPLAKNLLQEPYKLTIVGTVRSNKEEIPEVLKNSRSRPVGTSMFCFDGPLTLVSYKPKPAKMVYLLSSCDEDASINESTGKPQMVMYYNQTKGGVDTLNQMCSVMTCSRKTNRWPMALLYGMINIACINSFIIYSHNVSSKGEKVQSRKKFMRNLYMSLTSSFMRKRLEAPTLKRYLRDNISNILPKEVPGTSDDSTEEPVMKKRTYCTYCPSKIRRKANASCKKCKKVICREHNIDMCQSCF

SEQ ID NO: 9 - protein, 594 aa, synthetic construct
MGSSLDDEHILSALLQSDDELVGEDSDSEVSDHVSEDDVQSDTEEAFIDEVHEVQPTSSGSEILDEQNVIEQPGSSLASNRILTLPQRTIRGKNKHCWSTSKSTRRSRVSALNIVRSQRGPTRMCRNIYDPLLCFKLFFTDEIISEIVKWTNAEISLKRRESMTSATFRDTNEDEIYAFFGILVMTAVRKDNHMSTDDLFDRSLSMVYVSVMSRDRFDFLIRCLRMDDKSIRPTLRENDVFTPVRKIWDLFIHQCIQNYTPGAHLTIDEQLLGFRGRCPFRVYIPNKPSKYGIKILMMCDSGTKYMINGMPYLGRGTQTNGVPLGEYYVKELSKPVHGSCRNITCDAWFTSIPLAKNLLQEPYKLTIVGTVRSNKEEIPEVLKNSRSRPVGTSMFCFDGPLTLVSYKPKPAKMVYLLSSCDEDASINESTGKPQMVMYYNQTKGGVDTLNQMCSVMTCSRKTNRWPMALLYGMINIACINSFIIYSHNVSSKGEKVQSRKKFMRNLYMSLTSSFMRKRLEAPTLKRYLRDNISNILPKEVPGTSDDSTEEPVMKKRTYCTYCPSKIRRKANASCKKCKKVICREHNIDMCQSCF

SEQ ID NO: 10 - protein, 1987 aa, synthetic construct
MDKKYSIGLDIGTNSVGWAVITDEYKVPSKKFKVLGNTDRHSIKKNLIGALLFDSGETAEATRLKRTARRRYTRRKNRICYLQEIFSNEMAKVDDSFFHRLEESFLVEEDKKHERHPIFGNIVDEVAYHEKYPTIYHLRKKLVDSTDKADLRLIYLALAHMIKFRGHFLIEGDLNPDNSDVDKLFIQLVQTYNQLFEENPINASGVDAKAILSARLSKSRRLENLIAQLPGEKKNGLFGNLIALSLGLTPNFKSNFDLAEDAKLQLSKDTYDDDLDNLLAQIGDQYADLFLAAKNLSDAILLSDILRVNTEITKAPLSASMIKRYDEHHQDLTLLKALVRQQLPEKYKEIFFDQSKNGYAGYIDGGASQEEFYKFIKPILEKMDGTEELLVKLNREDLLRKQRTFDNGSIPHQIHLGELHAILRRQEDFYPFLKDNREKIEKILTFRIPYYVGPLARGNSRFAWMTRKSEETITPWNFEEVVDKGASAQSFIERMTNFDKNLPNEKVLPKHSLLYEYFTVYNELTKVKYVTEGMRKPAFLSGEQKKAIVDLLFKTNRKVTVKQLKEDYFKKIECFDSVEISGVEDRFNASLGTYHDLLKIIKDKDFLDNEENEDILEDIVLTLTLFEDREMIEERLKTYAHLFDDKVMKQLKRRRYTGWGRLSRKLINGIRDKQSGKTILDFLKSDGFANRNFMQLIHDDSLTFKEDIQKAQVSGQGDSLHEHIANLAGSPAIKKGILQTVKVVDELVKVMGRHKPENIVIEMARENQTTQKGQKNSRERMKRIEEGIKELGSQILKEHPVENTQLQNEKLYLYYLQNGRDMYVDQELDINRLSDYDVDHIVPQSFLKDDSIDNKVLTRSDKNRGKSDNVPSEEVVKKMKNYWRQLLNAKLITQRKFDNLTKAERGGLSELDKAGFIKRQLVETRQITKHVAQILDSRMNTKYDENDKLIREVKVITLKSKLVSDFRKDFQFYKVREINNYHHAHDAYLNAVVGTALIKKYPKLESEFVYGDYKVYDVRKMIAKSEQEIGKATAKYFFYSNIMNFFKTEITLANGEIRKRPLIETNGETGEIVWDKGRDFATVRKVLSMPQVNIVKKTEVQTGGFSKESILPKRNSDKLIARKKDWDPKKYGGFDSPTVAYSVLVVAKVEKGKSKKLKSVKELLGITIMERSSFEKNPIDFLEAKGYKEVKKDLIIKLPKYSLFELENGRKRMLASAGELQKGNELALPSKYVNFLYLASHYEKLKGSPEDNEQKQLFVEQHKHYLDEIIEQISEFSKRVILADANLDKVLSAYNKHRDKPIREQAENIIHLFTLTNLGAPAAFKYFDTTIDRKRYTSTKEVLDATLIHQSITGLYETRIDLSQLGGDSRADPKKKRKVGGGGSGGGGSGGGGSGSSLDDEHILSALLQSDDELVGEDSDSEVSDHVSEDDVQSDTEEAFIDEVHEVQPTSSGSEILDEQNVIEQPGSSLASNRILTLPQRTIRGKNKHCWSTSKSTRRSRVSALNIVRSQRGPTRMCRNIYDPLLCFKLFFTDEIISEIVKWTNAEISLKRRESMTSATFRDTNEDEIYAFFGILVMTAVRKDNHMSTDDLFDRSLSMVYVSVMSRDRFDFLIRCLRMDDKSIRPTLRENDVFTPVRKIWDLFIHQCIQNYTPGAHLTIDEQLLGFRGRCPFRVYIPNKPSKYGIKILMMCDSGTKYMINGMPYLGRGTQTNGVPLGEYYVKELSKPVHGSCRNITCDAWFTSIPLAKNLLQEPYKLTIVGTVRSNKEEIPEVLKNSRSRPVGTSMFCFDGPLTLVSYKPKPAKMVYLLSSCDEDASINESTGKPQMVMYYNQTKGGVDTLNQMCSVMTCSRKTNRWPMALLYGMINIACINSFIIYSHNVSSKGEKVQSRKKFMRNLYMSLTSSFMRKRLEAPTLKRYLRDNISNILPKEVPGTSDDSTEEPVMKKRTYCTYCPSKIRRKANASCKKCKKVICREHNIDMCQSCF

SEQ ID NO: 11 - protein, 594 aa, synthetic construct
MGSSLDDEHILSALLQSDDELVGEDSDSEVSDHVSEDDVQSDTEEAFIDEVHEVQPTSSGSEILDEQNVIEQPGSSLASNRILTLPQRTIRGKNKHCWSTSKSTRRSRVSALNIVRSQRGPTRMCRNIYDPLLCFKLFFTDEIISEIVKWTNAEISLKRRESMTSATFRDTNEDEIYAFFGILVMTAVRKDNHMSTDDLFDRSLSMVYVSVMSRDRFDFLIRCLRMDDKSIRPTLRENDVFTPVRKIWDLFIHQCIQNYTPGAHLTIDEQLLGFRGRCPFRVYIPNKPSKYGIKILMMCDSGTKYMINGMPYLGRGTQTNGVPLGEYYVKELSKPVHGSCRNITCDNWFTSIPLAKNLLQEPYKLTIVGTVASNAREIPEVLKNSRSRPVGTSMFCFDGPLTLVSYKPKPAKMVYLLSSCDEDASINESTGKPQMVMYYNQTKGGVDTLNQMCSVMTCSRKTNRWPMALLYGMINIACINSFIIYSHNVSSKGEKVQSRKKFMRNLYMSLTSSFMRKRLEAPTLKRYLRDNISNILPKEVPGTSDDSTEEPVMKKRTYCTYCPSKIRRKANASCKKCKKVICREHNIDMCQSCF

SEQ ID NO: 12 - protein, 1987 aa, synthetic construct
MDKKYSIGLDIGTNSVGWAVITDEYKVPSKKFKVLGNTDRHSIKKNLIGALLFDSGETAEATRLKRTARRRYTRRKNRICYLQEIFSNEMAKVDDSFFHRLEESFLVEEDKKHERHPIFGNIVDEVAYHEKYPTIYHLRKKLVDSTDKADLRLIYLALAHMIKFRGHFLIEGDLNPDNSDVDKLFIQLVQTYNQLFEENPINASGVDAKAILSARLSKSRRLENLIAQLPGEKKNGLFGNLIALSLGLTPNFKSNFDLAEDAKLQLSKDTYDDDLDNLLAQIGDQYADLFLAAKNLSDAILLSDILRVNTEITKAPLSASMIKRYDEHHQDLTLLKALVRQQLPEKYKEIFFDQSKNGYAGYIDGGASQEEFYKFIKPILEKMDGTEELLVKLNREDLLRKQRTFDNGSIPHQIHLGELHAILRRQEDFYPFLKDNREKIEKILTFRIPYYVGPLARGNSRFAWMTRKSEETITPWNFEEVVDKGASAQSFIERMTNFDKNLPNEKVLPKHSLLYEYFTVYNELTKVKYVTEGMRKPAFLSGEQKKAIVDLLFKTNRKVTVKQLKEDYFKKIECFDSVEISGVEDRFNASLGTYHDLLKIIKDKDFLDNEENEDILEDIVLTLTLFEDREMIEERLKTYAHLFDDKVMKQLKRRRYTGWGRLSRKLINGIRDKQSGKTILDFLKSDGFANRNFMQLIHDDSLTFKEDIQKAQVSGQGDSLHEHIANLAGSPAIKKGILQTVKVVDELVKVMGRHKPENIVIEMARENQTTQKGQKNSRERMKRIEEGIKELGSQILKEHPVENTQLQNEKLYLYYLQNGRDMYVDQELDINRLSDYDVDHIVPQSFLKDDSIDNKVLTRSDKNRGKSDNVPSEEVVKKMKNYWRQLLNAKLITQRKFDNLTKAERGGLSELDKAGFIKRQLVETRQITKHVAQILDSRMNTKYDENDKLIREVKVITLKSKLVSDFRKDFQFYKVREINNYHHAHDAYLNAVVGTALIKKYPKLESEFVYGDYKVYDVRKMIAKSEQEIGKATAKYFFYSNIMNFFKTEITLANGEIRKRPLIETNGETGEIVWDKGRDFATVRKVLSMPQVNIVKKTEVQTGGFSKESILPKRNSDKLIARKKDWDPKKYGGFDSPTVAYSVLVVAKVEKGKSKKLKSVKELLGITIMERSSFEKNPIDFLEAKGYKEVKKDLIIKLPKYSLFELENGRKRMLASAGELQKGNELALPSKYVNFLYLASHYEKLKGSPEDNEQKQLFVEQHKHYLDEIIEQISEFSKRVILADANLDKVLSAYNKHRDKPIREQAENIIHLFTLTNLGAPAAFKYFDTTIDRKRYTSTKEVLDATLIHQSITGLYETRIDLSQLGGDSRADPKKKRKVGGGGSGGGGSGGGGSGSSLDDEHILSALLQSDDELVGEDSDSEVSDHVSEDDVQSDTEEAFIDEVHEVQPTSSGSEILDEQNVIEQPGSSLASNRILTLPQRTIRGKNKHCWSTSKSTRRSRVSALNIVRSQRGPTRMCRNIYDPLLCFKLFFTDEIISEIVKWTNAEISLKRRESMTSATFRDTNEDEIYAFFGILVMTAVRKDNHMSTDDLFDRSLSMVYVSVMSRDRFDFLIRCLRMDDKSIRPTLRENDVFTPVRKIWDLFIHQCIQNYTPGAHLTIDEQLLGFRGRCPFRVYIPNKPSKYGIKILMMCDSGTKYMINGMPYLGRGTQTNGVPLGEYYVKELSKPVHGSCRNITCDNWFTSIPLAKNLLQEPYKLTIVGTVASNAREIPEVLKNSRSRPVGTSMFCFDGPLTLVSYKPKPAKMVYLLSSCDEDASINESTGKPQMVMYYNQTKGGVDTLNQMCSVMTCSRKTNRWPMALLYGMINIACINSFIIYSHNVSSKGEKVQSRKKFMRNLYMSLTSSFMRKRLEAPTLKRYLRDNISNILPKEVPGTSDDSTEEPVMKKRTYCTYCPSKIRRKANASCKKCKKVICREHNIDMCQSCF

SEQ ID NO: 13 - DNA, 1785 bp, synthetic construct
  source 1..1785: mol_type = other DNA
atgggctctagcctggacgacgagcacatcctgagcgccctgctgcagagcgacgacgaactggtgggcgaggacagcgacagcgaggtcagcgaccacgtgtccgaggacgacgtgcagtccgacaccgaggaagccttcatcgacgaggtgcacgaagtgcagcctaccagcagcggctccgagatcctggacgagcagaacgtgatcgagcagcctggcagctccctggccagcaacagaatcctgaccctgccccagagaaccatcagaggcaagaacaagcactgctggtccacctccaagagcaccaggcggagcagagtgtccgccctgaacatcgtgcggagccagaggggccccaccagaatgtgcagaaacatctacgaccccctgctgtgcttcaagctgttcttcaccgacgagatcatcagcgagatcgtgaagtggaccaacgccgagatcagcctgaagaggcgggagagcatgaccagcgccaccttcagagacaccaacgaggacgagatctacgccttcttcggcatcctggtgatgaccgccgtgagaaaggacaaccacatgagcaccgacgacctgttcgacagatccctgagcatggtgtacgtgtccgtgatgagcagagacagattcgacttcctgatcagatgcctgagaatggacgacaagagcatcagacccaccctgcgggagaacgacgtgttcacccccgtgcggaagatctgggacctgttcatccaccagtgcatccagaactacacccctggcgcccacctgaccatcgatgagcagctgctgggcttcagaggcagatgccccttcagagtgtacatccccaacaagcccagcaagtacggcatcaagatcctgatgatgtgcgacagcggcaccaagtacatgatcaacggcatgccctacctgggcagaggcacccagacaaacggcgtgcccctgggcgagtactacgtgaaagaactgagcaagcctgtgcatggcagctgcaggaacatcacctgcgacaactggttcaccagcatccccctggccaagaacctgctgcaggaaccctacaagctgaccatcgtgggcaccgtgcggagcaacaagcgggagatcccagaggtgctgaagaacagcagatccagacctgtgggaacaagcatgttctgcttcgacggccccctgaccctggtgtcctacaagcccaagcccgccaagatggtgtacctgctgtccagctgcgacgaggacgccagcatcaacgagagcaccggcaagccccagatggtgatgtactacaaccagaccaagggcggcgtggacaccctggaccagatgtgcagcgtgatgacctgcagcagaaagaccaacagatggcccatggccctgctgtacggcatgatcaatatcgcctgcatcaacagcttcatcatctacagccacaacgtgtccagcaagggcgagaaggtgcagagccggaagaaattcatgcggaacctgtacatgagcctgacctccagcttcatgagaaagagactggaagcccccaccctgaagagatacctgcgggacaacatcagcaacatcctgcccaaggaagtgccaggaacaagcgacgacagcaccgaggaacccgtgatgaagaagaggacctactgcacctactgtcccagcaagatcagaagaaaggccaacgccagctgcaagaaatgcaaaaaagtgatctgccgggagcacaacatcgacatgtgccagagctgtttctga

SEQ ID NO: 14 - DNA, 5964 bp, synthetic construct
  source 1..5964: mol_type = other DNA
atggacaagaagtactccattgggctcgacatcggcacaaacagcgtcggctgggccgtcattacggacgagtacaaggtgccgagcaaaaaattcaaagttctgggcaataccgatcgccacagcataaagaagaacctcattggcgccctcctgttcgactccggggagacggccgaagccacgcggctcaaaagaacagcacggcgcagatatacccgcagaaagaatcggatctgctacctgcaggagatctttagtaatgagatggctaaggtggatgactctttcttccataggctggaggagtcctttttggtggaggaggataaaaagcacgagcgccacccaatctttggcaatatcgtggacgaggtggcgtaccatgaaaagtacccaaccatatatcatctgaggaagaagcttgtagacagtactgataaggctgacttgcggttgatctatctcgcgctggcgcatatgatcaaatttcggggacacttcctcatcgagggggacctgaacccagacaacagcgatgtcgacaaactctttatccaactggttcagacttacaatcagcttttcgaagagaacccgatcaacgcatccggagttgacgccaaagcaatcctgagcgctaggctgtccaaatcccggcggctcgaaaacctcatcgcacagctccctggggagaagaagaacggcctgtttggtaatcttatcgccctgtcactcgggctgacccccaactttaaatctaacttcgacctggccgaagatgccaagcttcaactgagcaaagacacctacgatgatgatctcgacaatctgctggcccagatcggcgaccagtacgcagacctttttttggcggcaaagaacctgtcagacgccattctgctgagtgatattctgcgagtgaacacggagatcaccaaagctccgctgagcgctagtatgatcaagcgctatgatgagcaccaccaagacttgactttgctgaaggcccttgtcagacagcaactgcctgagaagtacaaggaaattttcttcgatcagtctaaaaatggctacgccggatacattgacggcggagcaagccaggaggaattttacaaatttattaagcccatcttggaaaaaatggacggcaccgaggagctgctggtaaagcttaacagagaagatctgttgcgcaaacagcgcactttcgacaatggaagcatcccccaccagattcacctgggcgaactgcacgctatcctcaggcggcaagaggatttctacccctttttgaaagataacagggaaaagattgagaaaatcctcacatttcggataccctactatgtaggccccctcgcccggggaaattccagattcgcgtggatgactcgcaaatcagaagagaccatcactccctggaacttcgaggaagtcgtggataagggggcctctgcccagtccttcatcgaaaggatgactaactttgataaaaatctgcctaacgaaaaggtgcttcctaaacactctctgctgtacgagtacttcacagtttataacgagctcaccaaggtcaaatacgtcacagaagggatgagaaagccagcattcctgtctggagagcagaagaaagctatcgtggacctcctcttcaagacgaaccggaaagttaccgtgaaacagctcaaagaagactatttcaaaaagattgaatgtttcgactctgttgaaatcagcggagtggaggatcgcttcaacgcatccctgggaacgtatcacgatctcctgaaaatcattaaagacaaggacttcctggacaatgaggagaacgaggacattcttgaggacattgtcctcacccttacgttgtttgaagatagggagatgattgaagaacgcttgaaaacttacgctcatctcttcgacgacaaagtcatgaaacagctcaagaggcgccgatatacaggatgggggcggctgtcaagaaaactgatcaatgggatccgagacaagcagagtggaaagacaatcctggattttcttaagtccgatggatttgccaacaggaacttcatgcagttgatccatgatgactctctcacctttaaggaggacatccagaaagcacaagtttctggccagggggacagtcttcacgagcacatcgctaatcttgcaggtagcccagctatcaaaaagggaatactgcagaccgttaaggtcgtggatgaactcgtcaaagtaatgggaaggcataagcccgagaatatcgttatcgagatggcccgagagaaccaaactacccagaagggacagaagaacagtagggaaaggatgaagaggattgaagagggtataaaagaactggggtcccaaatccttaaggaacacccagttgaaaacacccagcttcagaatgagaagctctacctgtactacctgcagaacggcagggacatgtacgtggatcaggaactggacatcaatcggctctccgactacgacgtggatcatatcgtgccccagtcttttctcaaagatgattctattgataataaagtgttgacaagatccgataaaaatagagggaagagtgataacgtcccctcagaagaagttgtcaagaaaatgaaaaattattggcggcagctgctgaacgccaaactgatcacacaacggaagttcgataatctgactaaggctgaacgaggtggcctgtctgagttggataaagccggcttcatcaaaaggcagcttgttgagacacgccagatcaccaagcacgtggcccaaattctcgattcacgcatgaacaccaagtacgatgaaaatgacaaactgattcgagaggtgaaagttattactctgaagtctaagctggtctcagatttcagaaaggactttcagttttataaggtgagagagatcaacaattaccaccatgcgcatgatgcctacctgaatgcagtggtaggcactgcacttatcaaaaaatatcccaagcttgaatctgaatttgtttacggagactataaagtgtacgatgttaggaaaatgatcgcaaagtctgagcaggaaataggcaaggccaccgctaagtacttcttttacagcaatattatgaattttttcaagaccgagattacactggccaatggagagattcggaagcgaccacttatcgaaacaaacggagaaacaggagaaatcgtgtgggacaagggtagggatttcgcgacagtccggaaggtcctgtccatgccgcaggtgaacatcgttaaaaagaccgaagtacagaccggaggcttctccaaggaaagtatcctcccgaaaaggaacagcgacaagctgatcgcacgcaaaaaagattgggaccccaagaaatacggcggattcgattctcctacagtcgcttacagtgtactggttgtggccaaagtggagaaagggaagtctaaaaaactcaaaagcgtcaaggaactgctgggcatcacaatcatggagcgatcaagcttcgaaaaaaaccccatcgactttctcgaggcgaaaggatataaagaggtcaaaaaagacctcatcattaagcttcccaagtactctctctttgagcttgaaaacggccggaaacgaatgctcgctagtgcgggcgagctgcagaaaggtaacgagctggcactgccctctaaatacgttaatttcttgtatctggccagccactatgaaaagctcaaagggtctcccgaagataatgagcagaagcagctgttcgtggaacaacacaaacactaccttgatgagatcatcgagcaaataagcgaattctccaaaagagtgatcctcgccgacgctaacctcgataaggtgctttctgcttacaataagcacagggataagcccatcagggagcaggcagaaaacattatccacttgtttactctgaccaacttgggcgcgcctgcagccttcaagtacttcgacaccaccatagacagaaagcggtacacctctacaaaggaggtcctggacgccacactgattcatcagtcaattacggggctctatgaaacaagaatcgacctctctcagctcggtggagacagcagggctgaccccaagaagaagaggaaggtgggcggaggagggagtggcggaggcggaagcggcggcggaggcagcggctctagcctggacgacgagcacatcctgagcgccctgctgcagagcgacgacgaactggtgggcgaggacagcgacagcgaggtcagcgaccacgtgtccgaggacgacgtgcagtccgacaccgaggaagccttcatcgacgaggtgcacgaagtgcagcctaccagcagcggctccgagatcctggacgagcagaacgtgatcgagcagcctggcagctccctggccagcaacagaatcctgaccctgccccagagaaccatcagaggcaagaacaagcactgctggtccacctccaagagcaccaggcggagcagagtgtccgccctgaacatcgtgcggagccagaggggccccaccagaatgtgcagaaacatctacgaccccctgctgtgcttcaagctgttcttcaccgacgagatcatcagcgagatcgtgaagtggaccaacgccgagatcagcctgaagaggcgggagagcatgaccagcgccaccttcagagacaccaacgaggacgagatctacgccttcttcggcatcctggtgatgaccgccgtgagaaaggacaaccacatgagcaccgacgacctgttcgacagatccctgagcatggtgtacgtgtccgtgatgagcagagacagattcgacttcctgatcagatgcctgagaatggacgacaagagcatcagacccaccctgcgggagaacgacgtgttcacccccgtgcggaagatctgggacctgttcatccaccagtgcatccagaactacacccctggcgcccacctgaccatcgatgagcagctgctgggcttcagaggcagatgccccttcagagtgtacatccccaacaagcccagcaagtacggcatcaagatcctgatgatgtgcgacagcggcaccaagtacatgatcaacggcatgccctacctgggcagaggcacccagacaaacggcgtgcccctgggcgagtactacgtgaaagaactgagcaagcctgtgcatggcagctgcaggaacatcacctgcgacaactggttcaccagcatccccctggccaagaacctgctgcaggaaccctacaagctgaccatcgtgggcaccgtgcggagcaacaagcgggagatcccagaggtgctgaagaacagcagatccagacctgtgggaacaagcatgttctgcttcgacggccccctgaccctggtgtcctacaagcccaagcccgccaagatggtgtacctgctgtccagctgcgacgaggacgccagcatcaacgagagcaccggcaagccccagatggtgatgtactacaaccagaccaagggcggcgtggacaccctggaccagatgtgcagcgtgatgacctgcagcagaaagaccaacagatggcccatggccctgctgtacggcatgatcaatatcgcctgcatcaacagcttcatcatctacagccacaacgtgtccagcaagggcgagaaggtgcagagccggaagaaattcatgcggaacctgtacatgagcctgacctccagcttcatgagaaagagactggaagcccccaccctgaagagatacctgcgggacaacatcagcaacatcctgcccaaggaagtgccaggaacaagcgacgacagcaccgaggaacccgtgatgaagaagaggacctactgcacctactgtcccagcaagatcagaagaaaggccaacgccagctgcaagaaatgcaaaaaagtgatctgccgggagcacaacatcgacatgtgccagagctgtttctga

SEQ ID NO: 15 - DNA, 11772 bp, synthetic construct
  source 1..11772: mol_type = other DNA
ctagctagtcctgcaggtttaaacgaattcgccctttgctttctctgaccagcattctctcccctgggcctgtgccgctttctgtctgcagcttgtggcctgggtcacctctacggctggcccagatccttccctgccgcctccttcaggttccgtcttcctccactccctcttccccttgctctctgctgtgttgctgcccaaggatgctctttccggagcacttccttctcggcgctgcaccacgtgatgtcctctgagcggatcctccccgtgtctgggtcctctccgggcatctctcctccctcacccaaccccatgccgtcttcactcgctgggttcccttttccttctccttctggggcctgtgccatctctcgtttcttaggatggccttctccgacggatgtctcccttgcgtcccgcctccccttcttgtaggcctgcatcatcaccgtttttctggacaaccccaaagtaccccgtctccctggctttagccacctctccatcctcttgctttctttgcctggacaccccgttctcctgtggattcgggtcacctctcactcctttcatttgggcagctcccctaccccccttacctctctagtctgtgctagctcttccagccccctgtcatggcatcttccaggggtccgagagctcagctagtcttcttcctccaacccgggcccctatgtccacttcaggacagcatgtttgctgcctccagggatcctgtgtccccgagctgggaccaccttatattcccagggccggttaatgtggctctggttctgggtacttttatctgtcccctccaccccacagtggggcaagcttctgacctcttctcttcctcccacagggcctcgagagatctggcagcggagagggcagaggaagtcttctaacatgcggtgacgtggaggagaatcccggccctaggctcgagatgaccgagtacaagcccacggtgcgcctcgccacccgcgacgacgtccccagggccgtacgcaccctcgccgccgcgttcgccgactaccccgccacgcgccacaccgtcgatccggaccgccacatcgagcgggtcaccgagctgcaagaactcttcctcacgcgcgtcgggctcgacatcggcaaggtgtgggtcgcggacgacggcgccgcggtggcggtctggaccacgccggagagcgtcgaagcgggggcggtgttcgccgagatcggcccgcgcatggccgagttgagcggttcccggctggccgcgcagcaacagatggaaggcctcctggcgccgcaccggcccaaggagcccgcgtggttcctggccaccgtcggcgtctcgcccgaccaccagggcaagggtctgggcagcgccgtcgtgctccccggagtggaggcggccgagcgcgccggggtgcccgccttcctggagacctccgcgccccgcaacctccccttctacgagcggctcggcttcaccgtcaccgccgacgtcgaggtgcccgaaggaccgcgcacctggtgcatgacccgcaagcccggtgcctgatctagagggcccgtttaaacccgctgatcagcctcgactgtgccttctagttgccagccatctgttgtttgcccctcccccgtgccttccttgaccctggaaggtgccactcccactgtcctttcctaataaaatgaggaaattgcatcgcattgtctgagtaggtgtcattctattctggggggtggggtggggcaggacagcaagggggaggattgggaagacaatagcaggcatgctggggatgcggtgggctctatgggtctcgacattgattattgactagttattaatagtaatcaattacggggtcattagttcatagcccatatatggagttccgcgttacataacttacggtaaatggcccgcctggctgaccgcccaacgacccccgcccattgacgtcaataatgacgtatgttcccatagtaacgccaatagggactttccattgacgtcaatgggtggactatttacggtaaactgcccacttggcagtacatcaagtgtatcatatgccaagtacgccccctattgacgtcaatgacggtaaatggcccgcctggcattatgcccagtacatgaccttatgggactttcctacttggcagtacatctacgtattagtcatcgctattaccatgggtcgaggtgagccccacgttctgcttcactctccccatctcccccccctccccacccccaattttgtatttatttattttttaattattttgtgcagcgatgggggcggggggggggggggcgcgcgccaggcggggcggggcggggcgaggggcggggcggggcgaggcggagaggtgcggcggcagccaatcagagcggcgcgctccgaaagtttccttttatggcgaggcggcggcggcggcggccctataaaaagcgaagcgcgcggcgggcgggagtcgctgcgttgccttcgccccgtgccccgctccgcgccgcctcgcgccgcccgccccggctctgactgaccgcgttactcccacaggtgagcgggcgggacggcccttctcctccgggctgtaattagcgcttggtttaatgacggctcgtttcttttctgtggctgcgtgaaagccttaaagggctccgggagggccctttgtgcgggggggagcggctcggggggtgcgtgcgtgtgtgtgtgcgtggggagcgccgcgtgcggcccgcgctgcccggcggctgtgagcgctgcgggcgcggcgcggggctttgtgcgctccgcgtgtgcgcgaggggagcgcggccgggggcggtgccccgcggtgcgggggggctgcgaggggaacaaaggctgcgtgcggggtgtgtgcgtgggggggtgagcagggggtgtgggcgcggcggtcgggctgtaacccccccctgcacccccctccccgagttgctgagcacggcccggcttcgggtgcggggctccgtgcggggcgtggcgcggggctcgccgtgccgggcggggggtggcggcaggtgggggtgccgggcggggcggggccgcctcgggccggggagggctcgggggaggggcgcggcggccccggagcgccggcggctgtcgaggcgcggcgagccgcagccattgccttttatggtaatcgtgcgagagggcgcagggacttcctttgtcccaaatctggcggagccgaaatctgggaggcgccgccgcaccccctctagcgggcgcgggcgaagcggtgcggcgccggcaggaaggaaatgggcggggagggccttcgtgcgtcgccgcgccgccgtccccttctccatctccagcctcggggctgccgcagggggacggctgccttcgggggggacggggcagggcggggttcggcttctggcgtgtgaccggcggctctagagcctctgctaaccatgttcatgccttcttctttttcctacagctcctgggcaacgtgctggttgttgtgctgtctcatcattttggcaaagaattcgtcgacctagactgcagaacacgcagctagattaaccctagaaagataatcatattgtgacgtacgttaaagataatcatgcgtaaaattgacgcatgtgttttatcggtctgtatatcgaggtttatttattaatttgaatagatattaagttttattatatttacacttacatactaataataaattcaacaaacaatttatttatgtttatttatttattaaaaaaaaacaaaaactcaaaatttcttctataaagtaacaaaacttttatgagggacagcccccccccaaagcccccagggatgtaattacgtccctcccccgctagtgggcagcagcgagccgcccggggctccgctccggtccggcgctccccccgcatccccgagccggcagcgtgcggggacagcccgggcacggggaaggtggcacgggatcgctttcctctgaacgcttctcgctgctctttgagcctgcagacacctggggggatacggggaaaaggcctccacggccagactagtaatgtgtgtcagttagggtgtggaaagtccccaggctccccagcaggcagaagtatgcaaagcatgcatctcaattagtcagcaaccaggtgtggaaagtccccaggctccccagcaggcagaagtatgcaaagcatgcatctcaattagtcagcaaccatagtcccgcccctaactccgcccatcccgcccctaactccgcccagttccgcccattctccgccccatggctgactaattttttttatttatgcagaggccgaggccgcctctgcctctgagctattccagaagtagtgaggaggcttttttggaggcctaggcttttgcaaaaagctcccgggagcttgtatatccattttcggatctgatcagcacgtgttgacaattaatcatcggcatagtatatcggcatagtataatacgacaaggtgaggaactaaaccatggccaagcctttgtctcaagaagaatccaccctcattgaaagagcaacggctacaatcaacagcatccccatctctgaagactacagcgtcgccagcgcagctctctctagcgacggccgcatcttcactggtgtcaatgtatatcattttactgggggaccttgtgcagaactcgtggtgctgggcactgctgctgctgcggcagctggcaacctgacttgtatcgtcgcgatcggaaatgagaacaggggcatcttgagcccctgcggacggtgccgacaggtgcttctcgatctgcatcctgggatcaaagccatagtgaaggacagtgatggacagccgacggcagttgggattcgtgaattgctgccctctggttatgtgtgggagggctaagcacttcgtggccgaggagcaggactgacacgtgctacgagatttcgattccaccgccgccttctatgaaaggttgggcttcggaatcgttttccgggacgccggctggatgatcctccagcgcggggatctcatgctggagttcttcgcccaccccaacttgtttattgcagcttataatggttacaaataaagcaatagcatcacaaatttcacaaataaagcatttttttcactgcattctagttgtggtttgtccaaactcatcaatgtatcttatcatgtctggcggccatctataacaagaaaatatatatataataagttatcacgtaagtagaacatgaaataacaatataattatcgtatgagttaaatcttaaaagtcacgtaaaagataatcatgcgtcattttgactcacgcggtcgttatagttcaaaatcagtgacacttaccgcattgacaagcacgcctcacgggagctccaagcggcgactgagatgtcctaaatgcacagcgacggattcgcgctatttagaaagagagagcaatatttcaagaatgcatgcgtcaattttacgcagactatctttctagggttaatctagctgcatcaggatcatatcgtcgtctagacgccaccatggtgtccaagggcgaggaggtgatcaaggagttcatgcgcttcaaggtgcgcatggagggctccatgaacggccacgagttcgagatcgagggcgagggcgagggccgcccctacgagggcacccagaccgccaagctgaaggtgaccaagggcggccccctgcccttcgcctgggacatcctgtccccccagttcatgtacggctccaaggcctacgtgaagcaccccgccgacatccccgactacaagaagctgtccttccccgagggcttcaagtgggagcgcgtgatgaacttcgaggacggcggcctggtgaccgtgacccaggactcctccctgcaggacggcaccctgatctacaaggtgaagatgcgcggcaccaacttcccccccgacggccccgtgatgcagaagaagaccatgggctgggaggcctccaccgagcgcctgtacccccgcgacggcgtgctgaagggcgagatccaccaggccctgaagctgaaggacggcggccactacctggtggagttcaagaccatctacatggccaagaagcccgtgcagctgcccggctactactacgtggacaccaagctggacatcacctcccacaacgaggactacaccatcgtggagcagtacgagcgctccgagggccgccaccacctgttcctgtaaacgcgtgaattcactcctcaggtgcaggctgcctatcagaaggtggtggctggtgtggccaatgccctggctcacaaataccactgagatctttttccctctgccaaaaattatggggacatcatgaagccccttgagcatctgacttctggctaataaaggaaatttattttcattgcaatagtgtgttggaattttttgtgtctctcactcggaaggacatatgggagggcaaatcatttaaaacatcagaatgagtatttggtttagagtttggcaacatatgcccatatgctggctgccatgaacaaaggttggctataaagaggtcatcagtatatgaaacagccccctgctgtccattccttattccatagaaaagccttgacttgaggttagattttttttatattttgttttgtgttatttttttctttaacatccctaaaattttccttacatgttttactagccagatttttcctcctctcctgactactcccagtcatagctgtccctcttctcttatggagatccctcgacctgcagcccaagcttggcgtaatcatggtcatagctgtttcctgtgtgaaattgttatccgctcacaattccacacaacatacgagccggaagcataaagtgtaaagcctggggtgcctaatgagtgagctaactcacattaattgcgttgcgctcactgcccgctttccagtcgggaaacctgtcgtgccagcggatcgacagtactaagctttactagggacaggattggtgacagaaaagccccatccttaggcctcctccttcctagtctcctgatattgggtctaacccccacctcctgttaggcagattccttatctggtgacacacccccatttcctggagccatctctctccttgccagaacctctaaggtttgcttacgatggagccagagaggatcctgggagggagagcttggcagggggtgggagggaagggggggatgcgtgacctgcccggttctcagtggccaccctgcgctaccctctcccagaacctgagctgctctgacgcggctgtctggtgcgtttcactgatcctggtgctgcagcttccttacacttcccaagaggagaagcagtttggaaaaacaaaatcagaataagttggtcctgagttctaactttggctcttcacctttctagtccccaatttatattgttcctccgtgcgtcagttttacctgtgagataaggccagtagccagccccgtcctggcagggctgtggtgaggaggggggtgtccgtgtggaaaactccctttgtgagaatggtgcgtcctaggtgttcaccaggtcgtggccgcctctactccctttctctttctccatccttctttccttaaagagtccccagtgctatctgggacatattcctccgcccagagcagggtcccgcttccctaaggccctgctctgggcttctgggtttgagtccttggcaagcccaggagaggcgctcaggcttccctgtcccccttcctcgtccaccatctcatgcccctggctctcctgccccttccctacaggggttcctggctctgctctaagggcaagggcgaattcgcggccgctaaattcaattcgccctatagtgagtcgtattacaattcactggccgtcgttttacaacgtcgtgactgggaaaaccctggcgttacccaacttaatcgccttgcagcacatccccctttcgccagctggcgtaatagcgaagaggcccgcaccgatcgcccttcccaacagttgcgcagcctatacgtacggcagtttaaggtttacacctataaaagagagagccgttatcgtctgtttgtggatgtacagagtgatattattgacacgccggggcgacggatggtgatccccctggccagtgcacgtctgctgtcagataaagtctcccgtgaactttacccggtggtgcatatcggggatgaaagctggcgcatgatgaccaccgatatggccagtgtgccggtctccgttatcggggaagaagtggctgatctcagccaccgcgaaaatgacatcaaaaacgccattaacctgatgttctggggaatataaatgtcaggcatgagattatcaaaaaggatcttcacctagatccttttcacgtagaaagccagtccgcagaaacggtgctgaccccggatgaatgtcagctactgggctatctggacaagggaaaacgcaagcgcaaagagaaagcaggtagcttgcagtgggcttacatggcgatagctagactgggcggttttatggacagcaagcgaaccggaattgccagctggggcgccctctggtaaggttgggaagccctgcaaagtaaactggatggctttcttgccgccaaggatctgatggcgcaggggatcaagctctgatcaagagacaggatgaggatcgtttcgcatgattgaacaagatggattgcacgcaggttctccggccgcttgggtggagaggctattcggctatgactgggcacaacagacaatcggctgctctgatgccgccgtgttccggctgtcagcgcaggggcgcccggttctttttgtcaagaccgacctgtccggtgccctgaatgaactgcaagacgaggcagcgcggctatcgtggctggccacgacgggcgttccttgcgcagctgtgctcgacgttgtcactgaagcgggaagggactggctgctattgggcgaagtgccggggcaggatctcctgtcatctcaccttgctcctgccgagaaagtatccatcatggctgatgcaatgcggcggctgcatacgcttgatccggctacctgcccattcgaccaccaagcgaaacatcgcatcgagcgagcacgtactcggatggaagccggtcttgtcgatcaggatgatctggacgaagagcatcaggggctcgcgccagccgaactgttcgccaggctcaaggcgagcatgcccgacggcgaggatctcgtcgtgacccatgcatggcgatgcctgcttgccgaatatcatggtggaaaatggccgcttttctggattcatcgactgtggccggctgggtgtggcggaccgctatcaggacatagcgttggctacccgtgatattgctgaagagcttggcggcgaatgggctgaccgcttcctcgtgctttacggtatcgccgctcccgattcgcagcgcatcgccttctatcgccttcttgacgagttcttctgaattattaacgcttacaatttcctgatgcggtattttctccttacgcatctgtgcggtatttcacaccgcatcaggtggcacttttcggggaaatgtgcgcggaacccctatttgtttatttttctaaatacattcaaatatgtatccgctcatgagattatcaaaaaggatcttcacctagatccttttaaattaaaaatgaagttttaaatcaatctaaagtatatatgagtaaacttggtctgacagttaccaatgcttaatcagtgaggcacctatctcagcgatctgtctatttcgttcatccatagttgcctgactccccgtcgtgtagataactacgatacgggagggcttaccatctggccccagtgctgcaatgataccgcgagacccacgctcaccggctccagatttatcagcaataaaccagccagccggaagggccgagcgcagaagtggtcctgcaactttatccgcctccatccagtctattaattgttgccgggaagctagagtaagtagttcgccagttaatagtttgcgcaacgttgttgccattgctacaggcatcgtggtgtcacgctcgtcgtttggtatggcttcattcagctccggttcccaacgatcaaggcgagttacatgatcccccatgttgtgcaaaaaagcggttagctccttcggtcctccgatcgttgtcagaagtaagttggccgcagtgttatcactcatggttatggcagcactgcataattctcttactgtcatgccatccgtaagatgcttttctgtgactggtgagtactcaaccaagtcattctgagaatagtgtatgcggcgaccgagttgctcttgcccggcgtcaatacgggataataccgcgccacatagcagaactttaaaagtgctcatcattggaaaacgttcttcggggcgaaaactctcaaggatcttaccgctgttgagatccagttcgatgtaacccactcgtgcacccaactgatcttcagcatcttttactttcaccagcgtttctgggtgagcaaaaacaggaaggcaaaatgccgcaaaaaagggaataagggcgacacggaaatgttgaatactcatactcttcctttttcaatattattgaagcatttatcagggttattgtctcatgaccaaaatcccttaacgtgagttttcgttccactgagcgtcagaccccgtagaaaagatcaaaggatcttcttgagatcctttttttctgcgcgtaatctgctgcttgcaaacaaaaaaaccaccgctaccagcggtggtttgtttgccggatcaagagctaccaactctttttccgaaggtaactggcttcagcagagcgcagataccaaatactgttcttctagtgtagccgtagttaggccaccacttcaagaactctgtagcaccgcctacatacctcgctctgctaatcctgttaccagtggctgctgccagtggcgataagtcgtgtcttaccgggttggactcaagacgatagttaccggataaggcgcagcggtcgggctgaacggggggttcgtgcacacagcccagcttggagcgaacgacctacaccgaactgagatacctacagcgtgagctatgagaaagcgccacgcttcccgaagggagaaaggcggacaggtatccggtaagcggcagggtcggaacaggagagcgcacgagggagcttccagggggaaacgcctggtatctttatagtcctgtcgggtttcgccacctctgacttgagcgtcgatttttgtgatgctcgtcaggggggcggagcctatggaaaaacgccagcaacgcggcctttttacggttcctggccttttgctggccttttgctcacatgttctttcctgcgttatcccctgattctgtggataaccgtattaccgcctttgagtgagctgataccgctcgccgcagccgaacgaccgagcgcagcgagtcagtgagcgaggaagcggaagagcgcccaatacgcaaaccgcctctccccgcgcgttggccgattcattaatgcagctggcacgacaggtttcccgactggaaagcgggcagtgagcgcaacgcaattaatgtgagttagctcactcattaggcaccccaggctttacactttatgcttccggctcgtatgttgtgtggaattgtgagcggataacaatttcacacaggaaacagctatgaccatgattacgccaagctcagaattaaccctcactaaaggga

SEQ ID NO: 16 - DNA, 5357 bp, synthetic construct
  source 1..5357: mol_type = other DNA
tcgcgcgtttcggtgatgacggtgaaaacctctgacacatgcagctcccggagacggtcacagcttgtctgtaagcggatgccgggagcagacaagcccgtcagggcgcgtcagcgggtgttggcgggtgtcggggctggcttaactatgcggcatcagagcagattgtactgagagtgcaccatatgcggtgtgaaataccgcacagatgcgtaaggagaaaataccgcatcaggcgccattcgccattcaggctgcgcaactgttgggaagggcgatcggtgcgggcctcttcgctattacgccagctggcgaaagggggatgtgctgcaaggcgattaagttgggtaacgccagggttttcccagtcacgacgttgtaaaacgacggccagtgaattggagatcggtacttcgcataacttcgtatagcatacattatacgaagttatgaatgcgtcgagatacgcgtcgcggccgcttgcttggcgcgccgcaggccagtgtgtgagaccgggttgggactagggataacagggtaatcggctgtcgagtcgcttctcgattatggtagccgggctatttacttttgtaaaactttatggtttgtggaaaacaaatgtttttgaacatttaaaaagttcagatgttaaaaagttgaaaggttaatgtaaaacaatcaatattaaagaattttgatgccaaaactattagataaaaggttaatctacatccctactagaattctcatacttaactggttggttatgtggaagaaacatactttcacaataaagagctttaggatatgatgccattttatatcactagtaggcagaccagcagacttttttttattgtgatatgggataacctaggcatactgcactgtacactctgacatatgaagtgctctagtcaagtttaactggtgtccacagaggacatggtttaactggaattcgtcaagcctctggttctaatttctcatttgcaggggacgctacttacggcaaactgacactgaaatttatttgcactaccggcaaactgcccgtaccgtggcccacactggtgacaacattgacatacggagtgcagtgcttcgccagatatcccgatcacatgaaacagcacgatttctttaagagcgccatgcctgagggttacgtgcaagagcgaacaattttcttcaaagacgatggcaattacaaaactcgagcagaagtgaagtttgaaggggacaccctggtgaaccgcatcgagctgaagggcatcgacttcaaggaggacggcaacatcctggggcacaagctggagtacaactacaacagccacaaggtctatatcaccgccgacaagcagaagaacggcatcaaggtgaacttcaagacccgccacaacatcgaggacggcagcgtgcagctcgccgaccactaccagcagaacacccccatcggcgacggccccgtgctgctgcccgacaaccactacctgagcacccagtccgccctgagcaaagaccccaacgagaagcgcgatcacatggtcctgctggagttcgtgaccgccgccgggatcactctcggcatggacgagctgtacaagtaagtatgatttaaagctcgctttcttgctgtccaatttctattaaaggttcctttgttccctaagtccaactactaaactgggggatattatgaagggccttgagcatctggattctgcctaataaaaaacatttattttcattgcaatgatgtatttaaattatttctgaatattttactaaaaagggaatgtgggaggtcagtgcatttaaaacataaagaaatgaagagctagttcaaaccttgggaaaatacactatatcttaaactccatgaaagaaggtgaggctgcaaacagctaatgcacattggcaacagcccctgatgcctatgccttattcatccctcagaaaaggattcaagtagaggcttgatttggaggttaaagttttgctatgctgtattttacgatatcgatatctataacaagaaaatatatatataataagttatcacgtaagtagaacatgaaataacaatataattatcgtatgagttaaatcttaaaagtcacgtaaaagataatcatgcgtcattttgactcacgcggtcgttatagttcaaaatcagtgacacttaccgcattgacaagcacgcctcacgggagctccaagcggcgactgagatgtcctaaatgcacagcgacggattcgcgctatttagaaagagagagcaatatttcaagaatgacgcgtggattctcgagtaggttggtaccttttttggccggcttgtcgacgacggcggtctccgtcgtcaggatcatccgggccaccgccaccatggccaagcctttgtctcaagaagaatccaccctcattgaaagagcaacggctacaatcaacagcatccccatctctgaagactacagcgtcgccagcgcagctctctctagcgacggccgcatcttcactggtgtcaatgtatatcattttactgggggaccttgtgcagaactcgtggtgctgggcactgctgctgctgcggcagctggcaacctgacttgtatcgtcgcgatcggaaatgagaacaggggcatcttgagcccctgcggacggtgccgacaggtgcttctcgatctgcatcctgggatcaaagccatagtgaaggacagtgatggacagccgacggcagttgggattcgtgaattgctgccctctggttatgtgtgggagggctaagtttaaacccgctgatcagcctcgactgtgccttctagttgccagccatctgttgtttgcccctcccccgtgccttccttgaccctggaaggtgccactcccactgtcctttcctaataaaatgaggaaattgcatcgcattgtctgagtaggtgtcattctattctggggggtggggtggggcaggacagcaagggggaggattgggaagacaatagcaggcatgctggggatgcggtgggctctatggcttcatcggatgccgggaccgacgagtgcagaggcgtgcaaataacttcgtatagcatacattatacgaagttatgcgagcttggcgtaatcatggtcatagctgtttcctgtgtgaaattgttatccgctcacaattccacacaacatacgagccggaagcataaagtgtaaagcctggggtgcctaatgagtgagctaactcacattaattgcgttgcgctcactgcccgctttccagtcgggaaacctgtcgtgccagctgcattaatgaatcggccaacgcgcggggagaggcggtttgcgtattgggcgctcttccgcttcctcgctcactgactcgctgcgctcggtcgttcggctgcggcgagcggtatcagctcactcaaaggcggtaatacggttatccacagaatcaggggataacgcaggaaagaacatgtgagcaaaaggccagcaaaaggccaggaaccgtaaaaaggccgcgttgctggcgtttttccataggctccgcccccctgacgagcatcacaaaaatcgacgctcaagtcagaggtggcgaaacccgacaggactataaagataccaggcgtttccccctggaagctccctcgtgcgctctcctgttccgaccctgccgcttaccggatacctgtccgcctttctcccttcgggaagcgtggcgctttctcatagctcacgctgtaggtatctcagttcggtgtaggtcgttcgctccaagctgggctgtgtgcacgaaccccccgttcagcccgaccgctgcgccttatccggtaactatcgtcttgagtccaacccggtaagacacgacttatcgccactggcagcagccactggtaacaggattagcagagcgaggtatgtaggcggtgctacagagttcttgaagtggtggcctaactacggctacactagaagaacagtatttggtatctgcgctctgctgaagccagttaccttcggaaaaagagttggtagctcttgatccggcaaacaaaccaccgctggtagcggtggtttttttgtttgcaagcagcagattacgcgcagaaaaaaaggatctcaagaagatcctttgatcttttctacggggtctgacgctcagtggaacgaaaactcacgttaagggattttggtcatgagattatcaaaaaggatcttcacctagatccttttaaattaaaaatgaagttttaaatcaatctaaagtatatatgagtaaacttggtctgacagttaccaatgcttaatcagtgaggcacctatctcagcgatctgtctatttcgttcatccatagttgcctgactccccgtcgtgtagataactacgatacgggagggcttaccatctggccccagtgctgcaatgataccgcgagacccacgctcaccggctccagatttatcagcaataaaccagccagccggaagggccgagcgcagaagtggtcctgcaactttatccgcctccatccagtctattaattgttgccgggaagctagagtaagtagttcgccagttaatagtttgcgcaacgttgttgccattgctacaggcatcgtggtgtcacgctcgtcgtttggtatggcttcattcagctccggttcccaacgatcaaggcgagttacatgatcccccatgttgtgcaaaaaagcggttagctccttcggtcctccgatcgttgtcagaagtaagttggccgcagtgttatcactcatggttatggcagcactgcataattctcttactgtcatgccatccgtaagatgcttttctgtgactggtgagtactcaaccaagtcattctgagaatagtgtatgcggcgaccgagttgctcttgcccggcgtcaatacgggataataccgcgccacatagcagaactttaaaagtgctcatcattggaaaacgttcttcggggcgaaaactctcaaggatcttaccgctgttgagatccagttcgatgtaacccactcgtgcacccaactgatcttcagcatcttttactttcaccagcgtttctgggtgagcaaaaacaggaaggcaaaatgccgcaaaaaagggaataagggcgacacggaaatgttgaatactcatactcttcctttttcaatattattgaagcatttatcagggttattgtctcatgagcggatacatatttgaatgtatttagaaaaataaacaaataggggttccgcgcacatttccccgaaaagtgccacctgacgtctaagaaaccattattatcatgacattaacctataaaaataggcgtatcacgaggccctttcgtc

SEQ ID NO: 17 - DNA, 8606 bp, synthetic construct
  source 1..8606: mol_type = other DNA
ctgcagaacacgcagctagcggccgcattaaccctagaaagataatcatattgtgacgtacgttaaagataatcatgcgtaaaattgacgcatgtgttttatcggtctgtatatcgaggtttatttattaatttgaatagatattaagttttattatatttacacttacatactaataataaattcaacaaacaatttatttatgtttatttatttattaaaaaaaaacaaaaactcaaaatttcttctataaagtaacaaaacttttatgagggacagcccccccccaaagcccccagggatgtaattacgtccctcccccgctagggggcagcagcgagccgcccggggctccgctccggtccggcgctccccccgcatccccgagccggcagcgtgcggggacagcccgggcacggggaaggtggcacgggatcgctttcctctgaacgcttctcgctgctctttgagcctgcagacacctggggggatacggggaaaaggcctccacggccagactagtaatgtgtgtcagttagggtgtggaaagtccccaggctccccagcaggcagaagtatgcaaagcatgcatctcaattagtcagcaaccaggtgtggaaagtccccaggctccccagcaggcagaagtatgcaaagcatgcatctcaattagtcagcaaccatagtcccgcccctaactccgcccatcccgcccctaactccgcccagttccgcccattctccgccccatggctgactaattttttttatttatgcagaggccgaggccgcctctgcctctgagctattccagaagtagtgaggaggcttttttggaggcctaggcttttgcaaaaagctcccgggagcttgtatatccattttcggatctgatcagcacgtgttgacaattaatcatcggcatagtatatcggcatagtataatacgacaaggtgaggaatcgccaccatggttagtaagggcgaggaattgattaaggagaacatgcatatgaagctgtacatggaaggcactgtggataaccaccactttaaatgcaccagtgaaggcgaaggcaagccatatgagggaacacagactatgcggattaaagtggtggagggtggcccattgccattcgcttttgacattctcgctaccagttttctttatgggtccaagaccttcataaatcatactcaggggatcccagacttcttcaaacaatcttttccggaagggttcacctgggagcgggtgacaacttacgaggatgggggcgtgctgaccgcaactcaggataccagcctccaggacggatgcttgatctataacgttaagatccgcggcgtgaattttacctcaaatgggccggtgatgcagaaaaagaccctgggatgggaggctttcactgaaacgctctaccccgctgatggcggcctggagggcagaaatgatatggccctgaagctggtgggagggagccaccttatagctaacgccaagaccacttaccgctccaaaaagccagcaaagaatctcaagatgcccggggtgtactacgttgattaccgcctggagaggatcaaggaagccaataacgagacctacgtcgagcagcacgaggtggccgttgcccggtactgcgatcttccaagtaaacttggccataagctgaatggttccggtgagggcagaggaagtcttctaacatgcggtgacgtggaggagaatcccggccctggttccggtatgaccgagtacaagcccacggtgcgcctcgccacccgcgacgacgtccccagggccgtacgcaccctcgccgccgcgttcgccgactaccccgccacgcgccacaccgtcgatccggaccgccacatcgagcgggtcaccgagctgcaagaactcttcctcacgcgcgtcgggctcgacatcggcaaggtgtgggtcgcggacgacggcgccgcggtggcggtctggaccacgccggagagcgtcgaagcgggggcggtgttcgccgagatcggcccgcgcatggccgagttgagcggttcccggctggccgcgcagcaacagatggaaggcctcctggcgccgcaccggcccaaggagcccgcgtggttcctggccaccgtcggcgtctcgcccgaccaccagggcaagggtctgggcagcgccgtcgtgctccccggagtggaggcggccgagcgcgccggggtgcccgccttcctggagacctccgcgccccgcaacctccccttctacgagcggctcggcttcaccgtcaccgccgacgtcgaggtgcccgaaggaccgcgcacctggtgcatgacccgcaagcccggtgcctgacgacaccccaacttgtttattgcagcttataatggttacaaataaagcaatagcatcacaaatttcacaaataaagcatttttttcactgcattctagttgtggtttgtccaaactcatcaatgtatcttatcatgtctgggcgagctcacggggacagcccccccccaaagcccccagggatgtaattacgtccctcccccgctagggggcagcagcgagccgcccggggctccgctccggtccggcgctccccccgcatccccgagccggcagcgtgcggggacagcccgggcacggggaaggtggcacgggatcgctttcctctgaacgcttctcgctgctctttgagcctgcagacacctggggggatacggggaaaaagctttaggctgaaagagagatttagaatgacagaatcatagaacggcctgggttgcaaaggagcacagtgctcatccagatccaaccccctgctatgtgcagggtcatcaaccagcagcccaggctgcccagagccacatccagcctggccttgaatgcctgcagggatggggcatccacagcctccttgggcaacctgttcagtgcgtcaccaccctctgggggaaaaactgcctcctcatatccaacccaaacctcccctgtctcagtgtaaagccattcccccttgtcctatcaagggggagtttgctgtgacattgttggtctggggtgacacatgtttgccaattcagtgcatcacggagaggcagatcttggggataaggaagtgcaggacagcatggacgtgggacatgcaggtgttgagggctctgggacactctccaagtcacagcgttcagaacagccttaaggataagaagataggatagaaggacaaagagcaagttaaaacccagcatggagaggagcacaaaaaggccacagacactgctggtccctgtgtctgagcctgcatgtttgatggtgtctggatgcaagcagaaggggtggaagagcttgcctggagagatacagctgggtcagtaggactgggacaggcagctggagaattgccatgtagatgttcatacaatcgtcaaatcatgaaggctggaaaagccctccaagatccccaagaccaaccccaacccacccaccgtgcccactggccatgtccctcagtgccacatccccacagttcttcatcacctccagggacggtgacccccccacctccgtgggcagctgtgccactgcagcaccgctctttggagaaggtaaatcttgctaaatccagcccgaccctcccctggcacaacgtaaggccattatctctcatccaactccaggacggagtcagtgagaatattgcgctcttgaaaggagtgggaattcgttacataacttacggtaaatggcccgcctggctgaccgcccaacgacccccgcccattgacgtcaataatgacgtatgttcccatagtaacgccaatagggactttccattgacgtcaatgggtggagtatttacggtaaactgcccacttggcagtacatcaagtgtatcatatgccaagtacgccccctattgacgtcaatgacggtaaatggcccgcctggcattatgcccagtacatgaccttatgggactttcctacttggcagtacatctacgtattagtcatcgctattaccatggtcgaggtgagccccacgttctgcttcactctccccatctcccccccctccccacccccaattttgtatttatttattttttaattattttgtgcagcgatgggggcggggggggggggggggcgcgcgccaggcggggcggggcggggcgaggggcggggcggggcgaggcggagaggtgcggcggcagccaatcagagcggcgcgctccgaaagtttccttttatggcgaggcggcggcggcggcggccctataaaaagcgaagcgcgcggcgggcgggagtcgctgcgcgctgccttcgccccgtgccccgctccgccgccgcctcgcgccgcccgccccggctctgactgaccgcgttactcccacaggtgagcgggcgggacggcccttctcctccgggctgtaattagcgcttggtttaatgacggcttgtttcttttctgtggctgcgtgaaagccttgaggggctccgggagggccctttgtgcggggggagcggctcggggggtgcgtgcgtgtgtgtgtgcgtggggagcgccgcgtgcggctccgcgctgcccggcggctgtgagcgctgcgggcgcggcgcggggctttgtgcgctccgcagtgtgcgcgaggggagcgcggccgggggcggtgccccgcggtgcggggggggctgcgaggggaacaaaggctgcgtgcggggtgtgtgcgtgggggggtgagcagggggtgtgggcgcgtcggtcgggctgcaaccccccctgcacccccctccccgagttgctgagcacggcccggcttcgggtgcggggctccgtacggggcgtggcgcggggctcgccgtgccgggcggggggtggcggcaggtgggggtgccgggcggggcggggccgcctcgggccggggagggctcgggggaggggcgcggcggcccccggagcgccggcggctgtcgaggcgcggcgagccgcagccattgccttttatggtaatcgtgcgagagggcgcagggacttcctttgtcccaaatctgtgcggagccgaaatctgggaggcgccgccgcaccccctctagcgggcgcggggcgaagcggtgcggcgccggcaggaaggaaatgggcggggagggccttcgtgcgtcgccgcgccgccgtccccttctccctctccagcctcggggctgtccgcggggggacggctgccttcgggggggacggggcagggcggggttcggcttctggcgtgtgaccggcggctctagagcctctgctaaccatgttcatgccttcttctttttcctacagctcctgggcaacgtgctggttattgtgctgtctcatcattttggcaaagaattgatttgataccgcgggcgccaccatggtgtctaagggcgaagagctctttactggcgtggtgcccatcctggttgaattggacggagatgttaacggacacaaatttagcgtatctggagagggcgaaggtaagtaatcggttcaagtgattctcctgcctcagcctcccaagtagctgggattagaggtccccaccaccatgcctggctaattttttgtactttcagtagaaatggggttttgccatgttggccaggctgttctcgaactcctgagctcaggtgatccaactgtctcggcctcccaaagtgctgggattacaggcgtgagccactgtgcctagcctgagccaccacgccggcctaatttttaaattttttgtagagacagggtctcattatgttgcccagggtggtgtcaagctccaggtctcaagtgatccccctacctccgcctcccaaagttgtgggattgtaggcatgagccactgcaagaaaaccttaactgcagcctaataattgttttctttgggataacttttaaagtacattaaaagactatcaacttaatttctgatcatattttgttgaataaaataagtaaaatgtcttgtgaaacaaaatgctttttaacatccatataaagctatctatatatagctatctatgtctacccatgcgtcaattttacgcagactatctttctagggttaatcggcgcgccttaatctagctgcatcaggatcatatcgtcgggtcttttttccggctcagtcatcgcccaagctggcgctatctgggcatcggggaggaagaagcccgtgccttttcccgcgaggttgaagcggcatggaaagagtttgccgaggatgactgctgctgcattgacgttgagcgaaaacgcacgtttaccatgatgattcgggaaggtgtggccatgcacgcctttaacggtgaactgttcgttcaggccacctgggataccagttcgtcgcggcttttccggacacagttccggatggtcagcccgaagcgcatcagcaacccgaacaataccggcgacagccggaactgccgtgccggtgtgcagattaatgacagcggtgcggcgctgggatattacgtcagcgaggacgggtatcctggctggatgccgcagaaatggacatggataccccgtgagttacccggcgggcgcgcttggcgtaatcatggtcatagctgtttcctgtgtgaaattgttatccgctcacaattccacacaacatacgagccggaagcataaagtgtaaagcctggggtgcctaatgagtgagctaactcacattaattgcgttgcgctcactgcccgctttccagtcgggaaacctgtcgtgccagctgcattaatgaatcggccaacgcgcggggagaggcggtttgcgtattgggcgctcttccgcttcctcgctcactgactcgctgcgctcggtcgttcggctgcggcgagcggtatcagctcactcaaaggcggtaatacggttatccacagaatcaggggataacgcaggaaagaacatgtgagcaaaaggccagcaaaaggccaggaaccgtaaaaaggccgcgttgctggcgtttttccataggctccgcccccctgacgagcatcacaaaaatcgacgctcaagtcagaggtggcgaaacccgacaggactataaagataccaggcgtttccccctggaagctccctcgtgcgctctcctgttccgaccctgccgcttaccggatacctgtccgcctttctcccttcgggaagcgtggcgctttctcatagctcacgctgtaggtatctcagttcggtgtaggtcgttcgctccaagctgggctgtgtgcacgaaccccccgttcagcccgaccgctgcgccttatccggtaactatcgtcttgagtccaacccggtaagacacgacttatcgccactggcagcagccactggtaacaggattagcagagcgaggtatgtaggcggtgctacagagttcttgaagtggtggcctaactacggctacactagaagaacagtatttggtatctgcgctctgctgaagccagttaccttcggaaaaagagttggtagctcttgatccggcaaacaaaccaccgctggtagcggtggtttttttgtttgcaagcagcagattacgcgcagaaaaaaaggatctcaagaagatcctttgatcttttctacggggtctgacgctcagtggaacgaaaactcacgttaagggattttggtcatgagtgcgcggaacccctatttgtttatttttctaaatacattcaaatatgtatccgctcatgagacaataaccctgataaatgcttcaataatattgaaaaaggaagagtatgagggaagcggtgatcgccgaagtatcgactcaactatcagaggtagttggcgtcatcgagcgccatctcgaaccgacgttgctggccgtacatttgtacggctccgcagtggatggcggcctgaagccacacagtgatattgatttgctggttacggtgaccgtaaggcttgatgaaacaacgcggcgagctttgatcaacgaccttttggaaacttcggcttcccctggagagagcgagattctccgcgctgtagaagtcaccattgttgtgcacgacgacatcattccgtggcgttatccagctaagcgcgaactgcaatttggagaatggcagcgcaatgacattcttgcaggtatcttcgagccagccacgatcgacattgatctggctatcttgctgacaaaagcaagagaacatagcgttgccttggtaggtccagcggcggaggaactctttgatccggttcctgaacaggatctatttgaggcgctaaatgaaaccttaacgctatggaactcgccgcccgactgggctggcgatgagcgaaatgtagtgcttacgttgtcccgcatttggtacagcgcagtaaccggcaaaatcgcgccgaaggatgtcgctgccgactgggcaatggagcgcctgccggcccagtatcagcccgtcatacttgaagctagacaggcttatcttggacaagaagaagatcgcttggcctcgcgcgcagatcagttggaagaatttgtccactacgtgaaaggcgagatcaccaaggtagtcggcaaataaccctcgagccacccatgaccaaaatcccttaacgtgagtta

SEQ ID NO: 18 - DNA, 11803 bp, synthetic construct
  source 1..11803: mol_type = other DNA
gtgatgcggttttggcagtacatcaatgggcgtggatagcggtttgactcacggggatttccaagtctccaccccattgacgtcaatgggagtttgttttggcaccaaaatcaacgggactttccaaaatgtcgtaacaactccgccccattgacgcaaatgggcggtaggcgtgtacggtgggaggtctatataagcagagctcgtttagtgaaccgtcagatcgcctggagacgccatccacgctgttttgacctccatagaagacaccgggaccgatccagcctccggactctagaggatcgaacccttgccaccatggacaagaagtactccattgggctcgacatcggcacaaacagcgtcggctgggccgtcattacggacgagtacaaggtgccgagcaaaaaattcaaagttctgggcaataccgatcgccacagcataaagaagaacctcattggcgccctcctgttcgactccggggagacggccgaagccacgcggctcaaaagaacagcacggcgcagatatacccgcagaaagaatcggatctgctacctgcaggagatctttagtaatgagatggctaaggtggatgactctttcttccataggctggaggagtcctttttggtggaggaggataaaaagcacgagcgccacccaatctttggcaatatcgtggacgaggtggcgtaccatgaaaagtacccaaccatatatcatctgaggaagaagcttgtagacagtactgataaggctgacttgcggttgatctatctcgcgctggcgcatatgatcaaatttcggggacacttcctcatcgagggggacctgaacccagacaacagcgatgtcgacaaactctttatccaactggttcagacttacaatcagcttttcgaagagaacccgatcaacgcatccggagttgacgccaaagcaatcctgagcgctaggctgtccaaatcccggcggctcgaaaacctcatcgcacagctccctggggagaagaagaacggcctgtttggtaatcttatcgccctgtcactcgggctgacccccaactttaaatctaacttcgacctggccgaagatgccaagcttcaactgagcaaagacacctacgatgatgatctcgacaatctgctggcccagatcggcgaccagtacgcagacctttttttggcggcaaagaacctgtcagacgccattctgctgagtgatattctgcgagtgaacacggagatcaccaaagctccgctgagcgctagtatgatcaagcgctatgatgagcaccaccaagacttgactttgctgaaggcccttgtcagacagcaactgcctgagaagtacaaggaaattttcttcgatcagtctaaaaatggctacgccggatacattgacggcggagcaagccaggaggaattttacaaatttattaagcccatcttggaaaaaatggacggcaccgaggagctgctggtaaagcttaacagagaagatctgttgcgcaaacagcgcactttcgacaatggaagcatcccccaccagattcacctgggcgaactgcacgctatcctcaggcggcaagaggatttctacccctttttgaaagataacagggaaaagattgagaaaatcctcacatttcggataccctactatgtaggccccctcgcccggggaaattccagattcgcgtggatgactcgcaaatcagaagagaccatcactccctggaacttcgaggaagtcgtggataagggggcctctgcccagtccttcatcgaaaggatgactaactttgataaaaatctgcctaacgaaaaggtgcttcctaaacactctctgctgtacgagtacttcacagtttataacgagctcaccaaggtcaaatacgtcacagaagggatgagaaagccagcattcctgtctggagagcagaagaaagctatcgtggacctcctcttcaagacgaaccggaaagttaccgtgaaacagctcaaagaagactatttcaaaaagattgaatgtttcgactctgttgaaatcagcggagtggaggatcgcttcaacgcatccctgggaacgtatcacgatctcctgaaaatcattaaagacaaggacttcctggacaatgaggagaacgaggacattcttgaggacattgtcctcacccttacgttgtttgaagatagggagatgattgaagaacgcttgaaaacttacgctcatctcttcgacgacaaagtcatgaaacagctcaagaggcgccgatatacaggatgggggcggctgtcaagaaaactgatcaatgggatccgagacaagcagagtggaaagacaatcctggattttcttaagtccgatggatttgccaacaggaacttcatgcagttgatccatgatgactctctcacctttaaggaggacatccagaaagcacaagtttctggccagggggacagtcttcacgagcacatcgctaatcttgcaggtagcccagctatcaaaaagggaatactgcagaccgttaaggtcgtggatgaactcgtcaaagtaatgggaaggcataagcccgagaatatcgttatcgagatggcccgagagaaccaaactacccagaagggacagaagaacagtagggaaaggatgaagaggattgaagagggtataaaagaactggggtcccaaatccttaaggaacacccagttgaaaacacccagcttcagaatgagaagctctacctgtactacctgcagaacggcagggacatgtacgtggatcaggaactggacatcaatcggctctccgactacgacgtggatcatatcgtgccccagtcttttctcaaagatgattctattgataataaagtgttgacaagatccgataaaaatagagggaagagtgataacgtcccctcagaagaagttgtcaagaaaatgaaaaattattggcggcagctgctgaacgccaaactgatcacacaacggaagttcgataatctgactaaggctgaacgaggtggcctgtctgagttggataaagccggcttcatcaaaaggcagcttgttgagacacgccagatcaccaagcacgtggcccaaattctcgattcacgcatgaacaccaagtacgatgaaaatgacaaactgattcgagaggtgaaagttattactctgaagtctaagctggtctcagatttcagaaaggactttcagttttataaggtgagagagatcaacaattaccaccatgcgcatgatgcctacctgaatgcagtggtaggcactgcacttatcaaaaaatatcccaagcttgaatctgaatttgtttacggagactataaagtgtacgatgttaggaaaatgatcgcaaagtctgagcaggaaataggcaaggccaccgctaagtacttcttttacagcaatattatgaattttttcaagaccgagattacactggccaatggagagattcggaagcgaccacttatcgaaacaaacggagaaacaggagaaatcgtgtgggacaagggtagggatttcgcgacagtccggaaggtcctgtccatgccgcaggtgaacatcgttaaaaagaccgaagtacagaccggaggcttctccaaggaaagtatcctcccgaaaaggaacagcgacaagctgatcgcacgcaaaaaagattgggaccccaagaaatacggcggattcgattctcctacagtcgcttacagtgtactggttgtggccaaagtggagaaagggaagtctaaaaaactcaaaagcgtcaaggaactgctgggcatcacaatcatggagcgatcaagcttcgaaaaaaaccccatcgactttctcgaggcgaaaggatataaagaggtcaaaaaagacctcatcattaagcttcccaagtactctctctttgagcttgaaaacggccggaaacgaatgctcgctagtgcgggcgagctgcagaaaggtaacgagctggcactgccctctaaatacgttaatttcttgtatctggccagccactatgaaaagctcaaagggtctcccgaagataatgagcagaagcagctgttcgtggaacaacacaaacactaccttgatgagatcatcgagcaaataagcgaattctccaaaagagtgatcctcgccgacgctaacctcgataaggtgctttctgcttacaataagcacagggataagcccatcagggagcaggcagaaaacattatccacttgtttactctgaccaacttgggcgcgcctgcagccttcaagtacttcgacaccaccatagacagaaagcggtacacctctacaaaggaggtcctggacgccacactgattcatcagtcaattacggggctctatgaaacaagaatcgacctctctcagctcggtggagacagcagggctgaccccaagaagaagaggaaggtgggcggaggagggagtggcggaggcggaagcggcggcggaggcagcggctctagcctggacgacgagcacatcctgagcgccctgctgcagagcgacgacgaactggtgggcgaggacagcgacagcgaggtcagcgaccacgtgtccgaggacgacgtgcagtccgacaccgaggaagccttcatcgacgaggtgcacgaagtgcagcctaccagcagcggctccgagatcctggacgagcagaacgtgatcgagcagcctggcagctccctggccagcaacagaatcctgaccctgccccagagaaccatcagaggcaagaacaagcactgctggtccacctccaagagcaccaggcggagcagagtgtccgccctgaacatcgtgcggagccagaggggccccaccagaatgtgcagaaacatctacgaccccctgctgtgcttcaagctgttcttcaccgacgagatcatcagcgagatcgtgaagtggaccaacgccgagatcagcctgaagaggcgggagagcatgaccagcgccaccttcagagacaccaacgaggacgagatctacgccttcttcggcatcctggtgatgaccgccgtgagaaaggacaaccacatgagcaccgacgacctgttcgacagatccctgagcatggtgtacgtgtccgtgatgagcagagacagattcgacttcctgatcagatgcctgagaatggacgacaagagcatcagacccaccctgcgggagaacgacgtgttcacccccgtgcggaagatctgggacctgttcatccaccagtgcatccagaactacacccctggcgcccacctgaccatcgatgagcagctgctgggcttcagaggcagatgccccttcagagtgtacatccccaacaagcccagcaagtacggcatcaagatcctgatgatgtgcgacagcggcaccaagtacatgatcaacggcatgccctacctgggcagaggcacccagacaaacggcgtgcccctgggcgagtactacgtgaaagaactgagcaagcctgtgcatggcagctgcaggaacatcacctgcgacgcctggttcaccagcatccccctggccaagaacctgctgcaggaaccctacaagctgaccatcgtgggcaccgtgcggagcaacaaggaggagatcccagaggtgctgaagaacagcagatccagacctgtgggaacaagcatgttctgcttcgacggccccctgaccctggtgtcctacaagcccaagcccgccaagatggtgtacctgctgtccagctgcgacgaggacgccagcatcaacgagagcaccggcaagccccagatggtgatgtactacaaccagaccaagggcggcgtggacaccctgaaccagatgtgcagcgtgatgacctgcagcagaaagaccaacagatggcccatggccctgctgtacggcatgatcaatatcgcctgcatcaacagcttcatcatctacagccacaacgtgtccagcaagggcgagaaggtgcagagccggaagaaattcatgcggaacctgtacatgagcctgacctccagcttcatgagaaagagactggaagcccccaccctgaagagatacctgcgggacaacatcagcaacatcctgcccaaggaagtgccaggaacaagcgacgacagcaccgaggaacccgtgatgaagaagaggacctactgcacctactgtcccagcaagatcagaagaaaggccaacgccagctgcaagaaatgcaaaaaagtgatctgccgggagcacaacatcgacatgtgccagagctgtttctgaaagggttcgatccctaccggttagtaatgagtttaaacgggggaggctaactgaaacacggaaggagacaataccggaaggaacccgcgctatgacggcaataaaaagacagaataaaacgcacgggtgttgggtcgtttgttcataaacgcggggttcggtcccagggctggcactctgtcgataccccaccgagaccccattggggccaatacgcccgcgtttcttccttttccccaccccaccccccaagttcgggtgaaggcccagggctcgcagccaacgtcggggcggcaggccctgccatagcagatctgcgcagctggggctctagggggtatccccacgcgccctgtagcggcgcattaagcgcggcgggtgtggtggttacgcgcagcgtgaccgctacacttgccagcgccctagcgcccgctcctttcgctttcttcccttcctttctcgccacgttcgccggctttccccgtcaagctctaaatcgggggctccctttagggttccgatttagtgctttacggcacctcgaccccaaaaaacttgattagggtgatggttcacgtagtgggccatcgccctgatagacggtttttcgccctttgacgttggagtccacgttctttaatagtggactcttgttccaaactggaacaacactcaaccctatctcggtctattcttttgatttataagggattttgccgatttcggcctattggttaaaaaatgagctgatttaacaaaaatttaacgcgaattaattctgtggaatgtgtgtcagttagggtgtggaaagtccccaggctccccagcaggcagaagtatgcaaagcatgcatctcaattagtcagcaaccaggtgtggaaagtccccaggctccccagcaggcagaagtatgcaaagcatgcatctcaattagtcagcaaccatagtcccgcccctaactccgcccatcccgcccctaactccgcccagttccgcccattctccgccccatggctgactaattttttttatttatgcagaggccgaggccgcctctgcctctgagctattccagaagtagtgaggaggcttttttggaggcctaggcttttgcaaaaagctcccgggagcttgtatatccattttcggatctgatcaagagacaggatgaggatcgtttcgcatgattgaacaagatggattgcacgcaggttctccggccgcttgggtggagaggctattcggctatgactgggcacaacagacaatcggctgctctgatgccgccgtgttccggctgtcagcgcaggggcgcccggttctttttgtcaagaccgacctgtccggtgccctgaatgaactgcaggacgaggcagcgcggctatcgtggctggccacgacgggcgttccttgcgcagctgtgctcgacgttgtcactgaagcgggaagggactggctgctattgggcgaagtgccggggcaggatctcctgtcatctcaccttgctcctgccgagaaagtatccatcatggctgatgcaatgcggcggctgcatacgcttgatccggctacctgcccattcgaccaccaagcgaaacatcgcatcgagcgagcacgtactcggatggaagccggtcttgtcgatcaggatgatctggacgaagagcatcaggggctcgcgccagccgaactgttcgccaggctcaaggcgcgcatgcccgacggcgaggatctcgtcgtgacccatggcgatgcctgcttgccgaatatcatggtggaaaatggccgcttttctggattcatcgactgtggccggctgggtgtggcggaccgctatcaggacatagcgttggctacccgtgatattgctgaagagcttggcggcgaatgggctgaccgcttcctcgtgctttacggtatcgccgctcccgattcgcagcgcatcgccttctatcgccttcttgacgagttcttctgagcgggactctggggttcgcgaaatgaccgaccaagcgacgcccaacctgccatcacgagatttcgattccaccgccgccttctatgaaaggttgggcttcggaatcgttttccgggacgccggctggatgatcctccagcgcggggatctcatgctggagttcttcgcccaccccaacttgtttattgcagcttataatggttacaaataaagcaatagcatcacaaatttcacaaataaagcatttttttcactgcattctagttgtggtttgtccaaactcatcaatgtatcttatcatgtctgtataccgtcgacctctagctagagcttggcgtaatcatggtcatagctgtttcctgtgtgaaattgttatccgctcacaattccacacaacatacgagccggaagcataaagtgtaaagcctggggtgcctaatgagtgagctaactcacattaattgcgttgcgctcactgcccgctttccagtcgggaaacctgtcgtgccagctgcattaatgaatcggccaacgcgcggggagaggcggtttgcgtattgggcgctcttccgcttcctcgctcactgactcgctgcgctcggtcgttcggctgcggcgagcggtatcagctcactcaaaggcggtaatacggttatccacagaatcaggggataacgcaggaaagaacatgtgagcaaaaggccagcaaaaggccaggaaccgtaaaaaggccgcgttgctggcgtttttccataggctccgcccccctgacgagcatcacaaaaatcgacgctcaagtcagaggtggcgaaacccgacaggactataaagataccaggcgtttccccctggaagctccctcgtgcgctctcctgttccgaccctgccgcttaccggatacctgtccgcctttctcccttcgggaagcgtggcgctttctcatagctcacgctgtaggtatctcagttcggtgtaggtcgttcgctccaagctgggctgtgtgcacgaaccccccgttcagcccgaccgctgcgccttatccggtaactatcgtcttgagtccaacccggtaagacacgacttatcgccactggcagcagccactggtaacaggattagcagagcgaggtatgtaggcggtgctacagagttcttgaagtggtggcctaactacggctacactagaagaacagtatttggtatctgcgctctgctgaagccagttaccttcggaaaaagagttggtagctcttgatccggcaaacaaaccaccgctggtagcggtggtttttttgtttgcaagcagcagattacgcgcagaaaaaaaggatctcaagaagatcctttgatcttttctacggggtctgacgctcagtggaacgaaaactcacgttaagggattttggtcatgagattatcaaaaaggatcttcacctagatccttttaaattaaaaatgaagttttaaatcaatctaaagtatatatgagtaaacttggtctgacagttaccaatgcttaatcagtgaggcacctatctcagcgatctgtctatttcgttcatccatagttgcctgactccccgtcgtgtagataactacgatacgggagggcttaccatctggccccagtgctgcaatgataccgcgagacccacgctcaccggctccagatttatcagcaataaaccagccagccggaagggccgagcgcagaagtggtcctgcaactttatccgcctccatccagtctattaattgttgccgggaagctagagtaagtagttcgccagttaatagtttgcgcaacgttgttgccattgctacaggcatcgtggtgtcacgctcgtcgtttggtatggcttcattcagctccggttcccaacgatcaaggcgagttacatgatcccccatgttgtgcaaaaaagcggttagctccttcggtcctccgatcgttgtcagaagtaagttggccgcagtgttatcactcatggttatggcagcactgcataattctcttactgtcatgccatccgtaagatgcttttctgtgactggtgagtactcaaccaagtcattctgagaatagtgtatgcggcgaccgagttgctcttgcccggcgtcaatacgggataataccgcgccacatagcagaactttaaaagtgctcatcattggaaaacgttcttcggggcgaaaactctcaaggatcttaccgctgttgagatccagttcgatgtaacccactcgtgcacccaactgatcttcagcatcttttactttcaccagcgtttctgggtgagcaaaaacaggaaggcaaaatgccgcaaaaaagggaataagggcgacacggaaatgttgaatactcatactcttcctttttcaatattattgaagcatttatcagggttattgtctcatgagcggatacatatttgaatgtatttagaaaaataaacaaataggggttccgcgcacatttccccgaaaagtgccacctgacgtcgacggatcgggagatctcccgatcccctatggtgcactctcagtacaatctgctctgatgccgcatagttaagccagtatctgctccctgcttgtgtgttggaggtcgctgagtagtgcgcgagcaaaatttaagctacaacaaggcaaggcttgaccgacaattgcatgaagaatctgcttagggttaggcgttttgcgctgcttcgcgatgtacgggccagagggcctatttcccatgattccttcatatttgcatatacgatacaaggctgttagagagataattggaattaatttgactgtaaacacaaagatattagtacaaaatacgtgacgtagaaagtaataatttcttgggtagtttgcagttttaaaattatgttttaaaatggactatcatatgcttaccgtaacttgaaagtatttcgatttcttggctttatatatcttgtggaaaggacgaaacaccgtcgagtcgcttctcgattagttttagagctagaaatagcaagttaaaataaggctagtccgttatcaacttgaaaaagtggcaccgagtcggtgcttttttgttttagagctagaaatagcaagttaaaataaggctagtccgtttttagcgcgtgcgccaattctgcagacaaatgatatacgcgttgacattgattattgactagttattaatagtaatcaattacggggtcattagttcatagcccatatatggagttccgcgttacataacttacggtaaatggcccgcctggctgaccgcccaacgacccccgcccattgacgtcaataatgacgtatgttcccatagtaacgccaatagggactttccattgacgtcaatgggtggagtatttacggtaaactgcccacttggcagtacatcaagtgtatcatatgccaagtacgccccctattgacgtcaatgacggtaaatggcccgcctggcattatgcccagtacatgaccttatgggactttcctacttggcagtacatctacgtattagtcatcgctattaccatg

SEQ ID NO: 19 - DNA, 11803 bp, synthetic construct
  source 1..11803: mol_type = other DNA
gtgatgcggttttggcagtacatcaatgggcgtggatagcggtttgactcacggggatttccaagtctccaccccattgacgtcaatgggagtttgttttggcaccaaaatcaacgggactttccaaaatgtcgtaacaactccgccccattgacgcaaatgggcggtaggcgtgtacggtgggaggtctatataagcagagctcgtttagtgaaccgtcagatcgcctggagacgccatccacgctgttttgacctccatagaagacaccgggaccgatccagcctccggactctagaggatcgaacccttgccaccatggacaagaagtactccattgggctcgacatcggcacaaacagcgtcggctgggccgtcattacggacgagtacaaggtgccgagcaaaaaattcaaagttctgggcaataccgatcgccacagcataaagaagaacctcattggcgccctcctgttcgactccggggagacggccgaagccacgcggctcaaaagaacagcacggcgcagatatacccgcagaaagaatcggatctgctacctgcaggagatctttagtaatgagatggctaaggtggatgactctttcttccataggctggaggagtcctttttggtggaggaggataaaaagcacgagcgccacccaatctttggcaatatcgtggacgaggtggcgtaccatgaaaagtacccaaccatatatcatctgaggaagaagcttgtagacagtactgataaggctgacttgcggttgatctatctcgcgctggcgcatatgatcaaatttcggggacacttcctcatcgagggggacctgaacccagacaacagcgatgtcgacaaactctttatccaactggttcagacttacaatcagcttttcgaagagaacccgatcaacgcatccggagttgacgccaaagcaatcctgagcgctaggctgtccaaatcccggcggctcgaaaacctcatcgcacagctccctggggagaagaagaacggcctgtttggtaatcttatcgccctgtcactcgggctgacccccaactttaaatctaacttcgacctggccgaagatgccaagcttcaactgagcaaagacacctacgatgatgatctcgacaatctgctggcccagatcggcgaccagtacgcagacctttttttggcggcaaagaacctgtcagacgccattctgctgagtgatattctgcgagtgaacacggagatcaccaaagctccgctgagcgctagtatgatcaagcgctatgatgagcaccaccaagacttgactttgctgaaggcccttgtcagacagcaactgcctgagaagtacaaggaaattttcttcgatcagtctaaaaatggctacgccggatacattgacggcggagcaagccaggaggaattttacaaatttattaagcccatcttggaaaaaatggacggcaccgaggagctgctggtaaagcttaacagagaagatctgttgcgcaaacagcgcactttcgacaatggaagcatcccccaccagattcacctgggcgaactgcacgctatcctcaggcggcaagaggatttctacccctttttgaaagataacagggaaaagattgagaaaatcctcacatttcggataccctactatgtaggccccctcgcccggggaaattccagattcgcgtggatgactcgcaaatcagaagagaccatcactccctggaacttcgaggaagtcgtggataagggggcctctgcccagtccttcatcgaaaggatgactaactttgataaaaatctgcctaacgaaaaggtgcttcctaaacactctctgctgtacgagtacttcacagtttataacgagctcaccaaggtcaaatacgtcacagaagggatgagaaagccagcattcctgtctggagagcagaagaaagctatcgtggacctcctcttcaagacgaaccggaaagttaccgtgaaacagctcaaagaagactatttcaaaaagattgaatgtttcgactctgttgaaatcagcggagtggaggatcgcttcaacgcatccctgggaacgtatcacgatctcctgaaaatcattaaagacaaggacttcctggacaatgaggagaacgaggacattcttgaggacattgtcctcacccttacgttgtttgaagatagggagatgattgaagaacgcttgaaaacttacgctcatctcttcgacgacaaagtcatgaaacagctcaagaggcgccgatatacaggatgggggcggctgtcaagaaaactgatcaatgggatccgagacaagcagagtggaaagacaatcctggattttcttaagtccgatggatttgccaacaggaacttcatgcagttgatccatgatgactctctcacctttaaggaggacatccagaaagcacaagtttctggccagggggacagtcttcacgagcacatcgctaatcttgcaggtagcccagctatcaaaaagggaatactgcagaccgttaaggtcgtggatgaactcgtcaaagtaatgggaaggcataagcccgagaatatcgttatcgagatggcccgagagaaccaaactacccagaagggacagaagaacagtagggaaaggatgaagaggattgaagagggtataaaagaactggggtcccaaatccttaaggaacacccagttgaaaacacccagcttcagaatgagaagctctacctgtactacctgcagaacggcagggacatgtacgtggatcaggaactggacatcaatcggctctccgactacgacgtggatcatatcgtgccccagtcttttctcaaagatgattctattgataataaagtgttgacaagatccgataaaaatagagggaagagtgataacgtcccctcagaagaagttgtcaagaaaatgaaaaattattggcggcagctgctgaacgccaaactgatcacacaacggaagttcgataatctgactaaggctgaacgaggtggcctgtctgagttggataaagccggcttcatcaaaaggcagcttgttgagacacgccagatcaccaagcacgtggcccaaattctcgattcacgcatgaacaccaagtacgatgaaaatgacaaactgattcgagaggtgaaagttattactctgaagtctaagctggtctcagatttcagaaaggactttcagttttataaggtgagagagatcaacaattaccaccatgcgcatgatgcctacctgaatgcagtggtaggcactgcacttatcaaaaaatatcccaagcttgaatctgaatttgtttacggagactataaagtgtacgatgttaggaaaatgatcgcaaagtctgagcaggaaataggcaaggccaccgctaagtacttcttttacagcaatattatgaattttttcaagaccgagattacactggccaatggagagattcggaagcgaccacttatcgaaacaaacggagaaacaggagaaatcgtgtgggacaagggtagggatttcgcgacagtccggaaggtcctgtccatgccgcaggtgaacatcgttaaaaagaccgaagtacagaccggaggcttctccaaggaaagtatcctcccgaaaaggaacagcgacaagctgatcgcacgcaaaaaagattgggaccccaagaaatacggcggattcgattctcctacagtcgcttacagtgtactggttgtggccaaagtggagaaagggaagtctaaaaaactcaaaagcgtcaaggaactgctgggcatcacaatcatggagcgatcaagcttcgaaaaaaaccccatcgactttctcgaggcgaaaggatataaagaggtcaaaaaagacctcatcattaagcttcccaagtactctctctttgagcttgaaaacggccggaaacgaatgctcgctagtgcgggcgagctgcagaaaggtaacgagctggcactgccctctaaatacgttaatttcttgtatctggccagccactatgaaaagctcaaagggtctcccgaagataatgagcagaagcagctgttcgtggaacaacacaaacactaccttgatgagatcatcgagcaaataagcgaattctccaaaagagtgatcctcgccgacgctaacctcgataaggtgctttctgcttacaataagcacagggataagcccatcagggagcaggcagaaaacattatccacttgtttactctgaccaacttgggcgcgcctgcagccttcaagtacttcgacaccaccatagacagaaagcggtacacctctacaaaggaggtcctggacgccacactgattcatcagtcaattacggggctctatgaaacaagaatcgacctctctcagctcggtggagacagcagggctgaccccaagaagaagaggaaggtgggcggaggagggagtggcggaggcggaagcggcggcggaggcagcggctctagcctggacgacgagcacatcctgagcgccctgctgcagagcgacgacgaactggtgggcgaggacagcgacagcgaggtcagcgaccacgtgtccgaggacgacgtgcagtccgacaccgaggaagccttcatcgacgaggtgcacgaagtgcagcctaccagcagcggctccgagatcctggacgagcagaacgtgatcgagcagcctggcagctccctggccagcaacagaatcctgaccctgccccagagaaccatcagaggcaagaacaagcactgctggtccacctccaagagcaccaggcggagcagagtgtccgccctgaacatcgtgcggagccagaggggccccaccagaatgtgcagaaacatctacgaccccctgctgtgcttcaagctgttcttcaccgacgagatcatcagcgagatcgtgaagtggaccaacgccgagatcagcctgaagaggcgggagagcatgaccagcgccaccttcagagacaccaacgaggacgagatctacgccttcttcggcatcctggtgatgaccgccgtgagaaaggacaaccacatgagcaccgacgacctgttcgacagatccctgagcatggtgtacgtgtccgtgatgagcagagacagattcgacttcctgatcagatgcctgagaatggacgacaagagcatcagacccaccctgcgggagaacgacgtgttcacccccgtgcggaagatctgggacctgttcatccaccagtgcatccagaactacacccctggcgcccacctgaccatcgatgagcagctgctgggcttcagaggcagatgccccttcagagtgtacatccccaacaagcccagcaagtacggcatcaagatcctgatgatgtgcgacagcggcaccaagtacatgatcaacggcatgccctacctgggcagaggcacccagacaaacggcgtgcccctgggcgagtactacgtgaaagaactgagcaagcctgtgcatggcagctgcaggaacatcacctgcgacgcctggttcaccagcatccccctggccaagaacctgctgcaggaaccctacaagctgaccatcgtgggcaccgtgcggagcaacaaggaggagatcccagaggtgctgaagaacagcagatccagacctgtgggaacaagcatgttctgcttcgacggccccctgaccctggtgtcctacaagcccaagcccgccaagatggtgtacctgctgtccagctgcgacgaggacgccagcatcaacgagagcaccggcaagccccagatggtgatgtactacaaccagaccaagggcggcgtggacaccctgaaccagatgtgcagcgtgatgacctgcagcagaaagaccaacagatggcccatggccctgctgtacggcatgatcaatatcgcctgcatcaacagcttcatcatctacagccacaacgtgtccagcaagggcgagaaggtgcagagccggaagaaattcatgcggaacctgtacatgagcctgacctccagcttcatgagaaagagactggaagcccccaccctgaagagatacctgcgggacaacatcagcaacatcctgcccaaggaagtgccaggaacaagcgacgacagcaccgaggaacccgtgatgaagaagaggacctactgcacctactgtcccagcaagatcagaagaaaggccaacgccagctgcaagaaatgcaaaaaagtgatctgccgggagcacaacatcgacatgtgccagagctgtttctgaaagggttcgatccctaccggttagtaatgagtttaaacgggggaggctaactgaaacacggaaggagacaataccggaaggaacccgcgctatgacggcaataaaaagacagaataaaacgcacgggtgttgggtcgtttgttcataaacgcggggttcggtcccagggctggcactctgtcgataccccaccgagaccccattggggccaatacgcccgcgtttcttccttttccccaccccaccccccaagttcgggtgaaggcccagggctcgcagccaacgtcggggcggcaggccctgccatagcagatctgcgcagctggggctctagggggtatccccacgcgccctgtagcggcgcattaagcgcggcgggtgtggtggttacgcgcagcgtgaccgctacacttgccagcgccctagcgcccgctcctttcgctttcttcccttcctttctcgccacgttcgccggctttccccgtcaagctctaaatcgggggctccctttagggttccgatttagtgctttacggcacctcgaccccaaaaaacttgattagggtgatggttcacgtagtgggccatcgccctgatagacggtttttcgccctttgacgttggagtccacgttctttaatagtggactcttgttccaaactggaacaacactcaaccctatctcggtctattcttttgatttataagggattttgccgatttcggcctattggttaaaaaatgagctgatttaacaaaaatttaacgcgaattaattctgtggaatgtgtgtcagttagggtgtggaaagtccccaggctccccagcaggcagaagtatgcaaagcatgcatctcaattagtcagcaaccaggtgtggaaagtccccaggctccccagcaggcagaagtatgcaaagcatgcatctcaattagtcagcaaccatagtcccgcccctaactccgcccatcccgcccctaactccgcccagttccgcccattctccgccccatggctgactaattttttttatttatgcagaggccgaggccgcctctgcctctgagctattccagaagtagtgaggaggcttttttggaggcctaggcttttgcaaaaagctcccgggagcttgtatatccattttcggatctgatcaagagacaggatgaggatcgtttcgcatgattgaacaagatggattgcacgcaggttctccggccgcttgggtggagaggctattcggctatgactgggcacaacagacaatcggctgctctgatgccgccgtgttccggctgtcagcgcaggggcgcccggttctttttgtcaagaccgacctgtccggtgccctgaatgaactgcaggacgaggcagcgcggctatcgtggctggccacgacgggcgttccttgcgcagctgtgctcgacgttgtcactgaagcgggaagggactggctgctattgggcgaagtgccggggcaggatctcctgtcatctcaccttgctcctgccgagaaagtatccatcatggctgatgcaatgcggcggctgcatacgcttgatccggctacctgcccattcgaccaccaagcgaaacatcgcatcgagcgagcacgtactcggatggaagccggtcttgtcgatcaggatgatctggacgaagagcatcaggggctcgcgccagccgaactgttcgccaggctcaaggcgcgcatgcccgacggcgaggatctcgtcgtgacccatggcgatgcctgcttgccgaatatcatggtggaaaatggccgcttttctggattcatcgactgtggccggctgggtgtggcggaccgctatcaggacatagcgttggctacccgtgatattgctgaagagcttggcggcgaatgggctgaccgcttcctcgtgctttacggtatcgccgctcccgattcgcagcgcatcgccttctatcgccttcttgacgagttcttctgagcgggactctggggttcgcgaaatgaccgaccaagcgacgcccaacctgccatcacgagatttcgattccaccgccgccttctatgaaaggttgggcttcggaatcgttttccgggacgccggctggatgatcctccagcgcggggatctcatgctggagttcttcgcccaccccaacttgtttattgcagcttataatggttacaaataaagcaatagcatcacaaatttcacaaataaagcatttttttcactgcattctagttgtggtttgtccaaactcatcaatgtatcttatcatgtctgtataccgtcgacctctagctagagcttggcgtaatcatggtcatagctgtttcctgtgtgaaattgttatccgctcacaattccacacaacatacgagccggaagcataaagtgtaaagcctggggtgcctaatgagtgagctaactcacattaattgcgttgcgctcactgcccgctttccagtcgggaaacctgtcgtgccagctgcattaatgaatcggccaacgcgcggggagaggcggtttgcgtattgggcgctcttccgcttcctcgctcactgactcgctgcgctcggtcgttcggctgcggcgagcggtatcagctcactcaaaggcggtaatacggttatccacagaatcaggggataacgcaggaaagaacatgtgagcaaaaggccagcaaaaggccaggaaccgtaaaaaggccgcgttgctggcgtttttccataggctccgcccccctgacgagcatcacaaaaatcgacgctcaagtcagaggtggcgaaacccgacaggactataaagataccaggcgtttccccctggaagctccctcgtgcgctctcctgttccgaccctgccgcttaccggatacctgtccgcctttctcccttcgggaagcgtggcgctttctcatagctcacgctgtaggtatctcagttcggtgtaggtcgttcgctccaagctgggctgtgtgcacgaaccccccgttcagcccgaccgctgcgccttatccggtaactatcgtcttgagtccaacccggtaagacacgacttatcgccactggcagcagccactggtaacaggattagcagagcgaggtatgtaggcggtgctacagagttcttgaagtggtggcctaactacggctacactagaagaacagtatttggtatctgcgctctgctgaagccagttaccttcggaaaaagagttggtagctcttgatccggcaaacaaaccaccgctggtagcggtggtttttttgtttgcaagcagcagattacgcgcagaaaaaaaggatctcaagaagatcctttgatcttttctacggggtctgacgctcagtggaacgaaaactcacgttaagggattttggtcatgagattatcaaaaaggatcttcacctagatccttttaaattaaaaatgaagttttaaatcaatctaaagtatatatgagtaaacttggtctgacagttaccaatgcttaatcagtgaggcacctatctcagcgatctgtctatttcgttcatccatagttgcctgactccccgtcgtgtagataactacgatacgggagggcttaccatctggccccagtgctgcaatgataccgcgagacccacgctcaccggctccagatttatcagcaataaaccagccagccggaagggccgagcgcagaagtggtcctgcaactttatccgcctccatccagtctattaattgttgccgggaagctagagtaagtagttcgccagttaatagtttgcgcaacgttgttgccattgctacaggcatcgtggtgtcacgctcgtcgtttggtatggcttcattcagctccggttcccaacgatcaaggcgagttacatgatcccccatgttgtgcaaaaaagcggttagctccttcggtcctccgatcgttgtcagaagtaagttggccgcagtgttatcactcatggttatggcagcactgcataattctcttactgtcatgccatccgtaagatgcttttctgtgactggtgagtactcaaccaagtcattctgagaatagtgtatgcggcgaccgagttgctcttgcccggcgtcaatacgggataataccgcgccacatagcagaactttaaaagtgctcatcattggaaaacgttcttcggggcgaaaactctcaaggatcttaccgctgttgagatccagttcgatgtaacccactcgtgcacccaactgatcttcagcatcttttactttcaccagcgtttctgggtgagcaaaaacaggaaggcaaaatgccgcaaaaaagggaataagggcgacacggaaatgttgaatactcatactcttcctttttcaatattattgaagcatttatcagggttattgtctcatgagcggatacatatttgaatgtatttagaaaaataaacaaataggggttccgcgcacatttccccgaaaagtgccacctgacgtcgacggatcgggagatctcccgatcccctatggtgcactctcagtacaatctgctctgatgccgcatagttaagccagtatctgctccctgcttgtgtgttggaggtcgctgagtagtgcgcgagcaaaatttaagctacaacaaggcaaggcttgaccgacaattgcatgaagaatctgcttagggttaggcgttttgcgctgcttcgcgatgtacgggccagagggcctatttcccatgattccttcatatttgcatatacgatacaaggctgttagagagataattggaattaatttgactgtaaacacaaagatattagtacaaaatacgtgacgtagaaagtaataatttcttgggtagtttgcagttttaaaattatgttttaaaatggactatcatatgcttaccgtaacttgaaagtatttcgatttcttggctttatatatcttgtggaaaggacgaaacaccttagtcctagtgccatgaaggttttagagctagaaatagcaagttaaaataaggctagtccgttatcaacttgaaaaagtggcaccgagtcggtgcttttttgttttagagctagaaatagcaagttaaaataaggctagtccgtttttagcgcgtgcgccaattctgcagacaaatgatatacgcgttgacattgattattgactagttattaatagtaatcaattacggggtcattagttcatagcccatatatggagttccgcgttacataacttacggtaaatggcccgcctggctgaccgcccaacgacccccgcccattgacgtcaataatgacgtatgttcccatagtaacgccaatagggactttccattgacgtcaatgggtggagtatttacggtaaactgcccacttggcagtacatcaagtgtatcatatgccaagtacgccccctattgacgtcaatgacggtaaatggcccgcctggcattatgcccagtacatgaccttatgggactttcctacttggcagtacatctacgtattagtcatcgctattaccatg

SEQ ID NO: 20 - DNA, 11803 bp, synthetic construct
  source 1..11803: mol_type = other DNA
gtgatgcggttttggcagtacatcaatgggcgtggatagcggtttgactcacggggatttccaagtctccaccccattgacgtcaatgggagtttgttttggcaccaaaatcaacgggactttccaaaatgtcgtaacaactccgccccattgacgcaaatgggcggtaggcgtgtacggtgggaggtctatataagcagagctcgtttagtgaaccgtcagatcgcctggagacgccatccacgctgttttgacctccatagaagacaccgggaccgatccagcctccggactctagaggatcgaacccttgccaccatggacaagaagtactccattgggctcgacatcggcacaaacagcgtcggctgggccgtcattacggacgagtacaaggtgccgagcaaaaaattcaaagttctgggcaataccgatcgccacagcataaagaagaacctcattggcgccctcctgttcgactccggggagacggccgaagccacgcggctcaaaagaacagcacggcgcagatatacccgcagaaagaatcggatctgctacctgcaggagatctttagtaatgagatggctaaggtggatgactctttcttccataggctggaggagtcctttttggtggaggaggataaaaagcacgagcgccacccaatctttggcaatatcgtggacgaggtggcgtaccatgaaaagtacccaaccatatatcatctgaggaagaagcttgtagacagtactgataaggctgacttgcggttgatctatctcgcgctggcgcatatgatcaaatttcggggacacttcctcatcgagggggacctgaacccagacaacagcgatgtcgacaaactctttatccaactggttcagacttacaatcagcttttcgaagagaacccgatcaacgcatccggagttgacgccaaagcaatcctgagcgctaggctgtccaaatcccggcggctcgaaaacctcatcgcacagctccctggggagaagaagaacggcctgtttggtaatcttatcgccctgtcactcgggctgacccccaactttaaatctaacttcgacctggccgaagatgccaagcttcaactgagcaaagacacctacgatgatgatctcgacaatctgctggcccagatcggcgaccagtacgcagacctttttttggcggcaaagaacctgtcagacgccattctgctgagtgatattctgcgagtgaacacggagatcaccaaagctccgctgagcgctagtatgatcaagcgctatgatgagcaccaccaagacttgactttgctgaaggcccttgtcagacagcaactgcctgagaagtacaaggaaattttcttcgatcagtctaaaaatggctacgccggatacattgacggcggagcaagccaggaggaattttacaaatttattaagcccatcttggaaaaaatggacggcaccgaggagctgctggtaaagcttaacagagaagatctgttgcgcaaacagcgcactttcgacaatggaagcatcccccaccagattcacctgggcgaactgcacgctatcctcaggcggcaagaggatttctacccctttttgaaagataacagggaaaagattgagaaaatcctcacatttcggataccctactatgtaggccccctcgcccggggaaattccagattcgcgtggatgactcgcaaatcagaagagaccatcactccctggaacttcgaggaagtcgtggataagggggcctctgcccagtccttcatcgaaaggatgactaactttgataaaaatctgcctaacgaaaaggtgcttcctaaacactctctgctgtacgagtacttcacagtttataacgagctcaccaaggtcaaatacgtcacagaagggatgagaaagccagcattcctgtctggagagcagaagaaagctatcgtggacctcctcttcaagacgaaccggaaagttaccgtgaaacagctcaaagaagactatttcaaaaagattgaatgtttcgactctgttgaaatcagcggagtggaggatcgcttcaacgcatccctgggaacgtatcacgatctcctgaaaatcattaaagacaaggacttcctggacaatgaggagaacgaggacattcttgaggacattgtcctcacccttacgttgtttgaagatagggagatgattgaagaacgcttgaaaacttacgctcatctcttcgacgacaaagtcatgaaacagctcaagaggcgccgatatacaggatgggggcggctgtcaagaaaactgatcaatgggatccgagacaagcagagtggaaagacaatcctggattttcttaagtccgatggatttgccaacaggaacttcatgcagttgatccatgatgactctctcacctttaaggaggacatccagaaagcacaagtttctggccagggggacagtcttcacgagcacatcgctaatcttgcaggtagcccagctatcaaaaagggaatactgcagaccgttaaggtcgtggatgaactcgtcaaagtaatgggaaggcataagcccgagaatatcgttatcgagatggcccgagagaaccaaactacccagaagggacagaagaacagtagggaaaggatgaagaggattgaagagggtataaaagaactggggtcccaaatccttaaggaacacccagttgaaaacacccagcttcagaatgagaagctctacctgtactacctgcagaacggcagggacatgtacgtggatcaggaactggacatcaatcggctctccgactacgacgtggatcatatcgtgccccagtcttttctcaaagatgattctattgataataaagtgttgacaagatccgataaaaatagagggaagagtgataacgtcccctcagaagaagttgtcaagaaaatgaaaaattattggcggcagctgctgaacgccaaactgatcacacaacggaagttcgataatctgactaaggctgaacgaggtggcctgtctgagttggataaagccggcttcatcaaaaggcagcttgttgagacacgccagatcaccaagcacgtggcccaaattctcgattcacgcatgaacaccaagtacgatgaaaatgacaaactgattcgagaggtgaaagttattactctgaagtctaagctggtctcagatttcagaaaggactttcagttttataaggtgagagagatcaacaattaccaccatgcgcatgatgcctacctgaatgcagtggtaggcactgcacttatcaaaaaatatcccaagcttgaatctgaatttgtttacggagactataaagtgtacgatgttaggaaaatgatcgcaaagtctgagcaggaaataggcaaggccaccgctaagtacttcttttacagcaatattatgaattttttcaagaccgagattacactggccaatggagagattcggaagcgaccacttatcgaaacaaacggagaaacaggagaaatcgtgtgggacaagggtagggatttcgcgacagtccggaaggtcctgtccatgccgcaggtgaacatcgttaaaaagaccgaagtacagaccggaggcttctccaaggaaagtatcctcccgaaaaggaacagcgacaagctgatcgcacgcaaaaaagattgggaccccaagaaatacggcggattcgattctcctacagtcgcttacagtgtactggttgtggccaaagtggagaaagggaagtctaaaaaactcaaaagcgtcaaggaactgctgggcatcacaatcatggagcgatcaagcttcgaaaaaaaccccatcgactttctcgaggcgaaaggatataaagaggtcaaaaaagacctcatcattaagcttcccaagtactctctctttgagcttgaaaacggccggaaacgaatgctcgctagtgcgggcgagctgcagaaaggtaacgagctggcactgccctctaaatacgttaatttcttgtatctggccagccactatgaaaagctcaaagggtctcccgaagataatgagcagaagcagctgttcgtggaacaacacaaacactaccttgatgagatcatcgagcaaataagcgaattctccaaaagagtgatcctcgccgacgctaacctcgataaggtgctttctgcttacaataagcacagggataagcccatcagggagcaggcagaaaacattatccacttgtttactctgaccaacttgggcgcgcctgcagccttcaagtacttcgacaccaccatagacagaaagcggtacacctctacaaaggaggtcctggacgccacactgattcatcagtcaattacggggctctatgaaacaagaatcgacctctctcagctcggtggagacagcagggctgaccccaagaagaagaggaaggtgggcggaggagggagtggcggaggcggaagcggcggcggaggcagcggctctagcctggacgacgagcacatcctgagcgccctgctgcagagcgacgacgaactggtgggcgaggacagcgacagcgaggtcagcgaccacgtgtccgaggacgacgtgcagtccgacaccgaggaagccttcatcgacgaggtgcacgaagtgcagcctaccagcagcggctccgagatcctggacgagcagaacgtgatcgagcagcctggcagctccctggccagcaacagaatcctgaccctgccccagagaaccatcagaggcaagaacaagcactgctggtccacctccaagagcaccaggcggagcagagtgtccgccctgaacatcgtgcggagccagaggggccccaccagaatgtgcagaaacatctacgaccccctgctgtgcttcaagctgttcttcaccgacgagatcatcagcgagatcgtgaagtggaccaacgccgagatcagcctgaagaggcgggagagcatgaccagcgccaccttcagagacaccaacgaggacgagatctacgccttcttcggcatcctggtgatgaccgccgtgagaaaggacaaccacatgagcaccgacgacctgttcgacagatccctgagcatggtgtacgtgtccgtgatgagcagagacagattcgacttcctgatcagatgcctgagaatggacgacaagagcatcagacccaccctgcgggagaacgacgtgttcacccccgtgcggaagatctgggacctgttcatccaccagtgcatccagaactacacccctggcgcccacctgaccatcgatgagcagctgctgggcttcagaggcagatgccccttcagagtgtacatccccaacaagcccagcaagtacggcatcaagatcctgatgatgtgcgacagcggcaccaagtacatgatcaacggcatgccctacctgggcagaggcacccagacaaacggcgtgcccctgggcgagtactacgtgaaagaactgagcaagcctgtgcatggcagctgcaggaacatcacctgcgacgcctggttcaccagcatccccctggccaagaacctgctgcaggaaccctacaagctgaccatcgtgggcaccgtgcggagcaacaaggaggagatcccagaggtgctgaagaacagcagatccagacctgtgggaacaagcatgttctgcttcgacggccccctgaccctggtgtcctacaagcccaagcccgccaagatggtgtacctgctgtccagctgcgacgaggacgccagcatcaacgagagcaccggcaagccccagatggtgatgtactacaaccagaccaagggcggcgtggacaccctgaaccagatgtgcagcgtgatgacctgcagcagaaagaccaacagatggcccatggccctgctgtacggcatgatcaatatcgcctgcatcaacagcttcatcatctacagccacaacgtgtccagcaagggcgagaaggtgcagagccggaagaaattcatgcggaacctgtacatgagcctgacctccagcttcatgagaaagagactggaagcccccaccctgaagagatacctgcgggacaacatcagcaacatcctgcccaaggaagtgccaggaacaagcgacgacagcaccgaggaacccgtgatgaagaagaggacctactgcacctactgtcccagcaagatcagaagaaaggccaacgccagctgcaagaaatgcaaaaaagtgatctgccgggagcacaacatcgacatgtgccagagctgtttctgaaagggttcgatccctaccggttagtaatgagtttaaacgggggaggctaactgaaacacggaaggagacaataccggaaggaacccgcgctatgacggcaataaaaagacagaataaaacgcacgggtgttgggtcgtttgttcataaacgcggggttcggtcccagggctggcactctgtcgataccccaccgagaccccattggggccaatacgcccgcgtttcttccttttccccaccccaccccccaagttcgggtgaaggcccagggctcgcagccaacgtcggggcggcaggccctgccatagcagatctgcgcagctggggctctagggggtatccccacgcgccctgtagcggcgcattaagcgcggcgggtgtggtggttacgcgcagcgtgaccgctacacttgccagcgccctagcgcccgctcctttcgctttcttcccttcctttctcgccacgttcgccggctttccccgtcaagctctaaatcgggggctccctttagggttccgatttagtgctttacggcacctcgaccccaaaaaacttgattagggtgatggttcacgtagtgggccatcgccctgatagacggtttttcgccctttgacgttggagtccacgttctttaatagtggactcttgttccaaactggaacaacactcaaccctatctcggtctattcttttgatttataagggattttgccgatttcggcctattggttaaaaaatgagctgatttaacaaaaatttaacgcgaattaattctgtggaatgtgtgtcagttagggtgtggaaagtccccaggctccccagcaggcagaagtatgcaaagcatgcatctcaattagtcagcaaccaggtgtggaaagtccccaggctccccagcaggcagaagtatgcaaagcatgcatctcaattagtcagcaaccatagtcccgcccctaactccgcccatcccgcccctaactccgcccagttccgcccattctccgccccatggctgactaattttttttatttatgcagaggccgaggccgcctctgcctctgagctattccagaagtagtgaggaggcttttttggaggcctaggcttttgcaaaaagctcccgggagcttgtatatccattttcggatctgatcaagagacaggatgaggatcgtttcgcatgattgaacaagatggattgcacgcaggttctccggccgcttgggtggagaggctattcggctatgactgggcacaacagacaatcggctgctctgatgccgccgtgttccggctgtcagcgcaggggcgcccggttctttttgtcaagaccgacctgtccggtgccctgaatgaactgcaggacgaggcagcgcggctatcgtggctggccacgacgggcgttccttgcgcagctgtgctcgacgttgtcactgaagcgggaagggactggctgctattgggcgaagtgccggggcaggatctcctgtcatctcaccttgctcctgccgagaaagtatccatcatggctgatgcaatgcggcggctgcatacgcttgatccggctacctgcccattcgaccaccaagcgaaacatcgcatcgagcgagcacgtactcggatggaagccggtcttgtcgatcaggatgatctggacgaagagcatcaggggctcgcgccagccgaactgttcgccaggctcaaggcgcgcatgcccgacggcgaggatctcgtcgtgacccatggcgatgcctgcttgccgaatatcatggtggaaaatggccgcttttctggattcatcgactgtggccggctgggtgtggcggaccgctatcaggacatagcgttggctacccgtgatattgctgaagagcttggcggcgaatgggctgaccgcttcctcgtgctttacggtatcgccgctcccgattcgcagcgcatcgccttctatcgccttcttgacgagttcttctgagcgggactctggggttcgcgaaatgaccgaccaagcgacgcccaacctgccatcacgagatttcgattccaccgccgccttctatgaaaggttgggcttcggaatcgttttccgggacgccggctggatgatcctccagcgcggggatctcatgctggagttcttcgcccaccccaacttgtttattgcagcttataatggttacaaataaagcaatagcatcacaaatttcacaaataaagcatttttttcactgcattctagttgtggtttgtccaaactcatcaatgtatcttatcatgtctgtataccgtcgacctctagctagagcttggcgtaatcatggtcatagctgtttcctgtgtgaaattgttatccgctcacaattccacacaacatacgagccggaagcataaagtgtaaagcctggggtgcctaatgagtgagctaactcacattaattgcgttgcgctcactgcccgctttccagtcgggaaacctgtcgtgccagctgcattaatgaatcggccaacgcgcggggagaggcggtttgcgtattgggcgctcttccgcttcctcgctcactgactcgctgcgctcggtcgttcggctgcggcgagcggtatcagctcactcaaaggcggtaatacggttatccacagaatcaggggataacgcaggaaagaacatgtgagcaaaaggccagcaaaaggccaggaaccgtaaaaaggccgcgttgctggcgtttttccataggctccgcccccctgacgagcatcacaaaaatcgacgctcaagtcagaggtggcgaaacccgacaggactataaagataccaggcgtttccccctggaagctccctcgtgcgctctcctgttccgaccctgccgcttaccggatacctgtccgcctttctcccttcgggaagcgtggcgctttctcatagctcacgctgtaggtatctcagttcggtgtaggtcgttcgctccaagctgggctgtgtgcacgaaccccccgttcagcccgaccgctgcgccttatccggtaactatcgtcttgagtccaacccggtaagacacgacttatcgccactggcagcagccactggtaacaggattagcagagcgaggtatgtaggcggtgctacagagttcttgaagtggtggcctaactacggctacactagaagaacagtatttggtatctgcgctctgctgaagccagttaccttcggaaaaagagttggtagctcttgatccggcaaacaaaccaccgctggtagcggtggtttttttgtttgcaagcagcagattacgcgcagaaaaaaaggatctcaagaagatcctttgatcttttctacggggtctgacgctcagtggaacgaaaactcacgttaagggattttggtcatgagattatcaaaaaggatcttcacctagatccttttaaattaaaaatgaagttttaaatcaatctaaagtatatatgagtaaacttggtctgacagttaccaatgcttaatcagtgaggcacctatctcagcgatctgtctatttcgttcatccatagttgcctgactccccgtcgtgtagataactacgatacgggagggcttaccatctggccccagtgctgcaatgataccgcgagacccacgctcaccggctccagatttatcagcaataaaccagccagccggaagggccgagcgcagaagtggtcctgcaactttatccgcctccatccagtctattaattgttgccgggaagctagagtaagtagttcgccagttaatagtttgcgcaacgttgttgccattgctacaggcatcgtggtgtcacgctcgtcgtttggtatggcttcattcagctccggttcccaacgatcaaggcgagttacatgatcccccatgttgtgcaaaaaagcggttagctccttcggtcctccgatcgttgtcagaagtaagttggccgcagtgttatcactcatggttatggcagcactgcataattctcttactgtcatgccatccgtaagatgcttttctgtgactggtgagtactcaaccaagtcattctgagaatagtgtatgcggcgaccgagttgctcttgcccggcgtcaatacgggataataccgcgccacatagcagaactttaaaagtgctcatcattggaaaacgttcttcggggcgaaaactctcaaggatcttaccgctgttgagatccagttcgatgtaacccactcgtgcacccaactgatcttcagcatcttttactttcaccagcgtttctgggtgagcaaaaacaggaaggcaaaatgccgcaaaaaagggaataagggcgacacggaaatgttgaatactcatactcttcctttttcaatattattgaagcatttatcagggttattgtctcatgagcggatacatatttgaatgtatttagaaaaataaacaaataggggttccgcgcacatttccccgaaaagtgccacctgacgtcgacggatcgggagatctcccgatcccctatggtgcactctcagtacaatctgctctgatgccgcatagttaagccagtatctgctccctgcttgtgtgttggaggtcgctgagtagtgcgcgagcaaaatttaagctacaacaaggcaaggcttgaccgacaattgcatgaagaatctgcttagggttaggcgttttgcgctgcttcgcgatgtacgggccagagggcctatttcccatgattccttcatatttgcatatacgatacaaggctgttagagagataattggaattaatttgactgtaaacacaaagatattagtacaaaatacgtgacgtagaaagtaataatttcttgggtagtttgcagttttaaaattatgttttaaaatggactatcatatgcttaccgtaacttgaaagtatttcgatttcttggctttatatatcttgtggaaaggacgaaacacccatcagacttgatagcactggttttagagctagaaatagcaagttaaaataaggctagtccgttatcaacttgaaaaagtggcaccgagtcggtgcttttttgttttagagctagaaatagcaagttaaaataaggctagtccgtttttagcgcgtgcgccaattctgcagacaaatgatatacgcgttgacattgattattgactagttattaatagtaatcaattacggggtcattagttcatagcccatatatggagttccgcgttacataacttacggtaaatggcccgcctggctgaccgcccaacgacccccgcccattgacgtcaataatgacgtatgttcccatagtaacgccaatagggactttccattgacgtcaatgggtggagtatttacggtaaactgcccacttggcagtacatcaagtgtatcatatgccaagtacgccccctattgacgtcaatgacggtaaatggcccgcctggcattatgcccagtacatgaccttatgggactttcctacttggcagtacatctacgtattagtcatcgctattaccatg

SEQ ID NO: 21 - DNA, 9909 bp, synthetic construct
  source 1..9909: mol_type = other DNA
ctgcagaacacgcagctagattaaccctagaaagataatcatattgtgacgtacgttaaagataatcatgcgtaaaattgacgcatgtgttttatcggtctgtatatcgaggtttatttattaatttgaatagatattaagttttattatatttacacttacatactaataataaattcaacaaacaatttatttatgtttatttatttattaaaaaaaaacaaaaactcaaaatttcttctataaagtaacaaaacttttatgagggacagcccccccccaaagcccccagggatgtaattacgtccctcccccgctagggggcagcagcgagccgcccggggctccgctccggtccggcgctccccccgcatccccgagccggcagcgtgcggggacagcccgggcacggggaaggtggcacgggatcgctttcctctgaacgcttctcgctgctctttgagcctgcagacacctggggggatacggggaaaaggcctccacggccagactagtataacttcgtatagcatacattatacgaagttataatgtgtgtcagttagggtgtggaaagtccccaggctccccagcaggcagaagtatgcaaagcatgcatctcaattagtcagcaaccaggtgtggaaagtccccaggctccccagcaggcagaagtatgcaaagcatgcatctcaattagtcagcaaccatagtcccgcccctaactccgcccatcccgcccctaactccgcccagttccgcccattctccgccccatggctgactaattttttttatttatgcagaggccgaggccgcctctgcctctgagctattccagaagtagtgaggaggcttttttggaggcctaggcttttgcaaaaagctcccgggagcttgtatatccattttcggatctgatcagcacgtgttgacaattaatcatcggcatagtatatcggcatagtataatacgacaaggtgaggaatcgccaccatgattgaacaagatggattgcacgcaggttctccggccgcttgggtggagaggctattcggctatgactgggcacaacagacaatcggctgctctgatgccgccgtgttccggctgtcagcgcaggggcgcccggttctttttgtcaagaccgacctgtccggtgccctgaatgaactgcaagacgaggcagcgcggctatcgtggctggccacgacgggcgttccttgcgcagctgtgctcgacgttgtcactgaagcgggaagggactggctgctattgggcgaagtgccggggcaggatctcctgtcatctcaccttgctcctgccgagaaagtatccatcatggctgatgcaatgcggcggctgcatacgcttgatccggctacctgcccattcgaccaccaagcgaaacatcgcatcgagcgagcacgtactcggatggaagccggtcttgtcgatcaggatgatctggacgaagagcatcaggggctcgcgccagccgaactgttcgccaggctcaaggcgagcatgcccgacggcgaggatctcgtcgtgacccatggcgatgcctgcttgccgaatatcatggtggaaaatggccgcttttctggattcatcgactgtggccggctgggtgtggcggaccgctatcaggacatagcgttggctacccgtgatattgctgaagagcttggcggcgaatgggctgaccgcttcctcgtgctttacggtatcgccgctcccgattcgcagcgcatcgccttctatcgccttcttgacgagttcttctgacgacaccccaacttgtttattgcagcttataatggttacaaataaagcaatagcatcacaaatttcacaaataaagcatttttttcactgcattctagttgtggtttgtccaaactcatcaatgtatcttatcatgtctgataacttcgtatagcatacattatacgaagttatgcggccgcgagctcacggggacagcccccccccaaagcccccagggatgtaattacgtccctcccccgctagggggcagcagcgagccgcccggggctccgctccggtccggcgctccccccgcatccccgagccggcagcgtgcggggacagcccgggcacggggaaggtggcacgggatcgctttcctctgaacgcttctcgctgctctttgagcctgcagacacctggggggatacggggaaaaagctttaggctgaaagagagatttagaatgacagaatcatagaacggcctgggttgcaaaggagcacagtgctcatccagatccaaccccctgctatgtgcagggtcatcaaccagcagcccaggctgcccagagccacatccagcctggccttgaatgcctgcagggatggggcatccacagcctccttgggcaacctgttcagtgcgtcaccaccctctgggggaaaaactgcctcctcatatccaacccaaacctcccctgtctcagtgtaaagccattcccccttgtcctatcaagggggagtttgctgtgacattgttggtctggggtgacacatgtttgccaattcagtgcatcacggagaggcagatcttggggataaggaagtgcaggacagcatggacgtgggacatgcaggtgttgagggctctgggacactctccaagtcacagcgttcagaacagccttaaggataagaagataggatagaaggacaaagagcaagttaaaacccagcatggagaggagcacaaaaaggccacagacactgctggtccctgtgtctgagcctgcatgtttgatggtgtctggatgcaagcagaaggggtggaagagcttgcctggagagatacagctgggtcagtaggactgggacaggcagctggagaattgccatgtagatgttcatacaatcgtcaaatcatgaaggctggaaaagccctccaagatccccaagaccaaccccaacccacccaccgtgcccactggccatgtccctcagtgccacatccccacagttcttcatcacctccagggacggtgacccccccacctccgtgggcagctgtgccactgcagcaccgctctttggagaaggtaaatcttgctaaatccagcccgaccctcccctggcacaacgtaaggccattatctctcatccaactccaggacggagtcagtgagaatattgcggccgctcttgaaaggagtgggaattggctccggtgcccgtcagtgggcagagcgcacatcgcccacagtccccgagaagttggggggaggggtcggcaattgaaccggtgcctagagaaggtggcgcggggtaaactgggaaagtgatgtcgtgtactggctccgcctttttcccgagggtgggggagaaccgtatataagtgcagtagtcgccgtgaacgttctttttcgcaacgggtttgccgccagaacacaggtaagtgccgtgtgtggttcccgcgggcctggcctctttacgggttatggcccttgcgtgccttgaattacttccacctggctgcagtacgtgattcttgatcccgagcttcgggttggaagtgggtgggagagttcgaggccttgcgcttaaggagccccttcgcctcgtgcttgagttgaggcctggcctgggcgctggggccgccgcgtgcgaatctggtggcaccttcgcgcctgtctcgctgctttcgataagtctctagccatttaaaatttttgatgacctgctgcgacgctttttttctggcaagatagtcttgtaaatgcgggccaagatctgcacactggtatttcggtttttggggccgcgggcggcgacggggcccgtgcgtcccagcgcacatgttcggcgaggcggggcctgcgagcgcggccaccgagaatcggacgggggtagtctcaagctggccggcctgctctggtgcctggcctcgcgccgccgtgtatcgccccgccctgggcggcaaggctggcccggtcggcaccagttgcgtgagcggaaagatggccgcttcccggccctgctgcagggagctcaaaatggaggacgcggcgctcgggagagcgggcgggtgagtcacccacacaaaggaaaagggcctttccgtcctcagccgtcgcttcatgtgactccacggagtaccgggcgccgtccaggcacctcgattagttctcgagcttttggagtacgtcgtctttaggttggggggaggggttttatgcgatggagtttccccacactgagtgggtggagactgaagttaggccagcttggcacttgatgtaattctccttggaatttgccctttttgagtttggatcttggttcattctcaagcctcagacagtggttcaaagtttttttcttccatttcaggtgtcgtgaggaattagctagcttcgaggggctcgcatctctccttcacgcgcccgccgccctacctgaggccgccatccacgccggttgagtcgcgttctgccgcctcccgcctgtggtgcctcctgaactgcgtccgccgtctaggtaagtttaaagctcaggtcgagaccgggcctttgtccggcgctcccttggagcctacctagactcagccggctctccacgctttgcctgaccctgcttgctcaactctacgtctttgtttcgttttctgttctgcgccgttacagatccaagctgtgaccggcgcctacggtaccatggtgagcaagggcgaggagctgttcaccggggtggtgcccatcctggtcgagctggacggcgacgtaaacggccacaagttcagcgtgtccggcgagggcgagggcgatgccacctacggcaagctgaccctgaagttcatctgcaccaccggcaagctgcccgtgccctggcccaccctcgtgaccaccctgacctacggcgtgcagtgcttcagccgctaccccgaccacatgaagcagcacgacttcttcaagtccgccatgcccgaaggctacgtccaggagcgcaccatcttcttcaaggacgacggcaactacaagacccgcgccgaggtgaagttcgagggcgacaccctggtgaaccgcatcgagctgaagggcatcgacttcaaggaggacggcaacatcctggggcacaagctggagtacaactacaacagccacaacgtctatatcatggccgacaagcagaagaacggcatcaaggtgaacttcaagatccgccacaacatcgaggacggcagcgtgcagctcgccgaccactaccagcagaacacccccatcggcgacggccccgtgctgctgcccgacaaccactacctgagcacccagtccgccctgagcaaagaccccaacgagaagcgcgatcacatggtcctgctggagttcgtgaccgccgccgggatcactctcggcatggacgagctgtacaagtaagaattcgtcgactgtacaacgcgtgtttaaacttcgaatctagatacgtacatatgatttaaagctcgctttcttgctgtccaatttctattaaaggttcctttgttccctaagtccaactactaaactgggggatattatgaagggccttgagcatctggattctgcctaataaaaaacatttattttcattgcaatgatgtatttaaattatttctgaatattttactaaaaagggaatgtgggaggtcagtgcatttaaaacataaagaaatgaagagctagttcaaaccttgggaaaatacactatatcttaaactccatgaaagaaggtgaggctgcaaacagctaatgcacattggcaacagcccctgatgcctatgccttattcatccctcagaaaaggattcaagtagaggcttgatttggaggttaaagttttgctatgctgtattttacgatatcgagctcacggggacagcccccccccaaagcccccagggatgtaattacgtccctcccccgctagggggcagcagcgagccgcccggggctccgctccggtccggcgctccccccgcatccccgagccggcagcgtgcggggacagcccgggcacggggaaggtggcacgggatcgctttcctctgaacgcttctcgctgctctttgagcctgcagacacctggggggatacggggaaaaagctttaggctgaaagagagatttagaatgacagaatcatagaacggcctgggttgcaaaggagcacagtgctcatccagatccaaccccctgctatgtgcagggtcatcaaccagcagcccaggctgcccagagccacatccagcctggccttgaatgcctgcagggatggggcatccacagcctccttgggcaacctgttcagtgcgtcaccaccctctgggggaaaaactgcctcctcatatccaacccaaacctcccctgtctcagtgtaaagccattcccccttgtcctatcaagggggagtttgctgtgacattgttggtctggggtgacacatgtttgccaattcagtgcatcacggagaggcagatcttggggataaggaagtgcaggacagcatggacgtgggacatgcaggtgttgagggctctgggacactctccaagtcacagcgttcagaacagccttaaggataagaagataggatagaaggacaaagagcaagttaaaacccagcatggagaggagcacaaaaaggccacagacactgctggtccctgtgtctgagcctgcatgtttgatggtgtctggatgcaagcagaaggggtggaagagcttgcctggagagatacagctgggtcagtaggactgggacaggcagctggagaattgccatgtagatgttcatacaatcgtcaaatcatgaaggctggaaaagccctccaagatccccaagaccaaccccaacccacccaccgtgcccactggccatgtccctcagtgccacatccccacagttcttcatcacctccagggacggtgacccccccacctccgtgggcagctgtgccactgcagcaccgctctttggagaaggtaaatcttgctaaatccagcccgaccctcccctggcacaacgtaaggccattatctctcatccaactccaggacggagtcagtgagaatattgatatctataacaagaaaatatatatataataagttatcacgtaagtagaacatgaaataacaatataattatcgtatgagttaaatcttaaaagtcacgtaaaagataatcatgcgtcattttgactcacgcggtcgttatagttcaaaatcagtgacacttaccgcattgacaagcacgcctcacgggagctccaagcggcgactgagatgtcctaaatgcacagcgacggattcgcgctatttagaaagagagagcaatatttcaagaatgcatgcgtcaattttacgcagactatctttctagggttaatctagctgcatcaggatcatatcgtcgggtcttttttccggctcagtcatcgcccaagctggcgctatctgggcatcggggaggaagaagcccgtgccttttcccgcgaggttgaagcggcatggaaagagtttgccgaggatgactgctgctgcattgacgttgagcgaaaacgcacgtttaccatgatgattcgggaaggtgtggccatgcacgcctttaacggtgaactgttcgttcaggccacctgggataccagttcgtcgcggcttttccggacacagttccggatggtcagcccgaagcgcatcagcaacccgaacaataccggcgacagccggaactgccgtgccggtgtgcagattaatgacagcggtgcggcgctgggatattacgtcagcgaggacgggtatcctggctggatgccgcagaaatggacatggataccccgtgagttacccggcgggcgcgcttggcgtaatcatggtcatagctgtttcctgtgtgaaattgttatccgctcacaattccacacaacatacgagccggaagcataaagtgtaaagcctggggtgcctaatgagtgagctaactcacattaattgcgttgcgctcactgcccgctttccagtcgggaaacctgtcgtgccagctgcattaatgaatcggccaacgcgcggggagaggcggtttgcgtattgggcgctcttccgcttcctcgctcactgactcgctgcgctcggtcgttcggctgcggcgagcggtatcagctcactcaaaggcggtaatacggttatccacagaatcaggggataacgcaggaaagaacatgtgagcaaaaggccagcaaaaggccaggaaccgtaaaaaggccgcgttgctggcgtttttccataggctccgcccccctgacgagcatcacaaaaatcgacgctcaagtcagaggtggcgaaacccgacaggactataaagataccaggcgtttccccctggaagctccctcgtgcgctctcctgttccgaccctgccgcttaccggatacctgtccgcctttctcccttcgggaagcgtggcgctttctcatagctcacgctgtaggtatctcagttcggtgtaggtcgttcgctccaagctgggctgtgtgcacgaaccccccgttcagcccgaccgctgcgccttatccggtaactatcgtcttgagtccaacccggtaagacacgacttatcgccactggcagcagccactggtaacaggattagcagagcgaggtatgtaggcggtgctacagagttcttgaagtggtggcctaactacggctacactagaagaacagtatttggtatctgcgctctgctgaagccagttaccttcggaaaaagagttggtagctcttgatccggcaaacaaaccaccgctggtagcggtggtttttttgtttgcaagcagcagattacgcgcagaaaaaaaggatctcaagaagatcctttgatcttttctacggggtctgacgctcagtggaacgaaaactcacgttaagggattttggtcatgagtgcgcggaacccctatttgtttatttttctaaatacattcaaatatgtatccgctcatgagacaataaccctgataaatgcttcaataatattgaaaaaggaagagtatgagggaagcggtgatcgccgaagtatcgactcaactatcagaggtagttggcgtcatcgagcgccatctcgaaccgacgttgctggccgtacatttgtacggctccgcagtggatggcggcctgaagccacacagtgatattgatttgctggttacggtgaccgtaaggcttgatgaaacaacgcggcgagctttgatcaacgaccttttggaaacttcggcttcccctggagagagcgagattctccgcgctgtagaagtcaccattgttgtgcacgacgacatcattccgtggcgttatccagctaagcgcgaactgcaatttggagaatggcagcgcaatgacattcttgcaggtatcttcgagccagccacgatcgacattgatctggctatcttgctgacaaaagcaagagaacatagcgttgccttggtaggtccagcggcggaggaactctttgatccggttcctgaacaggatctatttgaggcgctaaatgaaaccttaacgctatggaactcgccgcccgactgggctggcgatgagcgaaatgtagtgcttacgttgtcccgcatttggtacagcgcagtaaccggcaaaatcgcgccgaaggatgtcgctgccgactgggcaatggagcgcctgccggcccagtatcagcccgtcatacttgaagctagacaggcttatcttggacaagaagaagatcgcttggcctcgcgcgcagatcagttggaagaatttgtccactacgtgaaaggcgagatcaccaaggtagtcggcaaataaccctcgagccacccatgaccaaaatcccttaacgtgagtta

SEQ ID NO: 22 - DNA, 21 bp, synthetic construct
  source 1..21: mol_type = other DNA
cactaccttgatgagatcatc

SEQ ID NO: 23 - DNA, 20 bp, synthetic construct
  source 1..20: mol_type = other DNA
tgaacaaacgacccaacacc

SEQ ID NO: 24 - DNA, 41 bp, synthetic construct
  source 1..41: mol_type = other DNA
tgtttactctgaccaacttgggcgcgcctgcagccttcaag

SEQ ID NO: 25 - DNA, 51 bp, synthetic construct
  source 1..51: mol_type = other DNA
ttactaaccggtagggatcgaaccctttcagaaacagctctggcacatgtc

SEQ ID NO: 26 - DNA, 28 bp, synthetic construct
  source 1..28: mol_type = other DNA
ccactgtgctggatatctgcagaattcc

SEQ ID NO: 27 - DNA, 22 bp, synthetic construct
  source 1..22: mol_type = other DNA
ctctctggctaactagagaacc

SEQ ID NO: 28 - DNA, 39 bp, synthetic construct
  source 1..39: mol_type = other DNA
aaacttaagcttgccaccatgggctctagcctggacgac

SEQ ID NO: 29 - DNA, 29 bp, synthetic construct
  source 1..29: mol_type = other DNA
actagtggatcctcagaaacagctctggc

SEQ ID NO: 30 - DNA, 35 bp, synthetic construct
  source 1..35: mol_type = other DNA
gagcatgaccagcaagaccttcagagacaccaacg

SEQ ID NO: 31 - DNA, 35 bp, synthetic construct
  source 1..35: mol_type = other DNA
gtctctgaaggtcttgctggtcatgctctcccgcc

SEQ ID NO: 32 - DNA, 36 bp, synthetic construct
  source 1..36: mol_type = other DNA
gtgtacatccccagaaagcccagcaagtacggcatc

SEQ ID NO: 33 - DNA, 35 bp, synthetic construct
  source 1..35: mol_type = other DNA
cttgctgggctttctggggatgtacactctgaagg

SEQ ID NO: 34 - DNA, 36 bp, synthetic construct
  source 1..36: mol_type = other DNA
cccaacaagcccagaaagtacggcatcaagatcctg

SEQ ID NO: 35 - DNA, 36 bp, synthetic construct
  source 1..36: mol_type = other DNA
gatgccgtactttctgggcttgttggggatgtacac

SEQ ID NO: 36 - DNA, 37 bp, synthetic construct
  source 1..37: mol_type = other DNA
gatgtgcgacagcagaaccaagtacatgatcaacggc

SEQ ID NO: 37 - DNA, 37 bp, synthetic construct
  source 1..37: mol_type = other DNA
catgtacttggttctgctgtcgcacatcatcaggatc

SEQ ID NO: 38 - DNA, 37 bp, synthetic construct
  source 1..37: mol_type = other DNA
gatgtactacaacagaaccaagggcggcgtggacacc

SEQ ID NO: 39 - DNA, 36 bp, synthetic construct
  source 1..36: mol_type = other DNA
gccgcccttggttctgttgtagtacatcaccatctg

SEQ ID NO: 40 - DNA, 36 bp, synthetic construct
  source 1..36: mol_type = other DNA
gagaaggtgcagaaccggaagaaattcatgcggaac

SEQ ID NO: 41 - DNA, 35 bp, synthetic construct
  source 1..35: mol_type = other DNA
gaatttcttccggttctgcaccttctcgcccttgc

SEQ ID NO: 42 - DNA, 37 bp, synthetic construct
  source 1..37: mol_type = other DNA
gagaaagagactgagagcccccaccctgaagagatac

SEQ ID NO: 43 - DNA, 37 bp, synthetic construct
  source 1..37: mol_type = other DNA
cagggtgggggctctcagtctctttctcatgaagctg

SEQ ID NO: 44 - DNA, 36 bp, synthetic construct
  source 1..36: mol_type = other DNA
gaaagagactggaaagacccaccctgaagagatacc

SEQ ID NO: 45 - DNA, 37 bp, synthetic construct
  source 1..37: mol_type = other DNA
cttcagggtgggtctttccagtctctttctcatgaag

SEQ ID NO: 46 - DNA, 36 bp, synthetic construct
  source 1..36: mol_type = other DNA
ctggaagcccccagactgaagagatacctgcgggac

SEQ ID NO: 47 - DNA, 35 bp, synthetic construct
  source 1..35: mol_type = other DNA
gtatctcttcagtctgggggcttccagtctctttc

SEQ ID NO: 48 - DNA, 36 bp, synthetic construct
  source 1..36: mol_type = other DNA
gatgaagaagaggagatactgcacctactgtcccag

SEQ ID NO: 49 - DNA, 36 bp, synthetic construct
  source 1..36: mol_type = other DNA
gtaggtgcagtatctcctcttcttcatcacgggttc

SEQ ID NO: 50 - DNA, 44 bp, synthetic construct
  source 1..44: mol_type = other DNA
gcaggaacatcacctgcgacgcctggttcaccagcatccccctg

SEQ ID NO: 51 - DNA, 29 bp, synthetic construct
  source 1..29: mol_type = other DNA
ccaggcgtcgcaggtgatgttcctgcagc

SEQ ID NO: 52 - DNA, 30 bp, synthetic construct
  source 1..30: mol_type = other DNA
aacaaggaggagatcccagaggtgctgaag

SEQ ID NO: 53 - DNA, 43 bp, synthetic construct
  source 1..43: mol_type = other DNA
gcacctctgggatctcctccttgttgctccgcacggtgcccac

SEQ ID NO: 54 - DNA, 36 bp, synthetic construct
  source 1..36: mol_type = other DNA
cgtggacaccctgaaccagatgtgcagcgtgatgac

SEQ ID NO: 55 - DNA, 34 bp, synthetic construct
  source 1..34: mol_type = other DNA
gcacatctggttcagggtgtccacgccgcccttg

SEQ ID NO: 56 - DNA, 37 bp, synthetic construct
  source 1..37: mol_type = other DNA
gtgggcaccgtggccagcaacaagcgggagatcccag

SEQ ID NO: 57 - DNA, 34 bp, synthetic construct
  source 1..34: mol_type = other DNA
gcttgttgctggccacggtgcccacgatggtcag

SEQ ID NO: 58 - DNA, 32 bp, synthetic construct
  source 1..32: mol_type = other DNA
ggagcaacgcccgggagatcccagaggtgctg

SEQ ID NO: 59 - DNA, 42 bp, synthetic construct
  source 1..42: mol_type = other DNA
tctgggatctcccgggcgttgctccgcacggtgcccacgatg

SEQ ID NO: 60 - DNA, 44 bp, synthetic construct
  source 1..44: mol_type = other DNA
gcaggaacatcacctgcgacgagtggttcaccagcatccccctg

SEQ ID NO: 61 - DNA, 39 bp, synthetic construct
  source 1..39: mol_type = other DNA
ccactcgtcgcaggtgatgttcctgcagctgccatgcac

SEQ ID NO: 62 - DNA, 38 bp, synthetic construct
  source 1..38: mol_type = other DNA
tgccctacctgggcgccggcacccagacaaacggcgtg

SEQ ID NO: 63 - DNA, 33 bp, synthetic construct
  source 1..33: mol_type = other DNA
tgggtgccggcgcccaggtagggcatgccgttg

SEQ ID NO: 64 - DNA, 34 bp, synthetic construct
  source 1..34: mol_type = other DNA
acggcatgcccgagctgggcagaggcacccagac

SEQ ID NO: 65 - DNA, 36 bp, synthetic construct
  source 1..36: mol_type = other DNA
cctctgcccagctcgggcatgccgttgatcatgtac

SEQ ID NO: 66 - DNA, 38 bp, synthetic construct
  source 1..38: mol_type = other DNA
tgccctacctgggcgagggcacccagacaaacggcgtg

SEQ ID NO: 67 - DNA, 33 bp, synthetic construct
  source 1..33: mol_type = other DNA
tgggtgccctcgcccaggtagggcatgccgttg

SEQ ID NO: 68 - DNA, 36 bp, synthetic construct
  source 1..36: mol_type = other DNA
ggcgtgcccgagggcgagtactacgtgaaagaactg

SEQ ID NO: 69 - DNA, 38 bp, synthetic construct
  source 1..38: mol_type = other DNA
cgtagtactcgccctcgggcacgccgtttgtctgggtg

SEQ ID NO: 70 - DNA, 37 bp, synthetic construct
  source 1..37: mol_type = other DNA
catcacctgcgacttctggttcaccagcatccccctg

SEQ ID NO: 71 - DNA, 35 bp, synthetic construct
  source 1..35: mol_type = other DNA
gctggtgaaccagaagtcgcaggtgatgttcctgc

SEQ ID NO: 72 - DNA, 37 bp, synthetic construct
  source 1..37: mol_type = other DNA
catcacctgcgacctgtggttcaccagcatccccctg

SEQ ID NO: 73 - DNA, 35 bp, synthetic construct
  source 1..35: mol_type = other DNA
gctggtgaaccacaggtcgcaggtgatgttcctgc

SEQ ID NO: 74 - DNA, 37 bp, synthetic construct
  source 1..37: mol_type = other DNA
catcacctgcgacatctggttcaccagcatccccctg

SEQ ID NO: 75 - DNA, 35 bp, synthetic construct
  source 1..35: mol_type = other DNA
gctggtgaaccagatgtcgcaggtgatgttcctgc

SEQ ID NO: 76 - DNA, 37 bp, synthetic construct
  source 1..37: mol_type = other DNA
catcacctgcgacatgtggttcaccagcatccccctg

SEQ ID NO: 77 - DNA, 35 bp, synthetic construct
  source 1..35: mol_type = other DNA
gctggtgaaccacatgtcgcaggtgatgttcctgc

SEQ ID NO: 78 - DNA, 37 bp, synthetic construct
  source 1..37: mol_type = other DNA
catcacctgcgacgtgtggttcaccagcatccccctg

SEQ ID NO: 79 - DNA, 35 bp, synthetic construct
  source 1..35: mol_type = other DNA
gctggtgaaccacacgtcgcaggtgatgttcctgc

SEQ ID NO: 80 - DNA, 37 bp, synthetic construct
  source 1..37: mol_type = other DNA
catcacctgcgacagctggttcaccagcatccccctg

SEQ ID NO: 81 - DNA, 35 bp, synthetic construct
  source 1..35: mol_type = other DNA
gctggtgaaccagctgtcgcaggtgatgttcctgc

SEQ ID NO: 82 - DNA, 37 bp, synthetic construct
  source 1..37: mol_type = other DNA
catcacctgcgacccctggttcaccagcatccccctg

SEQ ID NO: 83 - DNA, 35 bp, synthetic construct
  source 1..35: mol_type = other DNA
gctggtgaaccaggggtcgcaggtgatgttcctgc

SEQ ID NO: 84 - DNA, 37 bp, synthetic construct
  source 1..37: mol_type = other DNA
catcacctgcgacacctggttcaccagcatccccctg

SEQ ID NO: 85 - DNA, 35 bp, synthetic construct
  source 1..35: mol_type = other DNA
gctggtgaaccaggtgtcgcaggtgatgttcctgc

SEQ ID NO: 86 - DNA, 37 bp, synthetic construct
  source 1..37: mol_type = other DNA
catcacctgcgactactggttcaccagcatccccctg

SEQ ID NO: 87 - DNA, 35 bp, synthetic construct
  source 1..35: mol_type = other DNA
gctggtgaaccagtagtcgcaggtgatgttcctgc

SEQ ID NO: 88 - DNA, 37 bp, synthetic construct
  source 1..37: mol_type = other DNA
catcacctgcgaccactggttcaccagcatccccctg

SEQ ID NO: 89 - DNA, 35 bp, synthetic construct
  source 1..35: mol_type = other DNA
gctggtgaaccagtggtcgcaggtgatgttcctgc

SEQ ID NO: 90 - DNA, 37 bp, synthetic construct
  source 1..37: mol_type = other DNA
catcacctgcgaccagtggttcaccagcatccccctg

SEQ ID NO: 91 - DNA, 35 bp, synthetic construct
  source 1..35: mol_type = other DNA
gctggtgaaccactggtcgcaggtgatgttcctgc

SEQ ID NO: 92 - DNA, 37 bp, synthetic construct
  source 1..37: mol_type = other DNA
catcacctgcgacaagtggttcaccagcatccccctg

SEQ ID NO: 93 - DNA, 35 bp, synthetic construct
  source 1..35: mol_type = other DNA
gctggtgaaccacttgtcgcaggtgatgttcctgc

SEQ ID NO: 94 - DNA, 37 bp, synthetic construct
  source 1..37: mol_type = other DNA
catcacctgcgacgactggttcaccagcatccccctg

SEQ ID NO: 95 - DNA, 35 bp, synthetic construct
  source 1..35: mol_type = other DNA
gctggtgaaccagtcgtcgcaggtgatgttcctgc

SEQ ID NO: 96 - DNA, 37 bp, synthetic construct
  source 1..37: mol_type = other DNA
catcacctgcgactgctggttcaccagcatccccctg

SEQ ID NO: 97 - DNA, 35 bp, synthetic construct
  source 1..35: mol_type = other DNA
gctggtgaaccagcagtcgcaggtgatgttcctgc

SEQ ID NO: 98 - DNA, 37 bp, synthetic construct
  source 1..37: mol_type = other DNA
catcacctgcgactggtggttcaccagcatccccctg

SEQ ID NO: 99 - DNA, 35 bp, synthetic construct
  source 1..35: mol_type = other DNA
gctggtgaaccaccagtcgcaggtgatgttcctgc

SEQ ID NO: 100 - DNA, 37 bp, synthetic construct
  source 1..37: mol_type = other DNA
catcacctgcgacagatggttcaccagcatccccctg

SEQ ID NO: 101 - DNA, 35 bp, synthetic construct
  source 1..35: mol_type = other DNA
gctggtgaaccatctgtcgcaggtgatgttcctgc

SEQ ID NO: 102 - DNA, 37 bp, synthetic construct
  source 1..37: mol_type = other DNA
catcacctgcgacggctggttcaccagcatccccctg

SEQ ID NO: 103 - DNA, 35 bp, synthetic construct
  source 1..35: mol_type = other DNA
gctggtgaaccagccgtcgcaggtgatgttcctgc

SEQ ID NO: 104 - DNA, 36 bp, synthetic construct
  source 1..36: mol_type = other DNA
cgtggacaccctggcccagatgtgcagcgtgatgac

SEQ ID NO: 105 - DNA, 34 bp, synthetic construct
  source 1..34: mol_type = other DNA
gcacatctgggccagggtgtccacgccgcccttg

SEQ ID NO: 106 - DNA, 36 bp, synthetic construct
  source 1..36: mol_type = other DNA
cgtggacaccctgctgcagatgtgcagcgtgatgac

SEQ ID NO: 107 - DNA, 34 bp, synthetic construct
  source 1..34: mol_type = other DNA
gcacatctgcagcagggtgtccacgccgcccttg

SEQ ID NO: 108 - DNA, 36 bp, synthetic construct
  source 1..36: mol_type = other DNA
cgtggacaccctgatgcagatgtgcagcgtgatgac

SEQ ID NO: 109 - DNA, 34 bp, synthetic construct
  source 1..34: mol_type = other DNA
gcacatctgcatcagggtgtccacgccgcccttg

SEQ ID NO: 110 - DNA, 36 bp, synthetic construct
  source 1..36: mol_type = other DNA
cgtggacaccctgttccagatgtgcagcgtgatgac

SEQ ID NO: 111 - DNA, 35 bp, synthetic construct
  source 1..35: mol_type = other DNA
gcacatctggaacagggtgtccacgccgcccttgs

SEQ ID NO: 112 - DNA, 36 bp, synthetic construct
  source 1..36: mol_type = other DNA
cgtggacaccctgagccagatgtgcagcgtgatgac

SEQ ID NO: 113 - DNA, 34 bp, synthetic construct
  source 1..34: mol_type = other DNA
gcacatctggctcagggtgtccacgccgcccttg

SEQ ID NO: 114 - DNA, 36 bp, synthetic construct
  source 1..36: mol_type = other DNA
cgtggacaccctgacccagatgtgcagcgtgatgac

SEQ ID NO: 115 - DNA, 34 bp, synthetic construct
  source 1..34: mol_type = other DNA
gcacatctgggtcagggtgtccacgccgcccttg

SEQ ID NO: 116 - DNA, 36 bp, synthetic construct
  source 1..36: mol_type = other DNA
cgtggacaccctgtgccagatgtgcagcgtgatgac

SEQ ID NO: 117 - DNA, 34 bp, synthetic construct
  source 1..34: mol_type = other DNA
gcacatctggcacagggtgtccacgccgcccttg

SEQ ID NO: 118 - DNA, 36 bp, synthetic construct
  source 1..36: mol_type = other DNA
cgtggacaccctgtaccagatgtgcagcgtgatgac

SEQ ID NO: 119 - DNA, 34 bp, synthetic construct
  source 1..34: mol_type = other DNA
gcacatctggtacagggtgtccacgccgcccttg

SEQ ID NO: 120 - DNA, 36 bp, synthetic construct
  source 1..36: mol_type = other DNA
cgtggacaccctgcagcagatgtgcagcgtgatgac

SEQ ID NO: 121 - DNA, 34 bp, synthetic construct
  source 1..34: mol_type = other DNA
gcacatctgctgcagggtgtccacgccgcccttg

SEQ ID NO: 122 - DNA, 36 bp, synthetic construct
  source 1..36: mol_type = other DNA
cgtggacaccctgaagcagatgtgcagcgtgatgac

SEQ ID NO: 123 - DNA, 34 bp, synthetic construct
  source 1..34: mol_type = other DNA
gcacatctgcttcagggtgtccacgccgcccttg

SEQ ID NO: 124 - DNA, 36 bp, synthetic construct
  source 1..36: mol_type = other DNA
cgtggacaccctgagacagatgtgcagcgtgatgac

SEQ ID NO: 125 - DNA, 34 bp, synthetic construct
  source 1..34: mol_type = other DNA
gcacatctgtctcagggtgtccacgccgcccttg

SEQ ID NO: 126 - DNA, 20 bp, synthetic construct
  source 1..20: mol_type = other DNA
cagaacacagaagtgcagtc

SEQ ID NO: 127 - DNA, 20 bp, synthetic construct
  source 1..20: mol_type = other DNA
gatgcacttcaggatatgag

SEQ ID NO: 128 - DNA, 21 bp, synthetic construct
  source 1..21: mol_type = other DNA
atgtcctaaatgcacagcgac

SEQ ID NO: 129 - DNA, 20 bp, synthetic construct
  source 1..20: mol_type = other DNA
aacctcgatatacagaccga

SEQ ID NO: 130 - DNA, 18 bp, synthetic construct
  source 1..18: mol_type = other DNA
caccccacagtggccact

SEQ ID NO: 131 - DNA, 395 bp, synthetic construct
  source 1..395: mol_type = other DNA
gagggcctatttcccatgattccttcatatttgcatatacgatacaaggctgttagagagataattggaattaatttgactgtaaacacaaagatattagtacaaaatacgtgacgtagaaagtaataatttcttgggtagtttgcagttttaaaattatgttttaaaatggactatcatatgcttaccgtaacttgaaagtatttcgatttcttggctttatatatcttgtggaaaggacgaaacaccgtcgagtcgcttctcgattagttttagagctagaaatagcaagttaaaataaggctagtccgttatcaacttgaaaaagtggcaccgagtcggtgcttttttgttttagagctagaaatagcaagttaaaataaggctagtccgtt

SEQ ID NO: 132 - DNA, 19 bp, synthetic construct
  source 1..19: mol_type = other DNA
gtcgagtcgctttcgatta

SEQ ID NO: 133 - DNA, 22 bp, synthetic construct
  source 1..22: mol_type = other DNA
ttagtcctagtgcccatgaaag

SEQ ID NO: 134 - DNA, 17 bp, synthetic construct
  source 1..17: mol_type = other DNA
catcagacttgatgatg

SEQ ID NO: 135 - DNA, 5964 bp, synthetic construct
  source 1..5964: mol_type = other DNA
atggacaagaagtactccattgggctcgacatcggcacaaacagcgtcggctgggccgtcattacggacgagtacaaggtgccgagcaaaaaattcaaagttctgggcaataccgatcgccacagcataaagaagaacctcattggcgccctcctgttcgactccggggagacggccgaagccacgcggctcaaaagaacagcacggcgcagatatacccgcagaaagaatcggatctgctacctgcaggagatctttagtaatgagatggctaaggtggatgactctttcttccataggctggaggagtcctttttggtggaggaggataaaaagcacgagcgccacccaatctttggcaatatcgtggacgaggtggcgtaccatgaaaagtacccaaccatatatcatctgaggaagaagcttgtagacagtactgataaggctgacttgcggttgatctatctcgcgctggcgcatatgatcaaatttcggggacacttcctcatcgagggggacctgaacccagacaacagcgatgtcgacaaactctttatccaactggttcagacttacaatcagcttttcgaagagaacccgatcaacgcatccggagttgacgccaaagcaatcctgagcgctaggctgtccaaatcccggcggctcgaaaacctcatcgcacagctccctggggagaagaagaacggcctgtttggtaatcttatcgccctgtcactcgggctgacccccaactttaaatctaacttcgacctggccgaagatgccaagcttcaactgagcaaagacacctacgatgatgatctcgacaatctgctggcccagatcggcgaccagtacgcagacctttttttggcggcaaagaacctgtcagacgccattctgctgagtgatattctgcgagtgaacacggagatcaccaaagctccgctgagcgctagtatgatcaagcgctatgatgagcaccaccaagacttgactttgctgaaggcccttgtcagacagcaactgcctgagaagtacaaggaaattttcttcgatcagtctaaaaatggctacgccggatacattgacggcggagcaagccaggaggaattttacaaatttattaagcccatcttggaaaaaatggacggcaccgaggagctgctggtaaagcttaacagagaagatctgttgcgcaaacagcgcactttcgacaatggaagcatcccccaccagattcacctgggcgaactgcacgctatcctcaggcggcaagaggatttctacccctttttgaaagataacagggaaaagattgagaaaatcctcacatttcggataccctactatgtaggccccctcgcccggggaaattccagattcgcgtggatgactcgcaaatcagaagagaccatcactccctggaacttcgaggaagtcgtggataagggggcctctgcccagtccttcatcgaaaggatgactaactttgataaaaatctgcctaacgaaaaggtgcttcctaaacactctctgctgtacgagtacttcacagtttataacgagctcaccaaggtcaaatacgtcacagaagggatgagaaagccagcattcctgtctggagagcagaagaaagctatcgtggacctcctcttcaagacgaaccggaaagttaccgtgaaacagctcaaagaagactatttcaaaaagattgaatgtttcgactctgttgaaatcagcggagtggaggatcgcttcaacgcatccctgggaacgtatcacgatctcctgaaaatcattaaagacaaggacttcctggacaatgaggagaacgaggacattcttgaggacattgtcctcacccttacgttgtttgaagatagggagatgattgaagaacgcttgaaaacttacgctcatctcttcgacgacaaagtcatgaaacagctcaagaggcgccgatatacaggatgggggcggctgtcaagaaaactgatcaatgggatccgagacaagcagagtggaaagacaatcctggattttcttaagtccgatggatttgccaacaggaacttcatgcagttgatccatgatgactctctcacctttaaggaggacatccagaaagcacaagtttctggccagggggacagtcttcacgagcacatcgctaatcttgcaggtagcccagctatcaaaaagggaatactgcagaccgttaaggtcgtggatgaactcgtcaaagtaatgggaaggcataagcccgagaatatcgttatcgagatggcccgagagaaccaaactacccagaagggacagaagaacagtagggaaaggatgaagaggattgaagagggtataaaagaactggggtcccaaatccttaaggaacacccagttgaaaacacccagcttcagaatgagaagctctacctgtactacctgcagaacggcagggacatgtacgtggatcaggaactggacatcaatcggctctccgactacgacgtggatcatatcgtgccccagtcttttctcaaagatgattctattgataataaagtgttgacaagatccgataaaaatagagggaagagtgataacgtcccctcagaagaagttgtcaagaaaatgaaaaattattggcggcagctgctgaacgccaaactgatcacacaacggaagttcgataatctgactaaggctgaacgaggtggcctgtctgagttggataaagccggcttcatcaaaaggcagcttgttgagacacgccagatcaccaagcacgtggcccaaattctcgattcacgcatgaacaccaagtacgatgaaaatgacaaactgattcgagaggtgaaagttattactctgaagtctaagctggtctcagatttcagaaaggactttcagttttataaggtgagagagatcaacaattaccaccatgcgcatgatgcctacctgaatgcagtggtaggcactgcacttatcaaaaaatatcccaagcttgaatctgaatttgtttacggagactataaagtgtacgatgttaggaaaatgatcgcaaagtctgagcaggaaataggcaaggccaccgctaagtacttcttttacagcaatattatgaattttttcaagaccgagattacactggccaatggagagattcggaagcgaccacttatcgaaacaaacggagaaacaggagaaatcgtgtgggacaagggtagggatttcgcgacagtccggaaggtcctgtccatgccgcaggtgaacatcgttaaaaagaccgaagtacagaccggaggcttctccaaggaaagtatcctcccgaaaaggaacagcgacaagctgatcgcacgcaaaaaagattgggaccccaagaaatacggcggattcgattctcctacagtcgcttacagtgtactggttgtggccaaagtggagaaagggaagtctaaaaaactcaaaagcgtcaaggaactgctgggcatcacaatcatggagcgatcaagcttcgaaaaaaaccccatcgactttctcgaggcgaaaggatataaagaggtcaaaaaagacctcatcattaagcttcccaagtactctctctttgagcttgaaaacggccggaaacgaatgctcgctagtgcgggcgagctgcagaaaggtaacgagctggcactgccctctaaatacgttaatttcttgtatctggccagccactatgaaaagctcaaagggtctcccgaagataatgagcagaagcagctgttcgtggaacaacacaaacactaccttgatgagatcatcgagcaaataagcgaattctccaaaagagtgatcctcgccgacgctaacctcgataaggtgctttctgcttacaataagcacagggataagcccatcagggagcaggcagaaaacattatccacttgtttactctgaccaacttgggcgcgcctgcagccttcaagtacttcgacaccaccatagacagaaagcggtacacctctacaaaggaggtcctggacgccacactgattcatcagtcaattacggggctctatgaaacaagaatcgacctctctcagctcggtggagacagcagggctgaccccaagaagaagaggaaggtgggcggaggagggagtggcggaggcggaagcggcggcggaggcagcggctctagcctggacgacgagcacatcctgagcgccctgctgcagagcgacgacgaactggtgggcgaggacagcgacagcgaggtcagcgaccacgtgtccgaggacgacgtgcagtccgacaccgaggaagccttcatcgacgaggtgcacgaagtgcagcctaccagcagcggctccgagatcctggacgagcagaacgtgatcgagcagcctggcagctccctggccagcaacagaatcctgaccctgccccagagaaccatcagaggcaagaacaagcactgctggtccacctccaagagcaccaggcggagcagagtgtccgccctgaacatcgtgcggagccagaggggccccaccagaatgtgcagaaacatctacgaccccctgctgtgcttcaagctgttcttcaccgacgagatcatcagcgagatcgtgaagtggaccaacgccgagatcagcctgaagaggcgggagagcatgaccagcgccaccttcagagacaccaacgaggacgagatctacgccttcttcggcatcctggtgatgaccgccgtgagaaaggacaaccacatgagcaccgacgacctgttcgacagatccctgagcatggtgtacgtgtccgtgatgagcagagacagattcgacttcctgatcagatgcctgagaatggacgacaagagcatcagacccaccctgcgggagaacgacgtgttcacccccgtgcggaagatctgggacctgttcatccaccagtgcatccagaactacacccctggcgcccacctgaccatcgatgagcagctgctgggcttcagaggcagatgccccttcagagtgtacatccccaacaagcccagcaagtacggcatcaagatcctgatgatgtgcgacagcggcaccaagtacatgatcaacggcatgccctacctgggcagaggcacccagacaaacggcgtgcccctgggcgagtactacgtgaaagaactgagcaagcctgtgcatggcagctgcaggaacatcacctgcgacgcctggttcaccagcatccccctggccaagaacctgctgcaggaaccctacaagctgaccatcgtgggcaccgtgcggagcaacaaggaggagatcccagaggtgctgaagaacagcagatccagacctgtgggaacaagcatgttctgcttcgacggccccctgaccctggtgtcctacaagcccaagcccgccaagatggtgtacctgctgtccagctgcgacgaggacgccagcatcaacgagagcaccggcaagccccagatggtgatgtactacaaccagaccaagggcggcgtggacaccctgaaccagatgtgcagcgtgatgacctgcagcagaaagaccaacagatggcccatggccctgctgtacggcatgatcaatatcgcctgcatcaacagcttcatcatctacagccacaacgtgtccagcaagggcgagaaggtgcagagccggaagaaattcatgcggaacctgtacatgagcctgacctccagcttcatgagaaagagactggaagcccccaccctgaagagatacctgcgggacaacatcagcaacatcctgcccaaggaagtgccaggaacaagcgacgacagcaccgaggaacccgtgatgaagaagaggacctactgcacctactgtcccagcaagatcagaagaaaggccaacgccagctgcaagaaatgcaaaaaagtgatctgccgggagcacaacatcgacatgtgccagagctgtttctga

SEQ ID NO: 136 - DNA, 5964 bp, synthetic construct
  source 1..5964: mol_type = other DNA
atggacaagaagtactccattgggctcgacatcggcacaaacagcgtcggctgggccgtcattacggacgagtacaaggtgccgagcaaaaaattcaaagttctgggcaataccgatcgccacagcataaagaagaacctcattggcgccctcctgttcgactccggggagacggccgaagccacgcggctcaaaagaacagcacggcgcagatatacccgcagaaagaatcggatctgctacctgcaggagatctttagtaatgagatggctaaggtggatgactctttcttccataggctggaggagtcctttttggtggaggaggataaaaagcacgagcgccacccaatctttggcaatatcgtggacgaggtggcgtaccatgaaaagtacccaaccatatatcatctgaggaagaagcttgtagacagtactgataaggctgacttgcggttgatctatctcgcgctggcgcatatgatcaaatttcggggacacttcctcatcgagggggacctgaacccagacaacagcgatgtcgacaaactctttatccaactggttcagacttacaatcagcttttcgaagagaacccgatcaacgcatccggagttgacgccaaagcaatcctgagcgctaggctgtccaaatcccggcggctcgaaaacctcatcgcacagctccctggggagaagaagaacggcctgtttggtaatcttatcgccctgtcactcgggctgacccccaactttaaatctaacttcgacctggccgaagatgccaagcttcaactgagcaaagacacctacgatgatgatctcgacaatctgctggcccagatcggcgaccagtacgcagacctttttttggcggcaaagaacctgtcagacgccattctgctgagtgatattctgcgagtgaacacggagatcaccaaagctccgctgagcgctagtatgatcaagcgctatgatgagcaccaccaagacttgactttgctgaaggcccttgtcagacagcaactgcctgagaagtacaaggaaattttcttcgatcagtctaaaaatggctacgccggatacattgacggcggagcaagccaggaggaattttacaaatttattaagcccatcttggaaaaaatggacggcaccgaggagctgctggtaaagcttaacagagaagatctgttgcgcaaacagcgcactttcgacaatggaagcatcccccaccagattcacctgggcgaactgcacgctatcctcaggcggcaagaggatttctacccctttttgaaagataacagggaaaagattgagaaaatcctcacatttcggataccctactatgtaggccccctcgcccggggaaattccagattcgcgtggatgactcgcaaatcagaagagaccatcactccctggaacttcgaggaagtcgtggataagggggcctctgcccagtccttcatcgaaaggatgactaactttgataaaaatctgcctaacgaaaaggtgcttcctaaacactctctgctgtacgagtacttcacagtttataacgagctcaccaaggtcaaatacgtcacagaagggatgagaaagccagcattcctgtctggagagcagaagaaagctatcgtggacctcctcttcaagacgaaccggaaagttaccgtgaaacagctcaaagaagactatttcaaaaagattgaatgtttcgactctgttgaaatcagcggagtggaggatcgcttcaacgcatccctgggaacgtatcacgatctcctgaaaatcattaaagacaaggacttcctggacaatgaggagaacgaggacattcttgaggacattgtcctcacccttacgttgtttgaagatagggagatgattgaagaacgcttgaaaacttacgctcatctcttcgacgacaaagtcatgaaacagctcaagaggcgccgatatacaggatgggggcggctgtcaagaaaactgatcaatgggatccgagacaagcagagtggaaagacaatcctggattttcttaagtccgatggatttgccaacaggaacttcatgcagttgatccatgatgactctctcacctttaaggaggacatccagaaagcacaagtttctggccagggggacagtcttcacgagcacatcgctaatcttgcaggtagcccagctatcaaaaagggaatactgcagaccgttaaggtcgtggatgaactcgtcaaagtaatgggaaggcataagcccgagaatatcgttatcgagatggcccgagagaaccaaactacccagaagggacagaagaacagtagggaaaggatgaagaggattgaagagggtataaaagaactggggtcccaaatccttaaggaacacccagttgaaaacacccagcttcagaatgagaagctctacctgtactacctgcagaacggcagggacatgtacgtggatcaggaactggacatcaatcggctctccgactacgacgtggatcatatcgtgccccagtcttttctcaaagatgattctattgataataaagtgttgacaagatccgataaaaatagagggaagagtgataacgtcccctcagaagaagttgtcaagaaaatgaaaaattattggcggcagctgctgaacgccaaactgatcacacaacggaagttcgataatctgactaaggctgaacgaggtggcctgtctgagttggataaagccggcttcatcaaaaggcagcttgttgagacacgccagatcaccaagcacgtggcccaaattctcgattcacgcatgaacaccaagtacgatgaaaatgacaaactgattcgagaggtgaaagttattactctgaagtctaagctggtctcagatttcagaaaggactttcagttttataaggtgagagagatcaacaattaccaccatgcgcatgatgcctacctgaatgcagtggtaggcactgcacttatcaaaaaatatcccaagcttgaatctgaatttgtttacggagactataaagtgtacgatgttaggaaaatgatcgcaaagtctgagcaggaaataggcaaggccaccgctaagtacttcttttacagcaatattatgaattttttcaagaccgagattacactggccaatggagagattcggaagcgaccacttatcgaaacaaacggagaaacaggagaaatcgtgtgggacaagggtagggatttcgcgacagtccggaaggtcctgtccatgccgcaggtgaacatcgttaaaaagaccgaagtacagaccggaggcttctccaaggaaagtatcctcccgaaaaggaacagcgacaagctgatcgcacgcaaaaaagattgggaccccaagaaatacggcggattcgattctcctacagtcgcttacagtgtactggttgtggccaaagtggagaaagggaagtctaaaaaactcaaaagcgtcaaggaactgctgggcatcacaatcatggagcgatcaagcttcgaaaaaaaccccatcgactttctcgaggcgaaaggatataaagaggtcaaaaaagacctcatcattaagcttcccaagtactctctctttgagcttgaaaacggccggaaacgaatgctcgctagtgcgggcgagctgcagaaaggtaacgagctggcactgccctctaaatacgttaatttcttgtatctggccagccactatgaaaagctcaaagggtctcccgaagataatgagcagaagcagctgttcgtggaacaacacaaacactaccttgatgagatcatcgagcaaataagcgaattctccaaaagagtgatcctcgccgacgctaacctcgataaggtgctttctgcttacaataagcacagggataagcccatcagggagcaggcagaaaacattatccacttgtttactctgaccaacttgggcgcgcctgcagccttcaagtacttcgacaccaccatagacagaaagcggtacacctctacaaaggaggtcctggacgccacactgattcatcagtcaattacggggctctatgaaacaagaatcgacctctctcagctcggtggagacagcagggctgaccccaagaagaagaggaaggtgggcggaggagggagtggcggaggcggaagcggcggcggaggcagcggctctagcctggacgacgagcacatcctgagcgccctgctgcagagcgacgacgaactggtgggcgaggacagcgacagcgaggtcagcgaccacgtgtccgaggacgacgtgcagtccgacaccgaggaagccttcatcgacgaggtgcacgaagtgcagcctaccagcagcggctccgagatcctggacgagcagaacgtgatcgagcagcctggcagctccctggccagcaacagaatcctgaccctgccccagagaaccatcagaggcaagaacaagcactgctggtccacctccaagagcaccaggcggagcagagtgtccgccctgaacatcgtgcggagccagaggggccccaccagaatgtgcagaaacatctacgaccccctgctgtgcttcaagctgttcttcaccgacgagatcatcagcgagatcgtgaagtggaccaacgccgagatcagcctgaagaggcgggagagcatgaccagcgccaccttcagagacaccaacgaggacgagatctacgccttcttcggcatcctggtgatgaccgccgtgagaaaggacaaccacatgagcaccgacgacctgttcgacagatccctgagcatggtgtacgtgtccgtgatgagcagagacagattcgacttcctgatcagatgcctgagaatggacgacaagagcatcagacccaccctgcgggagaacgacgtgttcacccccgtgcggaagatctgggacctgttcatccaccagtgcatccagaactacacccctggcgcccacctgaccatcgatgagcagctgctgggcttcagaggcagatgccccttcagagtgtacatccccaacaagcccagcaagtacggcatcaagatcctgatgatgtgcgacagcggcaccaagtacatgatcaacggcatgccctacctgggcagaggcacccagacaaacggcgtgcccctgggcgagtactacgtgaaagaactgagcaagcctgtgcatggcagctgcaggaacatcacctgcgacgagtggttcaccagcatccccctggccaagaacctgctgcaggaaccctacaagctgaccatcgtgggcaccgtgcggagcaacaaggaggagatcccagaggtgctgaagaacagcagatccagacctgtgggaacaagcatgttctgcttcgacggccccctgaccctggtgtcctacaagcccaagcccgccaagatggtgtacctgctgtccagctgcgacgaggacgccagcatcaacgagagcaccggcaagccccagatggtgatgtactacaaccagaccaagggcggcgtggacaccctgaaccagatgtgcagcgtgatgacctgcagcagaaagaccaacagatggcccatggccctgctgtacggcatgatcaatatcgcctgcatcaacagcttcatcatctacagccacaacgtgtccagcaagggcgagaaggtgcagagccggaagaaattcatgcggaacctgtacatgagcctgacctccagcttcatgagaaagagactggaagcccccaccctgaagagatacctgcgggacaacatcagcaacatcctgcccaaggaagtgccaggaacaagcgacgacagcaccgaggaacccgtgatgaagaagaggacctactgcacctactgtcccagcaagatcagaagaaaggccaacgccagctgcaagaaatgcaaaaaagtgatctgccgggagcacaacatcgacatgtgccagagctgtttctga

SEQ ID NO: 137 - DNA, 5964 bp, synthetic construct
  source 1..5964: mol_type = other DNA
atggacaagaagtactccattgggctcgacatcggcacaaacagcgtcggctgggccgtcattacggacgagtacaaggtgccgagcaaaaaattcaaagttctgggcaataccgatcgccacagcataaagaagaacctcattggcgccctcctgttcgactccggggagacggccgaagccacgcggctcaaaagaacagcacggcgcagatatacccgcagaaagaatcggatctgctacctgcaggagatctttagtaatgagatggctaaggtggatgactctttcttccataggctggaggagtcctttttggtggaggaggataaaaagcacgagcgccacccaatctttggcaatatcgtggacgaggtggcgtaccatgaaaagtacccaaccatatatcatctgaggaagaagcttgtagacagtactgataaggctgacttgcggttgatctatctcgcgctggcgcatatgatcaaatttcggggacacttcctcatcgagggggacctgaacccagacaacagcgatgtcgacaaactctttatccaactggttcagacttacaatcagcttttcgaagagaacccgatcaacgcatccggagttgacgccaaagcaatcctgagcgctaggctgtccaaatcccggcggctcgaaaacctcatcgcacagctccctggggagaagaagaacggcctgtttggtaatcttatcgccctgtcactcgggctgacccccaactttaaatctaacttcgacctggccgaagatgccaagcttcaactgagcaaagacacctacgatgatgatctcgacaatctgctggcccagatcggcgaccagtacgcagacctttttttggcggcaaagaacctgtcagacgccattctgctgagtgatattctgcgagtgaacacggagatcaccaaagctccgctgagcgctagtatgatcaagcgctatgatgagcaccaccaagacttgactttgctgaaggcccttgtcagacagcaactgcctgagaagtacaaggaaattttcttcgatcagtctaaaaatggctacgccggatacattgacggcggagcaagccaggaggaattttacaaatttattaagcccatcttggaaaaaatggacggcaccgaggagctgctggtaaagcttaacagagaagatctgttgcgcaaacagcgcactttcgacaatggaagcatcccccaccagattcacctgggcgaactgcacgctatcctcaggcggcaagaggatttctacccctttttgaaagataacagggaaaagattgagaaaatcctcacatttcggataccctactatgtaggccccctcgcccggggaaattccagattcgcgtggatgactcgcaaatcagaagagaccatcactccctggaacttcgaggaagtcgtggataagggggcctctgcccagtccttcatcgaaaggatgactaactttgataaaaatctgcctaacgaaaaggtgcttcctaaacactctctgctgtacgagtacttcacagtttataacgagctcaccaaggtcaaatacgtcacagaagggatgagaaagccagcattcctgtctggagagcagaagaaagctatcgtggacctcctcttcaagacgaaccggaaagttaccgtgaaacagctcaaagaagactatttcaaaaagattgaatgtttcgactctgttgaaatcagcggagtggaggatcgcttcaacgcatccctgggaacgtatcacgatctcctgaaaatcattaaagacaaggacttcctggacaatgaggagaacgaggacattcttgaggacattgtcctcacccttacgttgtttgaagatagggagatgattgaagaacgcttgaaaacttacgctcatctcttcgacgacaaagtcatgaaacagctcaagaggcgccgatatacaggatgggggcggctgtcaagaaaactgatcaatgggatccgagacaagcagagtggaaagacaatcctggattttcttaagtccgatggatttgccaacaggaacttcatgcagttgatccatgatgactctctcacctttaaggaggacatccagaaagcacaagtttctggccagggggacagtcttcacgagcacatcgctaatcttgcaggtagcccagctatcaaaaagggaatactgcagaccgttaaggtcgtggatgaactcgtcaaagtaatgggaaggcataagcccgagaatatcgttatcgagatggcccgagagaaccaaactacccagaagggacagaagaacagtagggaaaggatgaagaggattgaagagggtataaaagaactggggtcccaaatccttaaggaacacccagttgaaaacacccagcttcagaatgagaagctctacctgtactacctgcagaacggcagggacatgtacgtggatcaggaactggacatcaatcggctctccgactacgacgtggatcatatcgtgccccagtcttttctcaaagatgattctattgataataaagtgttgacaagatccgataaaaatagagggaagagtgataacgtcccctcagaagaagttgtcaagaaaatgaaaaattattggcggcagctgctgaacgccaaactgatcacacaacggaagttcgataatctgactaaggctgaacgaggtggcctgtctgagttggataaagccggcttcatcaaaaggcagcttgttgagacacgccagatcaccaagcacgtggcccaaattctcgattcacgcatgaacaccaagtacgatgaaaatgacaaactgattcgagaggtgaaagttattactctgaagtctaagctggtctcagatttcagaaaggactttcagttttataaggtgagagagatcaacaattaccaccatgcgcatgatgcctacctgaatgcagtggtaggcactgcacttatcaaaaaatatcccaagcttgaatctgaatttgtttacggagactataaagtgtacgatgttaggaaaatgatcgcaaagtctgagcaggaaataggcaaggccaccgctaagtacttcttttacagcaatattatgaattttttcaagaccgagattacactggccaatggagagattcggaagcgaccacttatcgaaacaaacggagaaacaggagaaatcgtgtgggacaagggtagggatttcgcgacagtccggaaggtcctgtccatgccgcaggtgaacatcgttaaaaagaccgaagtacagaccggaggcttctccaaggaaagtatcctcccgaaaaggaacagcgacaagctgatcgcacgcaaaaaagattgggaccccaagaaatacggcggattcgattctcctacagtcgcttacagtgtactggttgtggccaaagtggagaaagggaagtctaaaaaactcaaaagcgtcaaggaactgctgggcatcacaatcatggagcgatcaagcttcgaaaaaaaccccatcgactttctcgaggcgaaaggatataaagaggtcaaaaaagacctcatcattaagcttcccaagtactctctctttgagcttgaaaacggccggaaacgaatgctcgctagtgcgggcgagctgcagaaaggtaacgagctggcactgccctctaaatacgttaatttcttgtatctggccagccactatgaaaagctcaaagggtctcccgaagataatgagcagaagcagctgttcgtggaacaacacaaacactaccttgatgagatcatcgagcaaataagcgaattctccaaaagagtgatcctcgccgacgctaacctcgataaggtgctttctgcttacaataagcacagggataagcccatcagggagcaggcagaaaacattatccacttgtttactctgaccaacttgggcgcgcctgcagccttcaagtacttcgacaccaccatagacagaaagcggtacacctctacaaaggaggtcctggacgccacactgattcatcagtcaattacggggctctatgaaacaagaatcgacctctctcagctcggtggagacagcagggctgaccccaagaagaagaggaaggtgggcggaggagggagtggcggaggcggaagcggcggcggaggcagcggctctagcctggacgacgagcacatcctgagcgccctgctgcagagcgacgacgaactggtgggcgaggacagcgacagcgaggtcagcgaccacgtgtccgaggacgacgtgcagtccgacaccgaggaagccttcatcgacgaggtgcacgaagtgcagcctaccagcagcggctccgagatcctggacgagcagaacgtgatcgagcagcctggcagctccctggccagcaacagaatcctgaccctgccccagagaaccatcagaggcaagaacaagcactgctggtccacctccaagagcaccaggcggagcagagtgtccgccctgaacatcgtgcggagccagaggggccccaccagaatgtgcagaaacatctacgaccccctgctgtgcttcaagctgttcttcaccgacgagatcatcagcgagatcgtgaagtggaccaacgccgagatcagcctgaagaggcgggagagcatgaccagcgccaccttcagagacaccaacgaggacgagatctacgccttcttcggcatcctggtgatgaccgccgtgagaaaggacaaccacatgagcaccgacgacctgttcgacagatccctgagcatggtgtacgtgtccgtgatgagcagagacagattcgacttcctgatcagatgcctgagaatggacgacaagagcatcagacccaccctgcgggagaacgacgtgttcacccccgtgcggaagatctgggacctgttcatccaccagtgcatccagaactacacccctggcgcccacctgaccatcgatgagcagctgctgggcttcagaggcagatgccccttcagagtgtacatccccaacaagcccagcaagtacggcatcaagatcctgatgatgtgcgacagcggcaccaagtacatgatcaacggcatgccctacctgggcgccggcacccagacaaacggcgtgcccctgggcgagtactacgtgaaagaactgagcaagcctgtgcatggcagctgcaggaacatcacctgcgacgagtggttcaccagcatccccctggccaagaacctgctgcaggaaccctacaagctgaccatcgtgggcaccgtgcggagcaacaagcgggagatcccagaggtgctgaagaacagcagatccagacctgtgggaacaagcatgttctgcttcgacggccccctgaccctggtgtcctacaagcccaagcccgccaagatggtgtacctgctgtccagctgcgacgaggacgccagcatcaacgagagcaccggcaagccccagatggtgatgtactacaaccagaccaagggcggcgtggacaccctgaaccagatgtgcagcgtgatgacctgcagcagaaagaccaacagatggcccatggccctgctgtacggcatgatcaatatcgcctgcatcaacagcttcatcatctacagccacaacgtgtccagcaagggcgagaaggtgcagagccggaagaaattcatgcggaacctgtacatgagcctgacctccagcttcatgagaaagagactggaagcccccaccctgaagagatacctgcgggacaacatcagcaacatcctgcccaaggaagtgccaggaacaagcgacgacagcaccgaggaacccgtgatgaagaagaggacctactgcacctactgtcccagcaagatcagaagaaaggccaacgccagctgcaagaaatgcaaaaaagtgatctgccgggagcacaacatcgacatgtgccagagctgtttctga

SEQ ID NO: 138 - DNA, 1785 bp, synthetic construct; identical to SEQ ID NO: 13
  source 1..1785: mol_type = other DNA

SEQ ID NO: 139 - DNA, 11803 bp, synthetic construct
  source 1..11803: mol_type = other DNA
gtgatgcggttttggcagtacatcaatgggcgtggatagcggtttgactcacggggatttccaagtctccaccccattgacgtcaatgggagtttgttttggcaccaaaatcaacgggactttccaaaatgtcgtaacaactccgccccattgacgcaaatgggcggtaggcgtgtacggtgggaggtctatataagcagagctcgtttagtgaaccgtcagatcgcctggagacgccatccacgctgttttgacctccatagaagacaccgggaccgatccagcctccggactctagaggatcgaacccttgccaccatggacaagaagtactccattgggctcgacatcggcacaaacagcgtcggctgggccgtcattacggacgagtacaaggtgccgagcaaaaaattcaaagttctgggcaataccgatcgccacagcataaagaagaacctcattggcgccctcctgttcgactccggggagacggccgaagccacgcggctcaaaagaacagcacggcgcagatatacccgcagaaagaatcggatctgctacctgcaggagatctttagtaatgagatggctaaggtggatgactctttcttccataggctggaggagtcctttttggtggaggaggataaaaagcacgagcgccacccaatctttggcaatatcgtggacgaggtggcgtaccatgaaaagtacccaaccatatatcatctgaggaagaagcttgtagacagtactgataaggctgacttgcggttgatctatctcgcgctggcgcatatgatcaaatttcggggacacttcctcatcgagggggacctgaacccagacaacagcgatgtcgacaaactctttatccaactggttcagacttacaatcagcttttcgaagagaacccgatcaacgcatccggagttgacgccaaagcaatcctgagcgctaggctgtccaaatcccggcggctcgaaaacctcatcgcacagctccctggggagaagaagaacggcctgtttggtaatcttatcgccctgtcactcgggctgacccccaactttaaatctaacttcgacctggccgaagatgccaagcttcaactgagcaaagacacctacgatgatgatctcgacaatctgctggcccagatcggcgaccagtacgcagacctttttttggcggcaaagaacctgtcagacgccattctgctgagtgatattctgcgagtgaacacggagatcaccaaagctccgctgagcgctagtatgatcaagcgctatgatgagcaccaccaagacttgactttgctgaaggcccttgtcagacagcaactgcctgagaagtacaaggaaattttcttcgatcagtctaaaaatggctacgccggatacattgacggcggagcaagccaggaggaattttacaaatttattaagcccatcttggaaaaaatggacggcaccgaggagctgctggtaaagcttaacagagaagatctgttgcgcaaacagcgcactttcgacaatggaagcatcccccaccagattcacctgggcgaactgcacgctatcctcaggcggcaagaggatttctacccctttttgaaagataacagggaaaagattgagaaaatcctcacatttcggataccctactatgtaggccccctcgcccggggaaattccagattcgcgtggatgactcgcaaatcagaagagaccatcactccctggaacttcgaggaagtcgtggataagggggcctctgcccagtccttcatcgaaaggatgactaactttgataaaaatctgcctaacgaaaaggtgcttcctaaacactctctgctgtacgagtacttcacagtttataacgagctcaccaaggtcaaatacgtcacagaagggatgagaaagccagcattcctgtctggagagcagaagaaagctatcgtggacctcctcttcaagacgaaccggaaagttaccgtgaaacagctcaaagaagactatttcaaaaagattgaatgtttcgactctgttgaaatcagcggagtggaggatcgcttcaacgcatccctgggaacgtatcacgatctcctgaaaatcattaaagacaaggacttcctggacaatgaggagaacgaggacattcttgaggacattgtcctcacccttacgttgtttgaagatagggagatgattgaagaacgcttgaaaacttacgctcatctcttcgacgacaaagtcatgaaacagctcaagaggcgccgatatacaggatgggggcggctgtcaagaaaactgatcaatgggatccgagacaagcagagtggaaagacaatcctggattttcttaagtccgatggatttgccaacaggaacttcatgcagttgatccatgatgactctctcacctttaaggaggacatccagaaagcacaagtttctggccagggggacagtcttcacgagcacatcgctaatcttgcaggtagcccagctatcaaaaagggaatactgcagaccgttaaggtcgtggatgaactcgtcaaagtaatgggaaggcataagcccgagaatatcgttatcgagatggcccgagagaaccaaactacccagaagggacagaagaacagtagggaaaggatgaagaggattgaagagggtataaaagaactggggtcccaaatccttaaggaacacccagttgaaaacacccagcttcagaatgagaagctctacctgtactacctgcagaacggcagggacatgtacgtggatcaggaactggacatcaatcggctctccgactacgacgtggatcatatcgtgccccagtcttttctcaaagatgattctattgataataaagtgttgacaagatccgataaaaatagagggaagagtgataacgtcccctcagaagaagttgtcaagaaaatgaaaaattattggcggcagctgctgaacgccaaactgatcacacaacggaagttcgataatctgactaaggctgaacgaggtggcctgtctgagttggataaagccggcttcatcaaaaggcagcttgttgagacacgccagatcaccaagcacgtggcccaaattctcgattcacgcatgaacaccaagtacgatgaaaatgacaaactgattcgagaggtgaaagttattactctgaagtctaagctggtctcagatttcagaaaggactttcagttttataaggtgagagagatcaacaattaccaccatgcgcatgatgcctacctgaatgcagtggtaggcactgcacttatcaaaaaatatcccaagcttgaatctgaatttgtttacggagactataaagtgtacgatgttaggaaaatgatcgcaaagtctgagcaggaaataggcaaggccaccgctaagtacttcttttacagcaatattatgaattttttcaagaccgagattacactggccaatggagagattcggaagcgaccacttatcgaaacaaacggagaaacaggagaaatcgtgtgggacaagggtagggatttcgcgacagtccggaaggtcctgtccatgccgcaggtgaacatcgttaaaaagaccgaagtacagaccggaggcttctccaaggaaagtatcctcccgaaaaggaacagcgacaagctgatcgcacgcaaaaaagattgggaccccaagaaatacggcggattcgattctcctacagtcgcttacagtgtactggttgtggccaaagtggagaaagggaagtctaaaaaactcaaaagcgtcaaggaactgctgggcatcacaatcatggagcgatcaagcttcgaaaaaaaccccatcgactttctcgaggcgaaaggatataaagaggtcaaaaaagacctcatcattaagcttcccaagtactctctctttgagcttgaaaacggccggaaacgaatgctcgctagtgcgggcgagctgcagaaaggtaacgagctggcactgccctctaaatacgttaatttcttgtatctggccagccactatgaaaagctcaaagggtctcccgaagataatgagcagaagcagctgttcgtggaacaacacaaacactaccttgatgagatcatcgagcaaataagcgaattctccaaaagagtgatcctcgccgacgctaacctcgataaggtgctttctgcttacaataagcacagggataagcccatcagggagcaggcagaaaacattatccacttgtttactctgaccaacttgggcgcgcctgcagccttcaagtacttcgacaccaccatagacagaaagcggtacacctctacaaaggaggtcctggacgccacactgattcatcagtcaattacggggctctatgaaacaagaatcgacctctctcagctcggtggagacagcagggctgaccccaagaagaagaggaaggtgggcggaggagggagtggcggaggcggaagcggcggcggaggcagcggctctagcctggacgacgagcacatcctgagcgccctgctgcagagcgacgacgaactggtgggcgaggacagcgacagcgaggtcagcgaccacgtgtccgaggacgacgtgcagtccgacaccgaggaagccttcatcgacgaggtgcacgaagtgcagcctaccagcagcggctccgagatcctggacgagcagaacgtgatcgagcagcctggcagctccctggccagcaacagaatcctgaccctgccccagagaaccatcagaggcaagaacaagcactgctggtccacctccaagagcaccaggcggagcagagtgtccgccctgaacatcgtgcggagccagaggggccccaccagaatgtgcagaaacatctacgaccccctgctgtgcttcaagctgttcttcaccgacgagatcatcagcgagatcgtgaagtggaccaacgccgagatcagcctgaagaggcgggagagcatgaccagcgccaccttcagagacaccaacgaggacgagatctacgccttcttcggcatcctggtgatgaccgccgtgagaaaggacaaccacatgagcaccgacgacctgttcgacagatccctgagcatggtgtacgtgtccgtgatgagcagagacagattcgacttcctgatcagatgcctgagaatggacgacaagagcatcagacccaccctgcgggagaacgacgtgttcacccccgtgcggaagatctgggacctgttcatccaccagtgcatccagaactacacccctggcgcccacctgaccatcgatgagcagctgctgggcttcagaggcagatgccccttcagagtgtacatccccaacaagcccagcaagtacggcatcaagatcctgatgatgtgcgacagcggcaccaagtacatgatcaacggcatgccctacctgggcagaggcacccagacaaacggcgtgcccctgggcgagtactacgtgaaagaactgagcaagcctgtgcatggcagctgcaggaacatcacctgcgacaactggttcaccagcatccccctggccaagaacctgctgcaggaaccctacaagctgaccatcgtgggcaccgtgcggagcaacaagcgggagatcccagaggtgctgaagaacagcagatccagacctgtgggaacaagcatgttctgcttcgacggccccctgaccctggtgtcctacaagcccaagcccgccaagatggtgtacctgctgtccagctgcgacgaggacgccagcatcaacgagagcaccggcaagccccagatggtgatgtactacaaccagaccaagggcggcgtggacaccctggaccagatgtgcagcgtgatgacctgcagcagaaagaccaacagatggcccatggccctgctgtacggcatgatcaatatcgcctgcatcaacagcttcatcatctacagccacaacgtgtccagcaagggcgagaaggtgcagagccggaagaaattcatgcggaacctgtacatgagcctgacctccagcttcatgagaaagagactggaagcccccaccctgaagagatacctgcgggacaacatcagcaacatcctgcccaaggaagtgccaggaacaagcgacgacagcaccgaggaacccgtgatgaagaagaggacctactgcacctactgtcccagcaagatcagaagaaaggccaacgccagctgcaagaaatgcaaaaaagtgatctgccgggagcacaacatcgacatgtgccagagctgtttctgaaagggttcgatccctaccggttagtaatgagtttaaacgggggaggctaactgaaacacggaaggagacaataccggaaggaacccgcgctatgacggcaataaaaagacagaataaaacgcacgggtgttgggtcgtttgttcataaacgcggggttcggtcccagggctggcactctgtcgataccccaccgagaccccattggggccaatacgcccgcgtttcttccttttccccaccccaccccccaagttcgggtgaaggcccagggctcgcagccaacgtcggggcggcaggccctgccatagcagatctgcgcagctggggctctagggggtatccccacgcgccctgtagcggcgcattaagcgcggcgggtgtggtggttacgcgcagcgtgaccgctacacttgccagcgccctagcgcccgctcctttcgctttcttcccttcctttctcgccacgttcgccggctttccccgtcaagctctaaatcgggggctccctttagggttccgatttagtgctttacggcacctcgaccccaaaaaacttgattagggtgatggttcacgtagtgggccatcgccctgatagacggtttttcgccctttgacgttggagtccacgttctttaatagtggactcttgttccaaactggaacaacactcaaccctatctcggtctattcttttgatttataagggattttgccgatttcggcctattggttaaaaaatgagctgatttaacaaaaatttaacgcgaattaattctgtggaatgtgtgtcagttagggtgtggaaagtccccaggctccccagcaggcagaagtatgcaaagcatgcatctcaattagtcagcaaccaggtgtggaaagtccccaggctccccagcaggcagaagtatgcaaagcatgcatctcaattagtcagcaaccatagtcccgcccctaactccgcccatcccgcccctaactccgcccagttccgcccattctccgccccatggctgactaattttttttatttatgcagaggccgaggccgcctctgcctctgagctattccagaagtagtgaggaggcttttttggaggcctaggcttttgcaaaaagctcccgggagcttgtatatccattttcggatctgatcaagagacaggatgaggatcgtttcgcatgattgaacaagatggattgcacgcaggttctccggccgcttgggtggagaggctattcggctatgactgggcacaacagacaatcggctgctctgatgccgccgtgttccggctgtcagcgcaggggcgcccggttctttttgtcaagaccgacctgtccggtgccctgaatgaactgcaggacgaggcagcgcggctatcgtggctggccacgacgggcgttccttgcgcagctgtgctcgacgttgtcactgaagcgggaagggactggctgctattgggcgaagtgccggggcaggatctcctgtcatctcaccttgctcctgccgagaaagtatccatcatggctgatgcaatgcggcggctgcatacgcttgatccggctacctgcccattcgaccaccaagcgaaacatcgcatcgagcgagcacgtactcggatggaagccggtcttgtcgatcaggatgatctggacgaagagcatcaggggctcgcgccagccgaactgttcgccaggctcaaggcgcgcatgcccgacggcgaggatctcgtcgtgacccatggcgatgcctgcttgccgaatatcatggtggaaaatggccgcttttctggattcatcgactgtggccggctgggtgtggcggaccgctatcaggacatagcgttggctacccgtgatattgctgaagagcttggcggcgaatgggctgaccgcttcctcgtgctttacggtatcgccgctcccgattcgcagcgcatcgccttctatcgccttcttgacgagttcttctgagcgggactctggggttcgcgaaatgaccgaccaagcgacgcccaacctgccatcacgagatttcgattccaccgccgccttctatgaaaggttgggcttcggaatcgttttccgggacgccggctggatgatcctccagcgcggggatctcatgctggagttcttcgcccaccccaacttgtttattgcagcttataatggttacaaataaagcaatagcatcacaaatttcacaaataaagcatttttttcactgcattctagttgtggtttgtccaaactcatcaatgtatcttatcatgtctgtataccgtcgacctctagctagagcttggcgtaatcatggtcatagctgtttcctgtgtgaaattgttatccgctcacaattccacacaacatacgagccggaagcataaagtgtaaagcctggggtgcctaatgagtgagctaactcacattaattgcgttgcgctcactgcccgctttccagtcgggaaacctgtcgtgccagctgcattaatgaatcggccaacgcgcggggagaggcggtttgcgtattgggcgctcttccgcttcctcgctcactgactcgctgcgctcggtcgttcggctgcggcgagcggtatcagctcactcaaaggcggtaatacggttatccacagaatcaggggataacgcaggaaagaacatgtgagcaaaaggccagcaaaaggccaggaaccgtaaaaaggccgcgttgctggcgtttttccataggctccgcccccctgacgagcatcacaaaaatcgacgctcaagtcagaggtggcgaaacccgacaggactataaagataccaggcgtttccccctggaagctccctcgtgcgctctcctgttccgaccctgccgcttaccggatacctgtccgcctttctcccttcgggaagcgtggcgctttctcatagctcacgctgtaggtatctcagttcggtgtaggtcgttcgctccaagctgggctgtgtgcacgaaccccccgttcagcccgaccgctgcgccttatccggtaactatcgtcttgagtccaacccggtaagacacgacttatcgccactggcagcagccactggtaacaggattagcagagcgaggtatgtaggcggtgctacagagttcttgaagtggtggcctaactacggctacactagaagaacagtatttggtatctgcgctctgctgaagccagttaccttcggaaaaagagttggtagctcttgatccggcaaacaaaccaccgctggtagcggtggtttttttgtttgcaagcagcagattacgcgcagaaaaaaaggatctcaagaagatcctttgatcttttctacggggtctgacgctcagtggaacgaaaactcacgttaagggattttggtcatgagattatcaaaaaggatcttcacctagatccttttaaattaaaaatgaagttttaaatcaatctaaagtatatatgagtaaacttggtctgacagttaccaatgcttaatcagtgaggcacctatctcagcgatctgtctatttcgttcatccatagttgcctgactccccgtcgtgtagataactacgatacgggagggcttaccatctggccccagtgctgcaatgataccgcgagacccacgctcaccggctccagatttatcagcaataaaccagccagccggaagggccgagcgcagaagtggtcctgcaactttatccgcctccatccagtctattaattgttgccgggaagctagagtaagtagttcgccagttaatagtttgcgcaacgttgttgccattgctacaggcatcgtggtgtcacgctcgtcgtttggtatggcttcattcagctccggttcccaacgatcaaggcgagttacatgatcccccatgttgtgcaaaaaagcggttagctccttcggtcctccgatcgttgtcagaagtaagttggccgcagtgttatcactcatggttatggcagcactgcataattctcttactgtcatgccatccgtaagatgcttttctgtgactggtgagtactcaaccaagtcattctgagaatagtgtatgcggcgaccgagttgctcttgcccggcgtcaatacgggataataccgcgccacatagcagaactttaaaagtgctcatcattggaaaacgttcttcggggcgaaaactctcaaggatcttaccgctgttgagatccagttcgatgtaacccactcgtgcacccaactgatcttcagcatcttttactttcaccagcgtttctgggtgagcaaaaacaggaaggcaaaatgccgcaaaaaagggaataagggcgacacggaaatgttgaatactcatactcttcctttttcaatattattgaagcatttatcagggttattgtctcatgagcggatacatatttgaatgtatttagaaaaataaacaaataggggttccgcgcacatttccccgaaaagtgccacctgacgtcgacggatcgggagatctcccgatcccctatggtgcactctcagtacaatctgctctgatgccgcatagttaagccagtatctgctccctgcttgtgtgttggaggtcgctgagtagtgcgcgagcaaaatttaagctacaacaaggcaaggcttgaccgacaattgcatgaagaatctgcttagggttaggcgttttgcgctgcttcgcgatgtacgggccagagggcctatttcccatgattccttcatatttgcatatacgatacaaggctgttagagagataattggaattaatttgactgtaaacacaaagatattagtacaaaatacgtgacgtagaaagtaataatttcttgggtagtttgcagttttaaaattatgttttaaaatggactatcatatgcttaccgtaacttgaaagtatttcgatttcttggctttatatatcttgtggaaaggacgaaacaccgtcgagtcgcttctcgattagttttagagctagaaatagcaagttaaaataaggctagtccgttatcaacttgaaaaagtggcaccgagtcggtgcttttttgttttagagctagaaatagcaagttaaaataaggctagtccgtttttagcgcgtgcgccaattctgcagacaaatgatatacgcgttgacattgattattgactagttattaatagtaatcaattacggggtcattagttcatagcccatatatggagttccgcgttacataacttacggtaaatggcccgcctggctgaccgcccaacgacccccgcccattgacgtcaataatgacgtatgttcccatagtaacgccaatagggactttccattgacgtcaatgggtggagtatttacggtaaactgcccacttggcagtacatcaagtgtatcatatgccaagtacgccccctattgacgtcaatgacggtaaatggcccgcctggcattatgcccagtacatgaccttatgggactttcctacttggcagtacatctacgtattagtcatcgctattaccatg

SEQ ID NO: 140 - DNA, 5964 bp, synthetic construct
  source 1..5964: mol_type = other DNA
atggacaagaagtactccattgggctcgacatcggcacaaacagcgtcggctgggccgtcattacggacgagtacaaggtgccgagcaaaaaattcaaagttctgggcaataccgatcgccacagcataaagaagaacctcattggcgccctcctgttcgactccggggagacggccgaagccacgcggctcaaaagaacagcacggcgcagatatacccgcagaaagaatcggatctgctacctgcaggagatctttagtaatgagatggctaaggtggatgactctttcttccataggctggaggagtcctttttggtggaggaggataaaaagcacgagcgccacccaatctttggcaatatcgtggacgaggtggcgtaccatgaaaagtacccaaccatatatcatctgaggaagaagcttgtagacagtactgataaggctgacttgcggttgatctatctcgcgctggcgcatatgatcaaatttcggggacacttcctcatcgagggggacctgaacccagacaacagcgatgtcgacaaactctttatccaactggttcagacttacaatcagcttttcgaagagaacccgatcaacgcatccggagttgacgccaaagcaatcctgagcgctaggctgtccaaatcccggcggctcgaaaacctcatcgcacagctccctggggagaagaagaacggcctgtttggtaatcttatcgccctgtcactcgggctgacccccaactttaaatctaacttcgacctggccgaagatgccaagcttcaactgagcaaagacacctacgatgatgatctcgacaatctgctggcccagatcggcgaccagtacgcagacctttttttggcggcaaagaacctgtcagacgccattctgctgagtgatattctgcgagtgaacacggagatcaccaaagctccgctgagcgctagtatgatcaagcgctatgatgagcaccaccaagacttgactttgctgaaggcccttgtcagacagcaactgcctgagaagtacaaggaaattttcttcgatcagtctaaaaatggctacgccggatacattgacggcggagcaagccaggaggaattttacaaatttattaagcccatcttggaaaaaatggacggcaccgaggagctgctggtaaagcttaacagagaagatctgttgcgcaaacagcgcactttcgacaatggaagcatcccccaccagattcacctgggcgaactgcacgctatcctcaggcggcaagaggatttctacccctttttgaaagataacagggaaaagattgagaaaatcctcacatttcggataccctactatgtaggccccctcgcccggggaaattccagattcgcgtggatgactcgcaaatcagaagagaccatcactccctggaacttcgaggaagtcgtggataagggggcctctgcccagtccttcatcgaaaggatgactaactttgataaaaatctgcctaacgaaaaggtgcttcctaaacactctctgctgtacgagtacttcacagtttataacgagctcaccaaggtcaaatacgtcacagaagggatgagaaagccagcattcctgtctggagagcagaagaaagctatcgtggacctcctcttcaagacgaaccggaaagttaccgtgaaacagctcaaagaagactatttcaaaaagattgaatgtttcgactctgttgaaatcagcggagtggaggatcgcttcaacgcatccctgggaacgtatcacgatctcctgaaaatcattaaagacaaggacttcctggacaatgaggagaacgaggacattcttgaggacattgtcctcacccttacgttgtttgaagatagggagatgattgaagaacgcttgaaaacttacgctcatctcttcgacgacaaagtcatgaaacagctcaagaggcgccgatatacaggatgggggcggctgtcaagaaaactgatcaatgggatccgagacaagcagagtggaaagacaatcctggattttcttaagtccgatggatttgccaacaggaacttcatgcagttgatccatgatgactctctcacctttaaggaggacatccagaaagcacaagtttctggccagggggacagtcttcacgagcacatcgctaatcttgcaggtagcccagctatcaaaaagggaatactgcagaccgttaaggtcgtggatgaactcgtcaaagtaatgggaaggcataagcccgagaatatcgttatcgagatggcccgagagaaccaaactacccagaagggacagaagaacagtagggaaaggatgaagaggattgaagagggtataaaagaactggggtcccaaatccttaaggaacacccagttgaaaacacccagcttcagaatgagaagctctacctgtactacctgcagaacggcagggacatgtacgtggatcaggaactggacatcaatcggctctccgactacgacgtggatcatatcgtgccccagtcttttctcaaagatgattctattgataataaagtgttgacaagatccgataaaaatagagggaagagtgataacgtcccctcagaagaagttgtcaagaaaatgaaaaattattggcggcagctgctgaacgccaaactgatcacacaacggaagttcgataatctgactaaggctgaacgaggtggcctgtctgagttggataaagccggcttcatcaaaaggcagcttgttgagacacgccagatcaccaagcacgtggcccaaattctcgattcacgcatgaacaccaagtacgatgaaaatgacaaactgattcgagaggtgaaagttattactctgaagtctaagctggtctcagatttcagaaaggactttcagttttataaggtgagagagatcaacaattaccaccatgcgcatgatgcctacctgaatgcagtggtaggcactgcacttatcaaaaaatatcccaagcttgaatctgaatttgtttacggagactataaagtgtacgatgttaggaaaatgatcgcaaagtctgagcaggaaataggcaaggccaccgctaagtacttcttttacagcaatattatgaattttttcaagaccgagattacactggccaatggagagattcggaagcgaccacttatcgaaacaaacggagaaacaggagaaatcgtgtgggacaagggtagggatttcgcgacagtccggaaggtcctgtccatgccgcaggtgaacatcgttaaaaagaccgaagtacagaccggaggcttctccaaggaaagtatcctcccgaaaaggaacagcgacaagctgatcgcacgcaaaaaagattgggaccccaagaaatacggcggattcgattctcctacagtcgcttacagtgtactggttgtggccaaagtggagaaagggaagtctaaaaaactcaaaagcgtcaaggaactgctgggcatcacaatcatggagcgatcaagcttcgaaaaaaaccccatcgactttctcgaggcgaaaggatataaagaggtcaaaaaagacctcatcattaagcttcccaagtactctctctttgagcttgaaaacggccggaaacgaatgctcgctagtgcgggcgagctgcagaaaggtaacgagctggcactgccctctaaatacgttaatttcttgtatctggccagccactatgaaaagctcaaagggtctcccgaagataatgagcagaagcagctgttcgtggaacaacacaaacactaccttgatgagatcatcgagcaaataagcgaattctccaaaagagtgatcctcgccgacgctaacctcgataaggtgctttctgcttacaataagcacagggataagcccatcagggagcaggcagaaaacattatccacttgtttactctgaccaacttgggcgcgcctgcagccttcaagtacttcgacaccaccatagacagaaagcggtacacctctacaaaggaggtcctggacgccacactgattcatcagtcaattacggggctctatgaaacaagaatcgacctctctcagctcggtggagacagcagggctgaccccaagaagaagaggaaggtgggcggaggagggagtggcggaggcggaagcggcggcggaggcagcggctctagcctggacgacgagcacatcctgagcgccctgctgcagagcgacgacgaactggtgggcgaggacagcgacagcgaggtcagcgaccacgtgtccgaggacgacgtgcagtccgacaccgaggaagccttcatcgacgaggtgcacgaagtgcagcctaccagcagcggctccgagatcctggacgagcagaacgtgatcgagcagcctggcagctccctggccagcaacagaatcctgaccctgccccagagaaccatcagaggcaagaacaagcactgctggtccacctccaagagcaccaggcggagcagagtgtccgccctgaacatcgtgcggagccagaggggccccaccagaatgtgcagaaacatctacgaccccctgctgtgcttcaagctgttcttcaccgacgagatcatcagcgagatcgtgaagtggaccaacgccgagatcagcctgaagaggcgggagagcatgaccagcgccaccttcagagacaccaacgaggacgagatctacgccttcttcggcatcctggtgatgaccgccgtgagaaaggacaaccacatgagcaccgacgacctgttcgacagatccctgagcatggtgtacgtgtccgtgatgagcagagacagattcgacttcctgatcagatgcctgagaatggacgacaagagcatcagacccaccctgcgggagaacgacgtgttcacccccgtgcggaagatctgggacctgttcatccaccagtgcatccagaactacacccctggcgcccacctgaccatcgatgagcagctgctgggcttcagaggcagatgccccttcagagtgtacatccccaacaagcccagcaagtacggcatcaagatcctgatgatgtgcgacagcggcaccaagtacatgatcaacggcatgccctacctgggcagaggcacccagacaaacggcgtgcccctgggcgagtactacgtgaaagaactgagcaagcctgtgcatggcagctgcaggaacatcacctgcgacaactggttcaccagcatccccctggccaagaacctgctgcaggaaccctacaagctgaccatcgtgggcaccgtggccagcaacgcccgggagatcccagaggtgctgaagaacagcagatccagacctgtgggaacaagcatgttctgcttcgacggccccctgaccctggtgtcctacaagcccaagcccgccaagatggtgtacctgctgtccagctgcgacgaggacgccagcatcaacgagagcaccggcaagccccagatggtgatgtactacaaccagaccaagggcggcgtggacaccctgaaccagatgtgcagcgtgatgacctgcagcagaaagaccaacagatggcccatggccctgctgtacggcatgatcaatatcgcctgcatcaacagcttcatcatctacagccacaacgtgtccagcaagggcgagaaggtgcagagccggaagaaattcatgcggaacctgtacatgagcctgacctccagcttcatgagaaagagactggaagcccccaccctgaagagatacctgcgggacaacatcagcaacatcctgcccaaggaagtgccaggaacaagcgacgacagcaccgaggaacccgtgatgaagaagaggacctactgcacctactgtcccagcaagatcagaagaaaggccaacgccagctgcaagaaatgcaaaaaagtgatctgccgggagcacaacatcgacatgtgccagagctgtttctga